European Patent Application EP 4 248 993 A1, published September 27, 2023. Title: New MERS CoV Vaccine. Applicant: Max-Delbrück-Centrum für Molekulare Medizin in der Helmholtz-Gemeinschaft. The sequence listing filed with the application follows.

SEQUENCE LISTING (153 sequences)

SEQ ID NO: 1 - protein, 217 aa, MERS-CoV
  wildtype receptor bindung domain of MERS-CoV
GSVVEQAEGVECDFSPLLSGTPPQVYNFKRLVFTNCNYNLTKLLSLFSVNDFTCSQISPAAIASNCYSSLILDYFSYPLSMKSDLSVSSAGPISQFNYKQSFSNPTCLILATVPHNLTTITKPLKYSYINKCSRLLSDDRTEVPQLVNANQYSPCVSIVPSTVWEDGDYYRKQLSPLEGGGWLVASGSTVAMTEQLQMGFGITVQYGTDTNSVCPKL

SEQ ID NO: 2 - protein, 217 aa, Artificial Sequence
  mutant receptor binding domain of MERS-CoV comprising substitution S94W
GSVVEQAEGVECDFSPLLSGTPPQVYNFKRLVFTNCNYNLTKLLSLFSVNDFTCSQISPAAIASNCYSSLILDYFSYPLSMKSDLSVSWAGPISQFNYKQSFSNPTCLILATVPHNLTTITKPLKYSYINKCSRLLSDDRTEVPQLVNANQYSPCVSIVPSTVWEDGDYYRKQLSPLEGGGWLVASGSTVAMTEQLQMGFGITVQYGTDTNSVCPKL

SEQ ID NO: 3 - protein, 217 aa, Artificial Sequence
  mutant receptor binding domain of MERS-CoV comprising substitution G96R
GSVVEQAEGVECDFSPLLSGTPPQVYNFKRLVFTNCNYNLTKLLSLFSVNDFTCSQISPAAIASNCYSSLILDYFSYPLSMKSDLSVSSARPISQFNYKQSFSNPTCLILATVPHNLTTITKPLKYSYINKCSRLLSDDRTEVPQLVNANQYSPCVSIVPSTVWEDGDYYRKQLSPLEGGGWLVASGSTVAMTEQLQMGFGITVQYGTDTNSVCPKL

SEQ ID NO: 4 - protein, 217 aa, Artificial Sequence
  mutant receptor binding domain of MERS-CoV comprising substitution G96Q
GSVVEQAEGVECDFSPLLSGTPPQVYNFKRLVFTNCNYNLTKLLSLFSVNDFTCSQISPAAIASNCYSSLILDYFSYPLSMKSDLSVSSAQPISQFNYKQSFSNPTCLILATVPHNLTTITKPLKYSYINKCSRLLSDDRTEVPQLVNANQYSPCVSIVPSTVWEDGDYYRKQLSPLEGGGWLVASGSTVAMTEQLQMGFGITVQYGTDTNSVCPKL

SEQ ID NO: 5 - protein, 217 aa, Artificial Sequence
  mutant receptor binding domain of MERS-CoV comprising substitution G96L
GSVVEQAEGVECDFSPLLSGTPPQVYNFKRLVFTNCNYNLTKLLSLFSVNDFTCSQISPAAIASNCYSSLILDYFSYPLSMKSDLSVSSALPISQFNYKQSFSNPTCLILATVPHNLTTITKPLKYSYINKCSRLLSDDRTEVPQLVNANQYSPCVSIVPSTVWEDGDYYRKQLSPLEGGGWLVASGSTVAMTEQLQMGFGITVQYGTDTNSVCPKL

SEQ ID NO: 6 - protein, 217 aa, Artificial Sequence
  mutant receptor binding domain of MERS-CoV comprising substitution G96W
GSVVEQAEGVECDFSPLLSGTPPQVYNFKRLVFTNCNYNLTKLLSLFSVNDFTCSQISPAAIASNCYSSLILDYFSYPLSMKSDLSVSSAWPISQFNYKQSFSNPTCLILATVPHNLTTITKPLKYSYINKCSRLLSDDRTEVPQLVNANQYSPCVSIVPSTVWEDGDYYRKQLSPLEGGGWLVASGSTVAMTEQLQMGFGITVQYGTDTNSVCPKL

SEQ ID NO: 7 - protein, 217 aa, Artificial Sequence
  mutant receptor binding domain of MERS-CoV comprising substitution G96Y
GSVVEQAEGVECDFSPLLSGTPPQVYNFKRLVFTNCNYNLTKLLSLFSVNDFTCSQISPAAIASNCYSSLILDYFSYPLSMKSDLSVSSAYPISQFNYKQSFSNPTCLILATVPHNLTTITKPLKYSYINKCSRLLSDDRTEVPQLVNANQYSPCVSIVPSTVWEDGDYYRKQLSPLEGGGWLVASGSTVAMTEQLQMGFGITVQYGTDTNSVCPKL

SEQ ID NO: 8 - protein, 217 aa, Artificial Sequence
  mutant receptor binding domain of MERS-CoV comprising substitution G96F
GSVVEQAEGVECDFSPLLSGTPPQVYNFKRLVFTNCNYNLTKLLSLFSVNDFTCSQISPAAIASNCYSSLILDYFSYPLSMKSDLSVSSAFPISQFNYKQSFSNPTCLILATVPHNLTTITKPLKYSYINKCSRLLSDDRTEVPQLVNANQYSPCVSIVPSTVWEDGDYYRKQLSPLEGGGWLVASGSTVAMTEQLQMGFGITVQYGTDTNSVCPKL

SEQ ID NO: 9 - protein, 217 aa, Artificial Sequence
  mutant receptor binding domain of MERS-CoV comprising substitution S132W
GSVVEQAEGVECDFSPLLSGTPPQVYNFKRLVFTNCNYNLTKLLSLFSVNDFTCSQISPAAIASNCYSSLILDYFSYPLSMKSDLSVSSAGPISQFNYKQSFSNPTCLILATVPHNLTTITKPLKYWYINKCSRLLSDDRTEVPQLVNANQYSPCVSIVPSTVWEDGDYYRKQLSPLEGGGWLVASGSTVAMTEQLQMGFGITVQYGTDTNSVCPKL

SEQ ID NO: 10 - protein, 217 aa, Artificial Sequence
  mutant receptor binding domain of MERS-CoV comprising substitution S138W
GSVVEQAEGVECDFSPLLSGTPPQVYNFKRLVFTNCNYNLTKLLSLFSVNDFTCSQISPAAIASNCYSSLILDYFSYPLSMKSDLSVSSAGPISQFNYKQSFSNPTCLILATVPHNLTTITKPLKYSYINKCWRLLSDDRTEVPQLVNANQYSPCVSIVPSTVWEDGDYYRKQLSPLEGGGWLVASGSTVAMTEQLQMGFGITVQYGTDTNSVCPKL

SEQ ID NO: 11 - protein, 217 aa, Artificial Sequence
  mutant receptor binding domain of MERS-CoV comprising substitution L140R
GSVVEQAEGVECDFSPLLSGTPPQVYNFKRLVFTNCNYNLTKLLSLFSVNDFTCSQISPAAIASNCYSSLILDYFSYPLSMKSDLSVSSAGPISQFNYKQSFSNPTCLILATVPHNLTTITKPLKYSYINKCSRRLSDDRTEVPQLVNANQYSPCVSIVPSTVWEDGDYYRKQLSPLEGGGWLVASGSTVAMTEQLQMGFGITVQYGTDTNSVCPKL

SEQ ID NO: 12 - protein, 217 aa, Artificial Sequence
  mutant receptor binding domain of MERS-CoV comprising substitution L140W
GSVVEQAEGVECDFSPLLSGTPPQVYNFKRLVFTNCNYNLTKLLSLFSVNDFTCSQISPAAIASNCYSSLILDYFSYPLSMKSDLSVSSAGPISQFNYKQSFSNPTCLILATVPHNLTTITKPLKYSYINKCSRWLSDDRTEVPQLVNANQYSPCVSIVPSTVWEDGDYYRKQLSPLEGGGWLVASGSTVAMTEQLQMGFGITVQYGTDTNSVCPKL

SEQ ID NO: 13 - protein, 217 aa, Artificial Sequence
  mutant receptor binding domain of MERS-CoV comprising substitution L140Y
GSVVEQAEGVECDFSPLLSGTPPQVYNFKRLVFTNCNYNLTKLLSLFSVNDFTCSQISPAAIASNCYSSLILDYFSYPLSMKSDLSVSSAGPISQFNYKQSFSNPTCLILATVPHNLTTITKPLKYSYINKCSRYLSDDRTEVPQLVNANQYSPCVSIVPSTVWEDGDYYRKQLSPLEGGGWLVASGSTVAMTEQLQMGFGITVQYGTDTNSVCPKL

SEQ ID NO: 14 - protein, 217 aa, Artificial Sequence
  mutant receptor binding domain of MERS-CoV comprising substitution L140H
GSVVEQAEGVECDFSPLLSGTPPQVYNFKRLVFTNCNYNLTKLLSLFSVNDFTCSQISPAAIASNCYSSLILDYFSYPLSMKSDLSVSSAGPISQFNYKQSFSNPTCLILATVPHNLTTITKPLKYSYINKCSRHLSDDRTEVPQLVNANQYSPCVSIVPSTVWEDGDYYRKQLSPLEGGGWLVASGSTVAMTEQLQMGFGITVQYGTDTNSVCPKL

SEQ ID NO: 15 - protein, 217 aa, Artificial Sequence
  mutant receptor binding domain of MERS-CoV comprising substitution G172H
GSVVEQAEGVECDFSPLLSGTPPQVYNFKRLVFTNCNYNLTKLLSLFSVNDFTCSQISPAAIASNCYSSLILDYFSYPLSMKSDLSVSSAGPISQFNYKQSFSNPTCLILATVPHNLTTITKPLKYSYINKCSRLLSDDRTEVPQLVNANQYSPCVSIVPSTVWEDHDYYRKQLSPLEGGGWLVASGSTVAMTEQLQMGFGITVQYGTDTNSVCPKL

SEQ ID NO: 16 - protein, 217 aa, Artificial Sequence
  mutant receptor binding domain of MERS-CoV comprising substitution G172W
GSVVEQAEGVECDFSPLLSGTPPQVYNFKRLVFTNCNYNLTKLLSLFSVNDFTCSQISPAAIASNCYSSLILDYFSYPLSMKSDLSVSSAGPISQFNYKQSFSNPTCLILATVPHNLTTITKPLKYSYINKCSRLLSDDRTEVPQLVNANQYSPCVSIVPSTVWEDWDYYRKQLSPLEGGGWLVASGSTVAMTEQLQMGFGITVQYGTDTNSVCPKL

SEQ ID NO: 17 - protein, 217 aa, Artificial Sequence
  mutant receptor binding domain of MERS-CoV comprising substitution G172E
GSVVEQAEGVECDFSPLLSGTPPQVYNFKRLVFTNCNYNLTKLLSLFSVNDFTCSQISPAAIASNCYSSLILDYFSYPLSMKSDLSVSSAGPISQFNYKQSFSNPTCLILATVPHNLTTITKPLKYSYINKCSRLLSDDRTEVPQLVNANQYSPCVSIVPSTVWEDEDYYRKQLSPLEGGGWLVASGSTVAMTEQLQMGFGITVQYGTDTNSVCPKL

SEQ ID NO: 18 - protein, 217 aa, Artificial Sequence
  mutant receptor binding domain of MERS-CoV comprising substitution G172K
GSVVEQAEGVECDFSPLLSGTPPQVYNFKRLVFTNCNYNLTKLLSLFSVNDFTCSQISPAAIASNCYSSLILDYFSYPLSMKSDLSVSSAGPISQFNYKQSFSNPTCLILATVPHNLTTITKPLKYSYINKCSRLLSDDRTEVPQLVNANQYSPCVSIVPSTVWEDKDYYRKQLSPLEGGGWLVASGSTVAMTEQLQMGFGITVQYGTDTNSVCPKL

SEQ ID NO: 19 - protein, 217 aa, Artificial Sequence
  mutant receptor binding domain of MERS-CoV comprising substitution G172F
GSVVEQAEGVECDFSPLLSGTPPQVYNFKRLVFTNCNYNLTKLLSLFSVNDFTCSQISPAAIASNCYSSLILDYFSYPLSMKSDLSVSSAGPISQFNYKQSFSNPTCLILATVPHNLTTITKPLKYSYINKCSRLLSDDRTEVPQLVNANQYSPCVSIVPSTVWEDFDYYRKQLSPLEGGGWLVASGSTVAMTEQLQMGFGITVQYGTDTNSVCPKL

SEQ ID NO: 20 - protein, 217 aa, Artificial Sequence
  mutant receptor binding domain of MERS-CoV comprising substitution G172L
GSVVEQAEGVECDFSPLLSGTPPQVYNFKRLVFTNCNYNLTKLLSLFSVNDFTCSQISPAAIASNCYSSLILDYFSYPLSMKSDLSVSSAGPISQFNYKQSFSNPTCLILATVPHNLTTITKPLKYSYINKCSRLLSDDRTEVPQLVNANQYSPCVSIVPSTVWEDLDYYRKQLSPLEGGGWLVASGSTVAMTEQLQMGFGITVQYGTDTNSVCPKL

SEQ ID NO: 21 - protein, 217 aa, Artificial Sequence
  mutant receptor binding domain of MERS-CoV comprising substitution G172S
GSVVEQAEGVECDFSPLLSGTPPQVYNFKRLVFTNCNYNLTKLLSLFSVNDFTCSQISPAAIASNCYSSLILDYFSYPLSMKSDLSVSSAGPISQFNYKQSFSNPTCLILATVPHNLTTITKPLKYSYINKCSRLLSDDRTEVPQLVNANQYSPCVSIVPSTVWEDSDYYRKQLSPLEGGGWLVASGSTVAMTEQLQMGFGITVQYGTDTNSVCPKL

SEQ ID NO: 22 - protein, 217 aa, Artificial Sequence
  mutant receptor binding domain of MERS-CoV comprising substitution G172Y
GSVVEQAEGVECDFSPLLSGTPPQVYNFKRLVFTNCNYNLTKLLSLFSVNDFTCSQISPAAIASNCYSSLILDYFSYPLSMKSDLSVSSAGPISQFNYKQSFSNPTCLILATVPHNLTTITKPLKYSYINKCSRLLSDDRTEVPQLVNANQYSPCVSIVPSTVWEDYDYYRKQLSPLEGGGWLVASGSTVAMTEQLQMGFGITVQYGTDTNSVCPKL

SEQ ID NO: 23 - protein, 217 aa, Artificial Sequence
  mutant receptor binding domain of MERS-CoV comprising substitution G172C
GSVVEQAEGVECDFSPLLSGTPPQVYNFKRLVFTNCNYNLTKLLSLFSVNDFTCSQISPAAIASNCYSSLILDYFSYPLSMKSDLSVSSAGPISQFNYKQSFSNPTCLILATVPHNLTTITKPLKYSYINKCSRLLSDDRTEVPQLVNANQYSPCVSIVPSTVWEDCDYYRKQLSPLEGGGWLVASGSTVAMTEQLQMGFGITVQYGTDTNSVCPKL

SEQ ID NO: 24 - protein, 217 aa, Artificial Sequence
  mutant receptor binding domain of MERS-CoV comprising substitution G172P
GSVVEQAEGVECDFSPLLSGTPPQVYNFKRLVFTNCNYNLTKLLSLFSVNDFTCSQISPAAIASNCYSSLILDYFSYPLSMKSDLSVSSAGPISQFNYKQSFSNPTCLILATVPHNLTTITKPLKYSYINKCSRLLSDDRTEVPQLVNANQYSPCVSIVPSTVWEDPDYYRKQLSPLEGGGWLVASGSTVAMTEQLQMGFGITVQYGTDTNSVCPKL

SEQ ID NO: 25 - protein, 217 aa, Artificial Sequence
  mutant receptor binding domain of MERS-CoV comprising substitution G172Q
GSVVEQAEGVECDFSPLLSGTPPQVYNFKRLVFTNCNYNLTKLLSLFSVNDFTCSQISPAAIASNCYSSLILDYFSYPLSMKSDLSVSSAGPISQFNYKQSFSNPTCLILATVPHNLTTITKPLKYSYINKCSRLLSDDRTEVPQLVNANQYSPCVSIVPSTVWEDQDYYRKQLSPLEGGGWLVASGSTVAMTEQLQMGFGITVQYGTDTNSVCPKL

SEQ ID NO: 26 - protein, 217 aa, Artificial Sequence
  mutant receptor binding domain of MERS-CoV comprising substitution G172I
GSVVEQAEGVECDFSPLLSGTPPQVYNFKRLVFTNCNYNLTKLLSLFSVNDFTCSQISPAAIASNCYSSLILDYFSYPLSMKSDLSVSSAGPISQFNYKQSFSNPTCLILATVPHNLTTITKPLKYSYINKCSRLLSDDRTEVPQLVNANQYSPCVSIVPSTVWEDIDYYRKQLSPLEGGGWLVASGSTVAMTEQLQMGFGITVQYGTDTNSVCPKL

SEQ ID NO: 27 - protein, 217 aa, Artificial Sequence
  mutant receptor binding domain of MERS-CoV comprising substitution G172M
GSVVEQAEGVECDFSPLLSGTPPQVYNFKRLVFTNCNYNLTKLLSLFSVNDFTCSQISPAAIASNCYSSLILDYFSYPLSMKSDLSVSSAGPISQFNYKQSFSNPTCLILATVPHNLTTITKPLKYSYINKCSRLLSDDRTEVPQLVNANQYSPCVSIVPSTVWEDMDYYRKQLSPLEGGGWLVASGSTVAMTEQLQMGFGITVQYGTDTNSVCPKL

SEQ ID NO: 28 - protein, 217 aa, Artificial Sequence
  mutant receptor binding domain of MERS-CoV comprising substitution G172T
GSVVEQAEGVECDFSPLLSGTPPQVYNFKRLVFTNCNYNLTKLLSLFSVNDFTCSQISPAAIASNCYSSLILDYFSYPLSMKSDLSVSSAGPISQFNYKQSFSNPTCLILATVPHNLTTITKPLKYSYINKCSRLLSDDRTEVPQLVNANQYSPCVSIVPSTVWEDTDYYRKQLSPLEGGGWLVASGSTVAMTEQLQMGFGITVQYGTDTNSVCPKL

SEQ ID NO: 29 - protein, 217 aa, Artificial Sequence
  mutant receptor binding domain of MERS-CoV comprising substitution G172N
GSVVEQAEGVECDFSPLLSGTPPQVYNFKRLVFTNCNYNLTKLLSLFSVNDFTCSQISPAAIASNCYSSLILDYFSYPLSMKSDLSVSSAGPISQFNYKQSFSNPTCLILATVPHNLTTITKPLKYSYINKCSRLLSDDRTEVPQLVNANQYSPCVSIVPSTVWEDNDYYRKQLSPLEGGGWLVASGSTVAMTEQLQMGFGITVQYGTDTNSVCPKL

SEQ ID NO: 30 - protein, 217 aa, Artificial Sequence
  mutant receptor binding domain of MERS-CoV comprising substitution G172R
GSVVEQAEGVECDFSPLLSGTPPQVYNFKRLVFTNCNYNLTKLLSLFSVNDFTCSQISPAAIASNCYSSLILDYFSYPLSMKSDLSVSSAGPISQFNYKQSFSNPTCLILATVPHNLTTITKPLKYSYINKCSRLLSDDRTEVPQLVNANQYSPCVSIVPSTVWEDRDYYRKQLSPLEGGGWLVASGSTVAMTEQLQMGFGITVQYGTDTNSVCPKL

SEQ ID NO: 31 - protein, 217 aa, Artificial Sequence
  mutant receptor binding domain of MERS-CoV comprising substitution G172V
GSVVEQAEGVECDFSPLLSGTPPQVYNFKRLVFTNCNYNLTKLLSLFSVNDFTCSQISPAAIASNCYSSLILDYFSYPLSMKSDLSVSSAGPISQFNYKQSFSNPTCLILATVPHNLTTITKPLKYSYINKCSRLLSDDRTEVPQLVNANQYSPCVSIVPSTVWEDVDYYRKQLSPLEGGGWLVASGSTVAMTEQLQMGFGITVQYGTDTNSVCPKL

SEQ ID NO: 32 - protein, 217 aa, Artificial Sequence
  mutant receptor binding domain of MERS-CoV comprising substitution G172A
GSVVEQAEGVECDFSPLLSGTPPQVYNFKRLVFTNCNYNLTKLLSLFSVNDFTCSQISPAAIASNCYSSLILDYFSYPLSMKSDLSVSSAGPISQFNYKQSFSNPTCLILATVPHNLTTITKPLKYSYINKCSRLLSDDRTEVPQLVNANQYSPCVSIVPSTVWEDADYYRKQLSPLEGGGWLVASGSTVAMTEQLQMGFGITVQYGTDTNSVCPKL

SEQ ID NO: 33 - protein, 217 aa, Artificial Sequence
  mutant receptor binding domain of MERS-CoV comprising substitution G172D
GSVVEQAEGVECDFSPLLSGTPPQVYNFKRLVFTNCNYNLTKLLSLFSVNDFTCSQISPAAIASNCYSSLILDYFSYPLSMKSDLSVSSAGPISQFNYKQSFSNPTCLILATVPHNLTTITKPLKYSYINKCSRLLSDDRTEVPQLVNANQYSPCVSIVPSTVWEDDDYYRKQLSPLEGGGWLVASGSTVAMTEQLQMGFGITVQYGTDTNSVCPKL

SEQ ID NO: 34 - protein, 217 aa, Artificial Sequence
  mutant receptor binding domain of MERS-CoV comprising substitution V189W
GSVVEQAEGVECDFSPLLSGTPPQVYNFKRLVFTNCNYNLTKLLSLFSVNDFTCSQISPAAIASNCYSSLILDYFSYPLSMKSDLSVSSAGPISQFNYKQSFSNPTCLILATVPHNLTTITKPLKYSYINKCSRLLSDDRTEVPQLVNANQYSPCVSIVPSTVWEDGDYYRKQLSPLEGGGWLWASGSTVAMTEQLQMGFGITVQYGTDTNSVCPKL

SEQ ID NO: 35 - protein, 217 aa, Artificial Sequence
  mutant receptor binding domain of MERS-CoV comprising substitution V189Y
GSVVEQAEGVECDFSPLLSGTPPQVYNFKRLVFTNCNYNLTKLLSLFSVNDFTCSQISPAAIASNCYSSLILDYFSYPLSMKSDLSVSSAGPISQFNYKQSFSNPTCLILATVPHNLTTITKPLKYSYINKCSRLLSDDRTEVPQLVNANQYSPCVSIVPSTVWEDGDYYRKQLSPLEGGGWLYASGSTVAMTEQLQMGFGITVQYGTDTNSVCPKL

SEQ ID NO: 36 - protein, 217 aa, Artificial Sequence
  mutant receptor binding domain of MERS-CoV comprising substitution V189F
GSVVEQAEGVECDFSPLLSGTPPQVYNFKRLVFTNCNYNLTKLLSLFSVNDFTCSQISPAAIASNCYSSLILDYFSYPLSMKSDLSVSSAGPISQFNYKQSFSNPTCLILATVPHNLTTITKPLKYSYINKCSRLLSDDRTEVPQLVNANQYSPCVSIVPSTVWEDGDYYRKQLSPLEGGGWLFASGSTVAMTEQLQMGFGITVQYGTDTNSVCPKL

SEQ ID NO: 37 - protein, 217 aa, Artificial Sequence
  mutant receptor binding domain of MERS-CoV comprising substitution V189R
GSVVEQAEGVECDFSPLLSGTPPQVYNFKRLVFTNCNYNLTKLLSLFSVNDFTCSQISPAAIASNCYSSLILDYFSYPLSMKSDLSVSSAGPISQFNYKQSFSNPTCLILATVPHNLTTITKPLKYSYINKCSRLLSDDRTEVPQLVNANQYSPCVSIVPSTVWEDGDYYRKQLSPLEGGGWLRASGSTVAMTEQLQMGFGITVQYGTDTNSVCPKL

SEQ ID NO: 38 - protein, 217 aa, Artificial Sequence
  mutant receptor binding domain of MERS-CoV comprising substitution V189K
GSVVEQAEGVECDFSPLLSGTPPQVYNFKRLVFTNCNYNLTKLLSLFSVNDFTCSQISPAAIASNCYSSLILDYFSYPLSMKSDLSVSSAGPISQFNYKQSFSNPTCLILATVPHNLTTITKPLKYSYINKCSRLLSDDRTEVPQLVNANQYSPCVSIVPSTVWEDGDYYRKQLSPLEGGGWLKASGSTVAMTEQLQMGFGITVQYGTDTNSVCPKL

SEQ ID NO: 39 - protein, 217 aa, Artificial Sequence
  mutant receptor binding domain of MERS-CoV comprising substitution S191Y
GSVVEQAEGVECDFSPLLSGTPPQVYNFKRLVFTNCNYNLTKLLSLFSVNDFTCSQISPAAIASNCYSSLILDYFSYPLSMKSDLSVSSAGPISQFNYKQSFSNPTCLILATVPHNLTTITKPLKYSYINKCSRLLSDDRTEVPQLVNANQYSPCVSIVPSTVWEDGDYYRKQLSPLEGGGWLVAYGSTVAMTEQLQMGFGITVQYGTDTNSVCPKL

SEQ ID NO: 40 - protein, 217 aa, Artificial Sequence
  mutant receptor binding domain of MERS-CoV comprising substitution S191W
GSVVEQAEGVECDFSPLLSGTPPQVYNFKRLVFTNCNYNLTKLLSLFSVNDFTCSQISPAAIASNCYSSLILDYFSYPLSMKSDLSVSSAGPISQFNYKQSFSNPTCLILATVPHNLTTITKPLKYSYINKCSRLLSDDRTEVPQLVNANQYSPCVSIVPSTVWEDGDYYRKQLSPLEGGGWLVAWGSTVAMTEQLQMGFGITVQYGTDTNSVCPKL

SEQ ID NO: 41 - protein, 217 aa, Artificial Sequence
  mutant receptor binding domain of MERS-CoV comprising substitution S191F
GSVVEQAEGVECDFSPLLSGTPPQVYNFKRLVFTNCNYNLTKLLSLFSVNDFTCSQISPAAIASNCYSSLILDYFSYPLSMKSDLSVSSAGPISQFNYKQSFSNPTCLILATVPHNLTTITKPLKYSYINKCSRLLSDDRTEVPQLVNANQYSPCVSIVPSTVWEDGDYYRKQLSPLEGGGWLVAFGSTVAMTEQLQMGFGITVQYGTDTNSVCPKL

SEQ ID NO: 42 - protein, 217 aa, Artificial Sequence
  mutant receptor binding domain of MERS-CoV comprising substitution R139L
GSVVEQAEGVECDFSPLLSGTPPQVYNFKRLVFTNCNYNLTKLLSLFSVNDFTCSQISPAAIASNCYSSLILDYFSYPLSMKSDLSVSSAGPISQFNYKQSFSNPTCLILATVPHNLTTITKPLKYSYINKCSLLLSDDRTEVPQLVNANQYSPCVSIVPSTVWEDGDYYRKQLSPLEGGGWLVASGSTVAMTEQLQMGFGITVQYGTDTNSVCPKL

SEQ ID NO: 43 - protein, 217 aa, Artificial Sequence
  mutant receptor binding domain of MERS-CoV comprising substitution V168W
GSVVEQAEGVECDFSPLLSGTPPQVYNFKRLVFTNCNYNLTKLLSLFSVNDFTCSQISPAAIASNCYSSLILDYFSYPLSMKSDLSVSSAGPISQFNYKQSFSNPTCLILATVPHNLTTITKPLKYSYINKCSRLLSDDRTEVPQLVNANQYSPCVSIVPSTWWEDGDYYRKQLSPLEGGGWLVASGSTVAMTEQLQMGFGITVQYGTDTNSVCPKL

SEQ ID NO: 44 - protein, 217 aa, Artificial Sequence
  mutant receptor binding domain of MERS-CoV comprising substitution A190W
GSVVEQAEGVECDFSPLLSGTPPQVYNFKRLVFTNCNYNLTKLLSLFSVNDFTCSQISPAAIASNCYSSLILDYFSYPLSMKSDLSVSSAGPISQFNYKQSFSNPTCLILATVPHNLTTITKPLKYSYINKCSRLLSDDRTEVPQLVNANQYSPCVSIVPSTVWEDGDYYRKQLSPLEGGGWLVWSGSTVAMTEQLQMGFGITVQYGTDTNSVCPKL

SEQ ID NO: 45 - protein, 217 aa, Artificial Sequence
  mutant receptor binding domain of MERS-CoV comprising substitution S193W
GSVVEQAEGVECDFSPLLSGTPPQVYNFKRLVFTNCNYNLTKLLSLFSVNDFTCSQISPAAIASNCYSSLILDYFSYPLSMKSDLSVSSAGPISQFNYKQSFSNPTCLILATVPHNLTTITKPLKYSYINKCSRLLSDDRTEVPQLVNANQYSPCVSIVPSTVWEDGDYYRKQLSPLEGGGWLVASGWTVAMTEQLQMGFGITVQYGTDTNSVCPKL

SEQ ID NO: 46 - protein, 1273 aa, Artificial Sequence
  wildtype spike of MERS-CoV
VDVGPDSVKSACIEVDIQQTFFDKTWPRPIDVSKADGIIYPQGRTYSNITITYQGLFPYQGDHGDMYVYSAGHATGTTPQKLFVANYSQDVKQFANGFVVRIGAAANSTGTVIISPSTSATIRKIYPAFMLGSSVGNFSDGKMGRFFNHTLVLLPDGCGTLLRAFYCILEPRSGNHCPAGNSYTSFATYHTPATDCSDGNYNRNASLNSFKEYFNLRNCTFMYTYNITEDEILEWFGITQTAQGVHLFSSRYVDLYGGNMFQFATLPVYDTIKYYSIIPHSIRSIQSDRKAWAAFYVYKLQPLTFLLDFSVDGYIRRAIDCGFNDLSQLHCSYESFDVESGVYSVSSFEAKPSGSVVEQAEGVECDFSPLLSGTPPQVYNFKRLVFTNCNYNLTKLLSLFSVNDFTCSQISPAAIASNCYSSLILDYFSYPLSMKSDLSVSSAGPISQFNYKQSFSNPTCLILATVPHNLTTITKPLKYSYINKCSRLLSDDRTEVPQLVNANQYSPCVSIVPSTVWEDGDYYRKQLSPLEGGGWLVASGSTVAMTEQLQMGFGITVQYGTDTNSVCPKLEFANDTKIASQLGNCVEYSLYGVSGRGVFQNCTAVGVRQQRFVYDAYQNLVGYYSDDGNYYCLRACVSVPVSVIYDKETKTHATLFGSVACEHISSTMSQYSRSTRSMLKRRDSTYGPLQTPVGCVLGLVNSSLFVEDCKLPLGQSLCALPDTPSTLTPRSVRSVPGEMRLASIAFNHPIQVDQLNSSYFKLSIPTNFSFGVTQEYIQTTIQKVTVDCKQYVCNGFQKCEQLLREYGQFCSKINQALHGANLRQDDSVRNLFASVKSSQSSPIIPGFGGDFNLTLLEPVSISTGSRSARSAIEDLLFDKVTIADPGYMQGYDDCMQQGPASARDLICAQYVAGYKVLPPLMDVNMEAAYTSSLLGSIAGVGWTAGLSSFAAIPFAQSIFYRLNGVGITQQVLSENQKLIANKFNQALGAMQTGFTTTNEAFQKVQDAVNNNAQALSKLASELSNTFGAISASIGDIIQRLDVLEQDAQIDRLINGRLTTLNAFVAQQLVRSESAALSAQLAKDKVNECVKAQSKRSGFCGQGTHIVSFVVNAPNGLYFMHVGYYPSNHIEVVSAYGLCDAANPTNCIAPVNGYFIKTNNTRIVDEWSYTGSSFYAPEPITSLNTKYVAPQVTYQNISTNLPPPLLGNSTGIDFQDELDEFFKNVSTSIPNFGSLTQINTTLLDLTYEMLSLQQVVKALNESYIDLKELGNYTY

SEQ ID NO: 47 - protein, 1273 aa, Artificial Sequence
  mutant spike of MERS-CoV comprising substitutionVPP: V458C P1060K P1061C
VDVGPDSVKSACIEVDIQQTFFDKTWPRPIDVSKADGIIYPQGRTYSNITITYQGLFPYQGDHGDMYVYSAGHATGTTPQKLFVANYSQDVKQFANGFVVRIGAAANSTGTVIISPSTSATIRKIYPAFMLGSSVGNFSDGKMGRFFNHTLVLLPDGCGTLLRAFYCILEPRSGNHCPAGNSYTSFATYHTPATDCSDGNYNRNASLNSFKEYFNLRNCTFMYTYNITEDEILEWFGITQTAQGVHLFSSRYVDLYGGNMFQFATLPVYDTIKYYSIIPHSIRSIQSDRKAWAAFYVYKLQPLTFLLDFSVDGYIRRAIDCGFNDLSQLHCSYESFDVESGVYSVSSFEAKPSGSVVEQAEGVECDFSPLLSGTPPQVYNFKRLVFTNCNYNLTKLLSLFSVNDFTCSQISPAAIASNCYSSLILDYFSYPLSMKSDLSCSSAGPISQFNYKQSFSNPTCLILATVPHNLTTITKPLKYSYINKCSRLLSDDRTEVPQLVNANQYSPCVSIVPSTVWEDGDYYRKQLSPLEGGGWLVASGSTVAMTEQLQMGFGITVQYGTDTNSVCPKLEFANDTKIASQLGNCVEYSLYGVSGRGVFQNCTAVGVRQQRFVYDAYQNLVGYYSDDGNYYCLRACVSVPVSVIYDKETKTHATLFGSVACEHISSTMSQYSRSTRSMLKRRDSTYGPLQTPVGCVLGLVNSSLFVEDCKLPLGQSLCALPDTPSTLTPASVGSVPGEMRLASIAFNHPIQVDQLNSSYFKLSIPTNFSFGVTQEYIQTTIQKVTVDCKQYVCNGFQKCEQLLREYGQFCSKINQALHGANLRQDDSVRNLFASVKSSQSSPIIPGFGGDFNLTLLEPVSISTGSRSARSAIEDLLFDKVTIADPGYMQGYDDCMQQGPASARDLICAQYVAGYKVLPPLMDVNMEAAYTSSLLGSIAGVGWTAGLSSFAAIPFAQSIFYRLNGVGITQQVLSENQKLIANKFNQALGAMQTGFTTTNEAFQKVQDAVNNNAQALSKLASELSNTFGAISASIGDIIQRLDKCEQDAQIDRLINGRLTTLNAFVAQQLVRSESAALSAQLAKDKVNECVKAQSKRSGFCGQGTHIVSFVVNAPNGLYFMHVGYYPSNHIEVVSAYGLCDAANPTNCIAPVNGYFIKTNNTRIVDEWSYTGSSFYAPEPITSLNTKYVAPQVTYQNISTNLPPPLLGNSTGIDFQDELDEFFKNVSTSIPNFGSLTQINTTLLDLTYEMLSLQQVVKALNESYIDLKELGNYTY

SEQ ID NO: 48 - protein, 1273 aa, Artificial Sequence
  mutant spike of MERS-CoV comprising substitution TS T424C S459C
VDVGPDSVKSACIEVDIQQTFFDKTWPRPIDVSKADGIIYPQGRTYSNITITYQGLFPYQGDHGDMYVYSAGHATGTTPQKLFVANYSQDVKQFANGFVVRIGAAANSTGTVIISPSTSATIRKIYPAFMLGSSVGNFSDGKMGRFFNHTLVLLPDGCGTLLRAFYCILEPRSGNHCPAGNSYTSFATYHTPATDCSDGNYNRNASLNSFKEYFNLRNCTFMYTYNITEDEILEWFGITQTAQGVHLFSSRYVDLYGGNMFQFATLPVYDTIKYYSIIPHSIRSIQSDRKAWAAFYVYKLQPLTFLLDFSVDGYIRRAIDCGFNDLSQLHCSYESFDVESGVYSVSSFEAKPSGSVVEQAEGVECDFSPLLSGTPPQVYNFKRLVFTNCNYNLTKLLSLFSVNDFCCSQISPAAIASNCYSSLILDYFSYPLSMKSDLSVCSAGPISQFNYKQSFSNPTCLILATVPHNLTTITKPLKYSYINKCSRLLSDDRTEVPQLVNANQYSPCVSIVPSTVWEDGDYYRKQLSPLEGGGWLVASGSTVAMTEQLQMGFGITVQYGTDTNSVCPKLEFANDTKIASQLGNCVEYSLYGVSGRGVFQNCTAVGVRQQRFVYDAYQNLVGYYSDDGNYYCLRACVSVPVSVIYDKETKTHATLFGSVACEHISSTMSQYSRSTRSMLKRRDSTYGPLQTPVGCVLGLVNSSLFVEDCKLPLGQSLCALPDTPSTLTPASVGSVPGEMRLASIAFNHPIQVDQLNSSYFKLSIPTNFSFGVTQEYIQTTIQKVTVDCKQYVCNGFQKCEQLLREYGQFCSKINQALHGANLRQDDSVRNLFASVKSSQSSPIIPGFGGDFNLTLLEPVSISTGSRSARSAIEDLLFDKVTIADPGYMQGYDDCMQQGPASARDLICAQYVAGYKVLPPLMDVNMEAAYTSSLLGSIAGVGWTAGLSSFAAIPFAQSIFYRLNGVGITQQVLSENQKLIANKFNQALGAMQTGFTTTNEAFQKVQDAVNNNAQALSKLASELSNTFGAISASIGDIIQRLDPPEQDAQIDRLINGRLTTLNAFVAQQLVRSESAALSAQLAKDKVNECVKAQSKRSGFCGQGTHIVSFVVNAPNGLYFMHVGYYPSNHIEVVSAYGLCDAANPTNCIAPVNGYFIKTNNTRIVDEWSYTGSSFYAPEPITSLNTKYVAPQVTYQNISTNLPPPLLGNSTGIDFQDELDEFFKNVSTSIPNFGSLTQINTTLLDLTYEMLSLQQVVKALNESYIDLKELGNYTY

SEQ ID NO: 49 - protein, 1273 aa, Artificial Sequence
  mutant spike of MERS-CoV comprising substitution F39A
VDVGPDSVKSACIEVDIQQTAFDKTWPRPIDVSKADGIIYPQGRTYSNITITYQGLFPYQGDHGDMYVYSAGHATGTTPQKLFVANYSQDVKQFANGFVVRIGAAANSTGTVIISPSTSATIRKIYPAFMLGSSVGNFSDGKMGRFFNHTLVLLPDGCGTLLRAFYCILEPRSGNHCPAGNSYTSFATYHTPATDCSDGNYNRNASLNSFKEYFNLRNCTFMYTYNITEDEILEWFGITQTAQGVHLFSSRYVDLYGGNMFQFATLPVYDTIKYYSIIPHSIRSIQSDRKAWAAFYVYKLQPLTFLLDFSVDGYIRRAIDCGFNDLSQLHCSYESFDVESGVYSVSSFEAKPSGSVVEQAEGVECDFSPLLSGTPPQVYNFKRLVFTNCNYNLTKLLSLFSVNDFTCSQISPAAIASNCYSSLILDYFSYPLSMKSDLSVSSAGPISQFNYKQSFSNPTCLILATVPHNLTTITKPLKYSYINKCSRLLSDDRTEVPQLVNANQYSPCVSIVPSTVWEDGDYYRKQLSPLEGGGWLVASGSTVAMTEQLQMGFGITVQYGTDTNSVCPKLEFANDTKIASQLGNCVEYSLYGVSGRGVFQNCTAVGVRQQRFVYDAYQNLVGYYSDDGNYYCLRACVSVPVSVIYDKETKTHATLFGSVACEHISSTMSQYSRSTRSMLKRRDSTYGPLQTPVGCVLGLVNSSLFVEDCKLPLGQSLCALPDTPSTLTPASVGSVPGEMRLASIAFNHPIQVDQLNSSYFKLSIPTNFSFGVTQEYIQTTIQKVTVDCKQYVCNGFQKCEQLLREYGQFCSKINQALHGANLRQDDSVRNLFASVKSSQSSPIIPGFGGDFNLTLLEPVSISTGSRSARSAIEDLLFDKVTIADPGYMQGYDDCMQQGPASARDLICAQYVAGYKVLPPLMDVNMEAAYTSSLLGSIAGVGWTAGLSSFAAIPFAQSIFYRLNGVGITQQVLSENQKLIANKFNQALGAMQTGFTTTNEAFQKVQDAVNNNAQALSKLASELSNTFGAISASIGDIIQRLDPPEQDAQIDRLINGRLTTLNAFVAQQLVRSESAALSAQLAKDKVNECVKAQSKRSGFCGQGTHIVSFVVNAPNGLYFMHVGYYPSNHIEVVSAYGLCDAANPTNCIAPVNGYFIKTNNTRIVDEWSYTGSSFYAPEPITSLNTKYVAPQVTYQNISTNLPPPLLGNSTGIDFQDELDEFFKNVSTSIPNFGSLTQINTTLLDLTYEMLSLQQVVKALNESYIDLKELGNYTY

SEQ ID NO: 50 - protein, 1273 aa, Artificial Sequence
  mutant spike of MERS-CoV comprising substitution H91A
VDVGPDSVKSACIEVDIQQTFFDKTWPRPIDVSKADGIIYPQGRTYSNITITYQGLFPYQGDHGDMYVYSAGAATGTTPQKLFVANYSQDVKQFANGFVVRIGAAANSTGTVIISPSTSATIRKIYPAFMLGSSVGNFSDGKMGRFFNHTLVLLPDGCGTLLRAFYCILEPRSGNHCPAGNSYTSFATYHTPATDCSDGNYNRNASLNSFKEYFNLRNCTFMYTYNITEDEILEWFGITQTAQGVHLFSSRYVDLYGGNMFQFATLPVYDTIKYYSIIPHSIRSIQSDRKAWAAFYVYKLQPLTFLLDFSVDGYIRRAIDCGFNDLSQLHCSYESFDVESGVYSVSSFEAKPSGSVVEQAEGVECDFSPLLSGTPPQVYNFKRLVFTNCNYNLTKLLSLFSVNDFTCSQISPAAIASNCYSSLILDYFSYPLSMKSDLSVSSAGPISQFNYKQSFSNPTCLILATVPHNLTTITKPLKYSYINKCSRLLSDDRTEVPQLVNANQYSPCVSIVPSTVWEDGDYYRKQLSPLEGGGWLVASGSTVAMTEQLQMGFGITVQYGTDTNSVCPKLEFANDTKIASQLGNCVEYSLYGVSGRGVFQNCTAVGVRQQRFVYDAYQNLVGYYSDDGNYYCLRACVSVPVSVIYDKETKTHATLFGSVACEHISSTMSQYSRSTRSMLKRRDSTYGPLQTPVGCVLGLVNSSLFVEDCKLPLGQSLCALPDTPSTLTPASVGSVPGEMRLASIAFNHPIQVDQLNSSYFKLSIPTNFSFGVTQEYIQTTIQKVTVDCKQYVCNGFQKCEQLLREYGQFCSKINQALHGANLRQDDSVRNLFASVKSSQSSPIIPGFGGDFNLTLLEPVSISTGSRSARSAIEDLLFDKVTIADPGYMQGYDDCMQQGPASARDLICAQYVAGYKVLPPLMDVNMEAAYTSSLLGSIAGVGWTAGLSSFAAIPFAQSIFYRLNGVGITQQVLSENQKLIANKFNQALGAMQTGFTTTNEAFQKVQDAVNNNAQALSKLASELSNTFGAISASIGDIIQRLDPPEQDAQIDRLINGRLTTLNAFVAQQLVRSESAALSAQLAKDKVNECVKAQSKRSGFCGQGTHIVSFVVNAPNGLYFMHVGYYPSNHIEVVSAYGLCDAANPTNCIAPVNGYFIKTNNTRIVDEWSYTGSSFYAPEPITSLNTKYVAPQVTYQNISTNLPPPLLGNSTGIDFQDELDEFFKNVSTSIPNFGSLTQINTTLLDLTYEMLSLQQVVKALNESYIDLKELGNYTY

SEQ ID NO: 51 - protein, 1273 aa, Artificial Sequence
  mutant spike of MERS-CoV comprising substitution S133A
VDVGPDSVKSACIEVDIQQTFFDKTWPRPIDVSKADGIIYPQGRTYSNITITYQGLFPYQGDHGDMYVYSAGHATGTTPQKLFVANYSQDVKQFANGFVVRIGAAANSTGTVIIAPSTSATIRKIYPAFMLGSSVGNFSDGKMGRFFNHTLVLLPDGCGTLLRAFYCILEPRSGNHCPAGNSYTSFATYHTPATDCSDGNYNRNASLNSFKEYFNLRNCTFMYTYNITEDEILEWFGITQTAQGVHLFSSRYVDLYGGNMFQFATLPVYDTIKYYSIIPHSIRSIQSDRKAWAAFYVYKLQPLTFLLDFSVDGYIRRAIDCGFNDLSQLHCSYESFDVESGVYSVSSFEAKPSGSVVEQAEGVECDFSPLLSGTPPQVYNFKRLVFTNCNYNLTKLLSLFSVNDFTCSQISPAAIASNCYSSLILDYFSYPLSMKSDLSVSSAGPISQFNYKQSFSNPTCLILATVPHNLTTITKPLKYSYINKCSRLLSDDRTEVPQLVNANQYSPCVSIVPSTVWEDGDYYRKQLSPLEGGGWLVASGSTVAMTEQLQMGFGITVQYGTDTNSVCPKLEFANDTKIASQLGNCVEYSLYGVSGRGVFQNCTAVGVRQQRFVYDAYQNLVGYYSDDGNYYCLRACVSVPVSVIYDKETKTHATLFGSVACEHISSTMSQYSRSTRSMLKRRDSTYGPLQTPVGCVLGLVNSSLFVEDCKLPLGQSLCALPDTPSTLTPASVGSVPGEMRLASIAFNHPIQVDQLNSSYFKLSIPTNFSFGVTQEYIQTTIQKVTVDCKQYVCNGFQKCEQLLREYGQFCSKINQALHGANLRQDDSVRNLFASVKSSQSSPIIPGFGGDFNLTLLEPVSISTGSRSARSAIEDLLFDKVTIADPGYMQGYDDCMQQGPASARDLICAQYVAGYKVLPPLMDVNMEAAYTSSLLGSIAGVGWTAGLSSFAAIPFAQSIFYRLNGVGITQQVLSENQKLIANKFNQALGAMQTGFTTTNEAFQKVQDAVNNNAQALSKLASELSNTFGAISASIGDIIQRLDPPEQDAQIDRLINGRLTTLNAFVAQQLVRSESAALSAQLAKDKVNECVKAQSKRSGFCGQGTHIVSFVVNAPNGLYFMHVGYYPSNHIEVVSAYGLCDAANPTNCIAPVNGYFIKTNNTRIVDEWSYTGSSFYAPEPITSLNTKYVAPQVTYQNISTNLPPPLLGNSTGIDFQDELDEFFKNVSTSIPNFGSLTQINTTLLDLTYEMLSLQQVVKALNESYIDLKELGNYTY

SEQ ID NO: 52 - protein, 1273 aa, Artificial Sequence
  mutant spike of MERS-CoV comprising substitution R307A
VDVGPDSVKSACIEVDIQQTFFDKTWPRPIDVSKADGIIYPQGRTYSNITITYQGLFPYQGDHGDMYVYSAGHATGTTPQKLFVANYSQDVKQFANGFVVRIGAAANSTGTVIISPSTSATIRKIYPAFMLGSSVGNFSDGKMGRFFNHTLVLLPDGCGTLLRAFYCILEPRSGNHCPAGNSYTSFATYHTPATDCSDGNYNRNASLNSFKEYFNLRNCTFMYTYNITEDEILEWFGITQTAQGVHLFSSRYVDLYGGNMFQFATLPVYDTIKYYSIIPHSIRSIQSDAKAWAAFYVYKLQPLTFLLDFSVDGYIRRAIDCGFNDLSQLHCSYESFDVESGVYSVSSFEAKPSGSVVEQAEGVECDFSPLLSGTPPQVYNFKRLVFTNCNYNLTKLLSLFSVNDFTCSQISPAAIASNCYSSLILDYFSYPLSMKSDLSVSSAGPISQFNYKQSFSNPTCLILATVPHNLTTITKPLKYSYINKCSRLLSDDRTEVPQLVNANQYSPCVSIVPSTVWEDGDYYRKQLSPLEGGGWLVASGSTVAMTEQLQMGFGITVQYGTDTNSVCPKLEFANDTKIASQLGNCVEYSLYGVSGRGVFQNCTAVGVRQQRFVYDAYQNLVGYYSDDGNYYCLRACVSVPVSVIYDKETKTHATLFGSVACEHISSTMSQYSRSTRSMLKRRDSTYGPLQTPVGCVLGLVNSSLFVEDCKLPLGQSLCALPDTPSTLTPASVGSVPGEMRLASIAFNHPIQVDQLNSSYFKLSIPTNFSFGVTQEYIQTTIQKVTVDCKQYVCNGFQKCEQLLREYGQFCSKINQALHGANLRQDDSVRNLFASVKSSQSSPIIPGFGGDFNLTLLEPVSISTGSRSARSAIEDLLFDKVTIADPGYMQGYDDCMQQGPASARDLICAQYVAGYKVLPPLMDVNMEAAYTSSLLGSIAGVGWTAGLSSFAAIPFAQSIFYRLNGVGITQQVLSENQKLIANKFNQALGAMQTGFTTTNEAFQKVQDAVNNNAQALSKLASELSNTFGAISASIGDIIQRLDPPEQDAQIDRLINGRLTTLNAFVAQQLVRSESAALSAQLAKDKVNECVKAQSKRSGFCGQGTHIVSFVVNAPNGLYFMHVGYYPSNHIEVVSAYGLCDAANPTNCIAPVNGYFIKTNNTRIVDEWSYTGSSFYAPEPITSLNTKYVAPQVTYQNISTNLPPPLLGNSTGIDFQDELDEFFKNVSTSIPNFGSLTQINTTLLDLTYEMLSLQQVVKALNESYIDLKELGNYTY

SEQ ID NO: 53 - protein, 1273 aa, Artificial Sequence
  mutant spike of MERS-CoV comprising substitution TS T424C S459C + F39A
VDVGPDSVKSACIEVDIQQTAFDKTWPRPIDVSKADGIIYPQGRTYSNITITYQGLFPYQGDHGDMYVYSAGHATGTTPQKLFVANYSQDVKQFANGFVVRIGAAANSTGTVIISPSTSATIRKIYPAFMLGSSVGNFSDGKMGRFFNHTLVLLPDGCGTLLRAFYCILEPRSGNHCPAGNSYTSFATYHTPATDCSDGNYNRNASLNSFKEYFNLRNCTFMYTYNITEDEILEWFGITQTAQGVHLFSSRYVDLYGGNMFQFATLPVYDTIKYYSIIPHSIRSIQSDRKAWAAFYVYKLQPLTFLLDFSVDGYIRRAIDCGFNDLSQLHCSYESFDVESGVYSVSSFEAKPSGSVVEQAEGVECDFSPLLSGTPPQVYNFKRLVFTNCNYNLTKLLSLFSVNDFCCSQISPAAIASNCYSSLILDYFSYPLSMKSDLSVCSAGPISQFNYKQSFSNPTCLILATVPHNLTTITKPLKYSYINKCSRLLSDDRTEVPQLVNANQYSPCVSIVPSTVWEDGDYYRKQLSPLEGGGWLVASGSTVAMTEQLQMGFGITVQYGTDTNSVCPKLEFANDTKIASQLGNCVEYSLYGVSGRGVFQNCTAVGVRQQRFVYDAYQNLVGYYSDDGNYYCLRACVSVPVSVIYDKETKTHATLFGSVACEHISSTMSQYSRSTRSMLKRRDSTYGPLQTPVGCVLGLVNSSLFVEDCKLPLGQSLCALPDTPSTLTPASVGSVPGEMRLASIAFNHPIQVDQLNSSYFKLSIPTNFSFGVTQEYIQTTIQKVTVDCKQYVCNGFQKCEQLLREYGQFCSKINQALHGANLRQDDSVRNLFASVKSSQSSPIIPGFGGDFNLTLLEPVSISTGSRSARSAIEDLLFDKVTIADPGYMQGYDDCMQQGPASARDLICAQYVAGYKVLPPLMDVNMEAAYTSSLLGSIAGVGWTAGLSSFAAIPFAQSIFYRLNGVGITQQVLSENQKLIANKFNQALGAMQTGFTTTNEAFQKVQDAVNNNAQALSKLASELSNTFGAISASIGDIIQRLDPPEQDAQIDRLINGRLTTLNAFVAQQLVRSESAALSAQLAKDKVNECVKAQSKRSGFCGQGTHIVSFVVNAPNGLYFMHVGYYPSNHIEVVSAYGLCDAANPTNCIAPVNGYFIKTNNTRIVDEWSYTGSSFYAPEPITSLNTKYVAPQVTYQNISTNLPPPLLGNSTGIDFQDELDEFFKNVSTSIPNFGSLTQINTTLLDLTYEMLSLQQVVKALNESYIDLKELGNYTY

SEQ ID NO: 54 - protein, 1273 aa, Artificial Sequence
  mutant spike of MERS-CoV comprising substitution TS T424C S459C + S133A
VDVGPDSVKSACIEVDIQQTFFDKTWPRPIDVSKADGIIYPQGRTYSNITITYQGLFPYQGDHGDMYVYSAGHATGTTPQKLFVANYSQDVKQFANGFVVRIGAAANSTGTVIIAPSTSATIRKIYPAFMLGSSVGNFSDGKMGRFFNHTLVLLPDGCGTLLRAFYCILEPRSGNHCPAGNSYTSFATYHTPATDCSDGNYNRNASLNSFKEYFNLRNCTFMYTYNITEDEILEWFGITQTAQGVHLFSSRYVDLYGGNMFQFATLPVYDTIKYYSIIPHSIRSIQSDRKAWAAFYVYKLQPLTFLLDFSVDGYIRRAIDCGFNDLSQLHCSYESFDVESGVYSVSSFEAKPSGSVVEQAEGVECDFSPLLSGTPPQVYNFKRLVFTNCNYNLTKLLSLFSVNDFCCSQISPAAIASNCYSSLILDYFSYPLSMKSDLSVCSAGPISQFNYKQSFSNPTCLILATVPHNLTTITKPLKYSYINKCSRLLSDDRTEVPQLVNANQYSPCVSIVPSTVWEDGDYYRKQLSPLEGGGWLVASGSTVAMTEQLQMGFGITVQYGTDTNSVCPKLEFANDTKIASQLGNCVEYSLYGVSGRGVFQNCTAVGVRQQRFVYDAYQNLVGYYSDDGNYYCLRACVSVPVSVIYDKETKTHATLFGSVACEHISSTMSQYSRSTRSMLKRRDSTYGPLQTPVGCVLGLVNSSLFVEDCKLPLGQSLCALPDTPSTLTPASVGSVPGEMRLASIAFNHPIQVDQLNSSYFKLSIPTNFSFGVTQEYIQTTIQKVTVDCKQYVCNGFQKCEQLLREYGQFCSKINQALHGANLRQDDSVRNLFASVKSSQSSPIIPGFGGDFNLTLLEPVSISTGSRSARSAIEDLLFDKVTIADPGYMQGYDDCMQQGPASARDLICAQYVAGYKVLPPLMDVNMEAAYTSSLLGSIAGVGWTAGLSSFAAIPFAQSIFYRLNGVGITQQVLSENQKLIANKFNQALGAMQTGFTTTNEAFQKVQDAVNNNAQALSKLASELSNTFGAISASIGDIIQRLDPPEQDAQIDRLINGRLTTLNAFVAQQLVRSESAALSAQLAKDKVNECVKAQSKRSGFCGQGTHIVSFVVNAPNGLYFMHVGYYPSNHIEVVSAYGLCDAANPTNCIAPVNGYFIKTNNTRIVDEWSYTGSSFYAPEPITSLNTKYVAPQVTYQNISTNLPPPLLGNSTGIDFQDELDEFFKNVSTSIPNFGSLTQINTTLLDLTYEMLSLQQVVKALNESYIDLKELGNYTY

SEQ ID NO: 55 - protein, 1273 aa, Artificial Sequence
  mutant spike of MERS-CoV comprising substitution TS T424C S459C + R307A
VDVGPDSVKSACIEVDIQQTFFDKTWPRPIDVSKADGIIYPQGRTYSNITITYQGLFPYQGDHGDMYVYSAGHATGTTPQKLFVANYSQDVKQFANGFVVRIGAAANSTGTVIISPSTSATIRKIYPAFMLGSSVGNFSDGKMGRFFNHTLVLLPDGCGTLLRAFYCILEPRSGNHCPAGNSYTSFATYHTPATDCSDGNYNRNASLNSFKEYFNLRNCTFMYTYNITEDEILEWFGITQTAQGVHLFSSRYVDLYGGNMFQFATLPVYDTIKYYSIIPHSIRSIQSDAKAWAAFYVYKLQPLTFLLDFSVDGYIRRAIDCGFNDLSQLHCSYESFDVESGVYSVSSFEAKPSGSVVEQAEGVECDFSPLLSGTPPQVYNFKRLVFTNCNYNLTKLLSLFSVNDFCCSQISPAAIASNCYSSLILDYFSYPLSMKSDLSVCSAGPISQFNYKQSFSNPTCLILATVPHNLTTITKPLKYSYINKCSRLLSDDRTEVPQLVNANQYSPCVSIVPSTVWEDGDYYRKQLSPLEGGGWLVASGSTVAMTEQLQMGFGITVQYGTDTNSVCPKLEFANDTKIASQLGNCVEYSLYGVSGRGVFQNCTAVGVRQQRFVYDAYQNLVGYYSDDGNYYCLRACVSVPVSVIYDKETKTHATLFGSVACEHISSTMSQYSRSTRSMLKRRDSTYGPLQTPVGCVLGLVNSSLFVEDCKLPLGQSLCALPDTPSTLTPASVGSVPGEMRLASIAFNHPIQVDQLNSSYFKLSIPTNFSFGVTQEYIQTTIQKVTVDCKQYVCNGFQKCEQLLREYGQFCSKINQALHGANLRQDDSVRNLFASVKSSQSSPIIPGFGGDFNLTLLEPVSISTGSRSARSAIEDLLFDKVTIADPGYMQGYDDCMQQGPASARDLICAQYVAGYKVLPPLMDVNMEAAYTSSLLGSIAGVGWTAGLSSFAAIPFAQSIFYRLNGVGITQQVLSENQKLIANKFNQALGAMQTGFTTTNEAFQKVQDAVNNNAQALSKLASELSNTFGAISASIGDIIQRLDPPEQDAQIDRLINGRLTTLNAFVAQQLVRSESAALSAQLAKDKVNECVKAQSKRSGFCGQGTHIVSFVVNAPNGLYFMHVGYYPSNHIEVVSAYGLCDAANPTNCIAPVNGYFIKTNNTRIVDEWSYTGSSFYAPEPITSLNTKYVAPQVTYQNISTNLPPPLLGNSTGIDFQDELDEFFKNVSTSIPNFGSLTQINTTLLDLTYEMLSLQQVVKALNESYIDLKELGNYTY

SEQ ID NO: 56 - protein, 1273 aa, Artificial Sequence
  mutant spike of MERS-CoV comprising substitution TS T424C S459C + H91A
VDVGPDSVKSACIEVDIQQTFFDKTWPRPIDVSKADGIIYPQGRTYSNITITYQGLFPYQGDHGDMYVYSAGAATGTTPQKLFVANYSQDVKQFANGFVVRIGAAANSTGTVIISPSTSATIRKIYPAFMLGSSVGNFSDGKMGRFFNHTLVLLPDGCGTLLRAFYCILEPRSGNHCPAGNSYTSFATYHTPATDCSDGNYNRNASLNSFKEYFNLRNCTFMYTYNITEDEILEWFGITQTAQGVHLFSSRYVDLYGGNMFQFATLPVYDTIKYYSIIPHSIRSIQSDRKAWAAFYVYKLQPLTFLLDFSVDGYIRRAIDCGFNDLSQLHCSYESFDVESGVYSVSSFEAKPSGSVVEQAEGVECDFSPLLSGTPPQVYNFKRLVFTNCNYNLTKLLSLFSVNDFCCSQISPAAIASNCYSSLILDYFSYPLSMKSDLSVCSAGPISQFNYKQSFSNPTCLILATVPHNLTTITKPLKYSYINKCSRLLSDDRTEVPQLVNANQYSPCVSIVPSTVWEDGDYYRKQLSPLEGGGWLVASGSTVAMTEQLQMGFGITVQYGTDTNSVCPKLEFANDTKIASQLGNCVEYSLYGVSGRGVFQNCTAVGVRQQRFVYDAYQNLVGYYSDDGNYYCLRACVSVPVSVIYDKETKTHATLFGSVACEHISSTMSQYSRSTRSMLKRRDSTYGPLQTPVGCVLGLVNSSLFVEDCKLPLGQSLCALPDTPSTLTPASVGSVPGEMRLASIAFNHPIQVDQLNSSYFKLSIPTNFSFGVTQEYIQTTIQKVTVDCKQYVCNGFQKCEQLLREYGQFCSKINQALHGANLRQDDSVRNLFASVKSSQSSPIIPGFGGDFNLTLLEPVSISTGSRSARSAIEDLLFDKVTIADPGYMQGYDDCMQQGPASARDLICAQYVAGYKVLPPLMDVNMEAAYTSSLLGSIAGVGWTAGLSSFAAIPFAQSIFYRLNGVGITQQVLSENQKLIANKFNQALGAMQTGFTTTNEAFQKVQDAVNNNAQALSKLASELSNTFGAISASIGDIIQRLDPPEQDAQIDRLINGRLTTLNAFVAQQLVRSESAALSAQLAKDKVNECVKAQSKRSGFCGQGTHIVSFVVNAPNGLYFMHVGYYPSNHIEVVSAYGLCDAANPTNCIAPVNGYFIKTNNTRIVDEWSYTGSSFYAPEPITSLNTKYVAPQVTYQNISTNLPPPLLGNSTGIDFQDELDEFFKNVSTSIPNFGSLTQINTTLLDLTYEMLSLQQVVKALNESYIDLKELGNYTY

SEQ ID NO: 57 - protein, 1273 aa, Artificial Sequence
  mutant spike of MERS-CoV comprising substitution S460W
VDVGPDSVKSACIEVDIQQTFFDKTWPRPIDVSKADGIIYPQGRTYSNITITYQGLFPYQGDHGDMYVYSAGHATGTTPQKLFVANYSQDVKQFANGFVVRIGAAANSTGTVIISPSTSATIRKIYPAFMLGSSVGNFSDGKMGRFFNHTLVLLPDGCGTLLRAFYCILEPRSGNHCPAGNSYTSFATYHTPATDCSDGNYNRNASLNSFKEYFNLRNCTFMYTYNITEDEILEWFGITQTAQGVHLFSSRYVDLYGGNMFQFATLPVYDTIKYYSIIPHSIRSIQSDRKAWAAFYVYKLQPLTFLLDFSVDGYIRRAIDCGFNDLSQLHCSYESFDVESGVYSVSSFEAKPSGSVVEQAEGVECDFSPLLSGTPPQVYNFKRLVFTNCNYNLTKLLSLFSVNDFTCSQISPAAIASNCYSSLILDYFSYPLSMKSDLSVSWAGPISQFNYKQSFSNPTCLILATVPHNLTTITKPLKYSYINKCSRLLSDDRTEVPQLVNANQYSPCVSIVPSTVWEDGDYYRKQLSPLEGGGWLVASGSTVAMTEQLQMGFGITVQYGTDTNSVCPKLEFANDTKIASQLGNCVEYSLYGVSGRGVFQNCTAVGVRQQRFVYDAYQNLVGYYSDDGNYYCLRACVSVPVSVIYDKETKTHATLFGSVACEHISSTMSQYSRSTRSMLKRRDSTYGPLQTPVGCVLGLVNSSLFVEDCKLPLGQSLCALPDTPSTLTPASVGSVPGEMRLASIAFNHPIQVDQLNSSYFKLSIPTNFSFGVTQEYIQTTIQKVTVDCKQYVCNGFQKCEQLLREYGQFCSKINQALHGANLRQDDSVRNLFASVKSSQSSPIIPGFGGDFNLTLLEPVSISTGSRSARSAIEDLLFDKVTIADPGYMQGYDDCMQQGPASARDLICAQYVAGYKVLPPLMDVNMEAAYTSSLLGSIAGVGWTAGLSSFAAIPFAQSIFYRLNGVGITQQVLSENQKLIANKFNQALGAMQTGFTTTNEAFQKVQDAVNNNAQALSKLASELSNTFGAISASIGDIIQRLDPPEQDAQIDRLINGRLTTLNAFVAQQLVRSESAALSAQLAKDKVNECVKAQSKRSGFCGQGTHIVSFVVNAPNGLYFMHVGYYPSNHIEVVSAYGLCDAANPTNCIAPVNGYFIKTNNTRIVDEWSYTGSSFYAPEPITSLNTKYVAPQVTYQNISTNLPPPLLGNSTGIDFQDELDEFFKNVSTSIPNFGSLTQINTTLLDLTYEMLSLQQVVKALNESYIDLKELGNYTY

SEQ ID NO: 58 - protein, 1273 aa, Artificial Sequence
  mutant spike of MERS-CoV comprising substitution G462R
VDVGPDSVKSACIEVDIQQTFFDKTWPRPIDVSKADGIIYPQGRTYSNITITYQGLFPYQGDHGDMYVYSAGHATGTTPQKLFVANYSQDVKQFANGFVVRIGAAANSTGTVIISPSTSATIRKIYPAFMLGSSVGNFSDGKMGRFFNHTLVLLPDGCGTLLRAFYCILEPRSGNHCPAGNSYTSFATYHTPATDCSDGNYNRNASLNSFKEYFNLRNCTFMYTYNITEDEILEWFGITQTAQGVHLFSSRYVDLYGGNMFQFATLPVYDTIKYYSIIPHSIRSIQSDRKAWAAFYVYKLQPLTFLLDFSVDGYIRRAIDCGFNDLSQLHCSYESFDVESGVYSVSSFEAKPSGSVVEQAEGVECDFSPLLSGTPPQVYNFKRLVFTNCNYNLTKLLSLFSVNDFTCSQISPAAIASNCYSSLILDYFSYPLSMKSDLSVSSARPISQFNYKQSFSNPTCLILATVPHNLTTITKPLKYSYINKCSRLLSDDRTEVPQLVNANQYSPCVSIVPSTVWEDGDYYRKQLSPLEGGGWLVASGSTVAMTEQLQMGFGITVQYGTDTNSVCPKLEFANDTKIASQLGNCVEYSLYGVSGRGVFQNCTAVGVRQQRFVYDAYQNLVGYYSDDGNYYCLRACVSVPVSVIYDKETKTHATLFGSVACEHISSTMSQYSRSTRSMLKRRDSTYGPLQTPVGCVLGLVNSSLFVEDCKLPLGQSLCALPDTPSTLTPASVGSVPGEMRLASIAFNHPIQVDQLNSSYFKLSIPTNFSFGVTQEYIQTTIQKVTVDCKQYVCNGFQKCEQLLREYGQFCSKINQALHGANLRQDDSVRNLFASVKSSQSSPIIPGFGGDFNLTLLEPVSISTGSRSARSAIEDLLFDKVTIADPGYMQGYDDCMQQGPASARDLICAQYVAGYKVLPPLMDVNMEAAYTSSLLGSIAGVGWTAGLSSFAAIPFAQSIFYRLNGVGITQQVLSENQKLIANKFNQALGAMQTGFTTTNEAFQKVQDAVNNNAQALSKLASELSNTFGAISASIGDIIQRLDPPEQDAQIDRLINGRLTTLNAFVAQQLVRSESAALSAQLAKDKVNECVKAQSKRSGFCGQGTHIVSFVVNAPNGLYFMHVGYYPSNHIEVVSAYGLCDAANPTNCIAPVNGYFIKTNNTRIVDEWSYTGSSFYAPEPITSLNTKYVAPQVTYQNISTNLPPPLLGNSTGIDFQDELDEFFKNVSTSIPNFGSLTQINTTLLDLTYEMLSLQQVVKALNESYIDLKELGNYTY

SEQ ID NO: 59 - protein, 1273 aa, Artificial Sequence
  mutant spike of MERS-CoV comprising substitution G462Q
VDVGPDSVKSACIEVDIQQTFFDKTWPRPIDVSKADGIIYPQGRTYSNITITYQGLFPYQGDHGDMYVYSAGHATGTTPQKLFVANYSQDVKQFANGFVVRIGAAANSTGTVIISPSTSATIRKIYPAFMLGSSVGNFSDGKMGRFFNHTLVLLPDGCGTLLRAFYCILEPRSGNHCPAGNSYTSFATYHTPATDCSDGNYNRNASLNSFKEYFNLRNCTFMYTYNITEDEILEWFGITQTAQGVHLFSSRYVDLYGGNMFQFATLPVYDTIKYYSIIPHSIRSIQSDRKAWAAFYVYKLQPLTFLLDFSVDGYIRRAIDCGFNDLSQLHCSYESFDVESGVYSVSSFEAKPSGSVVEQAEGVECDFSPLLSGTPPQVYNFKRLVFTNCNYNLTKLLSLFSVNDFTCSQISPAAIASNCYSSLILDYFSYPLSMKSDLSVSSAQPISQFNYKQSFSNPTCLILATVPHNLTTITKPLKYSYINKCSRLLSDDRTEVPQLVNANQYSPCVSIVPSTVWEDGDYYRKQLSPLEGGGWLVASGSTVAMTEQLQMGFGITVQYGTDTNSVCPKLEFANDTKIASQLGNCVEYSLYGVSGRGVFQNCTAVGVRQQRFVYDAYQNLVGYYSDDGNYYCLRACVSVPVSVIYDKETKTHATLFGSVACEHISSTMSQYSRSTRSMLKRRDSTYGPLQTPVGCVLGLVNSSLFVEDCKLPLGQSLCALPDTPSTLTPASVGSVPGEMRLASIAFNHPIQVDQLNSSYFKLSIPTNFSFGVTQEYIQTTIQKVTVDCKQYVCNGFQKCEQLLREYGQFCSKINQALHGANLRQDDSVRNLFASVKSSQSSPIIPGFGGDFNLTLLEPVSISTGSRSARSAIEDLLFDKVTIADPGYMQGYDDCMQQGPASARDLICAQYVAGYKVLPPLMDVNMEAAYTSSLLGSIAGVGWTAGLSSFAAIPFAQSIFYRLNGVGITQQVLSENQKLIANKFNQALGAMQTGFTTTNEAFQKVQDAVNNNAQALSKLASELSNTFGAISASIGDIIQRLDPPEQDAQIDRLINGRLTTLNAFVAQQLVRSESAALSAQLAKDKVNECVKAQSKRSGFCGQGTHIVSFVVNAPNGLYFMHVGYYPSNHIEVVSAYGLCDAANPTNCIAPVNGYFIKTNNTRIVDEWSYTGSSFYAPEPITSLNTKYVAPQVTYQNISTNLPPPLLGNSTGIDFQDELDEFFKNVSTSIPNFGSLTQINTTLLDLTYEMLSLQQVVKALNESYIDLKELGNYTY

SEQ ID NO: 60 - protein, 1273 aa, Artificial Sequence
  mutant spike of MERS-CoV comprising substitution G462L
VDVGPDSVKSACIEVDIQQTFFDKTWPRPIDVSKADGIIYPQGRTYSNITITYQGLFPYQGDHGDMYVYSAGHATGTTPQKLFVANYSQDVKQFANGFVVRIGAAANSTGTVIISPSTSATIRKIYPAFMLGSSVGNFSDGKMGRFFNHTLVLLPDGCGTLLRAFYCILEPRSGNHCPAGNSYTSFATYHTPATDCSDGNYNRNASLNSFKEYFNLRNCTFMYTYNITEDEILEWFGITQTAQGVHLFSSRYVDLYGGNMFQFATLPVYDTIKYYSIIPHSIRSIQSDRKAWAAFYVYKLQPLTFLLDFSVDGYIRRAIDCGFNDLSQLHCSYESFDVESGVYSVSSFEAKPSGSVVEQAEGVECDFSPLLSGTPPQVYNFKRLVFTNCNYNLTKLLSLFSVNDFTCSQISPAAIASNCYSSLILDYFSYPLSMKSDLSVSSALPISQFNYKQSFSNPTCLILATVPHNLTTITKPLKYSYINKCSRLLSDDRTEVPQLVNANQYSPCVSIVPSTVWEDGDYYRKQLSPLEGGGWLVASGSTVAMTEQLQMGFGITVQYGTDTNSVCPKLEFANDTKIASQLGNCVEYSLYGVSGRGVFQNCTAVGVRQQRFVYDAYQNLVGYYSDDGNYYCLRACVSVPVSVIYDKETKTHATLFGSVACEHISSTMSQYSRSTRSMLKRRDSTYGPLQTPVGCVLGLVNSSLFVEDCKLPLGQSLCALPDTPSTLTPASVGSVPGEMRLASIAFNHPIQVDQLNSSYFKLSIPTNFSFGVTQEYIQTTIQKVTVDCKQYVCNGFQKCEQLLREYGQFCSKINQALHGANLRQDDSVRNLFASVKSSQSSPIIPGFGGDFNLTLLEPVSISTGSRSARSAIEDLLFDKVTIADPGYMQGYDDCMQQGPASARDLICAQYVAGYKVLPPLMDVNMEAAYTSSLLGSIAGVGWTAGLSSFAAIPFAQSIFYRLNGVGITQQVLSENQKLIANKFNQALGAMQTGFTTTNEAFQKVQDAVNNNAQALSKLASELSNTFGAISASIGDIIQRLDPPEQDAQIDRLINGRLTTLNAFVAQQLVRSESAALSAQLAKDKVNECVKAQSKRSGFCGQGTHIVSFVVNAPNGLYFMHVGYYPSNHIEVVSAYGLCDAANPTNCIAPVNGYFIKTNNTRIVDEWSYTGSSFYAPEPITSLNTKYVAPQVTYQNISTNLPPPLLGNSTGIDFQDELDEFFKNVSTSIPNFGSLTQINTTLLDLTYEMLSLQQVVKALNESYIDLKELGNYTY

SEQ ID NO: 61 - protein, 1273 aa, Artificial Sequence
  mutant spike of MERS-CoV comprising substitution G462W
VDVGPDSVKSACIEVDIQQTFFDKTWPRPIDVSKADGIIYPQGRTYSNITITYQGLFPYQGDHGDMYVYSAGHATGTTPQKLFVANYSQDVKQFANGFVVRIGAAANSTGTVIISPSTSATIRKIYPAFMLGSSVGNFSDGKMGRFFNHTLVLLPDGCGTLLRAFYCILEPRSGNHCPAGNSYTSFATYHTPATDCSDGNYNRNASLNSFKEYFNLRNCTFMYTYNITEDEILEWFGITQTAQGVHLFSSRYVDLYGGNMFQFATLPVYDTIKYYSIIPHSIRSIQSDRKAWAAFYVYKLQPLTFLLDFSVDGYIRRAIDCGFNDLSQLHCSYESFDVESGVYSVSSFEAKPSGSVVEQAEGVECDFSPLLSGTPPQVYNFKRLVFTNCNYNLTKLLSLFSVNDFTCSQISPAAIASNCYSSLILDYFSYPLSMKSDLSVSSAWPISQFNYKQSFSNPTCLILATVPHNLTTITKPLKYSYINKCSRLLSDDRTEVPQLVNANQYSPCVSIVPSTVWEDGDYYRKQLSPLEGGGWLVASGSTVAMTEQLQMGFGITVQYGTDTNSVCPKLEFANDTKIASQLGNCVEYSLYGVSGRGVFQNCTAVGVRQQRFVYDAYQNLVGYYSDDGNYYCLRACVSVPVSVIYDKETKTHATLFGSVACEHISSTMSQYSRSTRSMLKRRDSTYGPLQTPVGCVLGLVNSSLFVEDCKLPLGQSLCALPDTPSTLTPASVGSVPGEMRLASIAFNHPIQVDQLNSSYFKLSIPTNFSFGVTQEYIQTTIQKVTVDCKQYVCNGFQKCEQLLREYGQFCSKINQALHGANLRQDDSVRNLFASVKSSQSSPIIPGFGGDFNLTLLEPVSISTGSRSARSAIEDLLFDKVTIADPGYMQGYDDCMQQGPASARDLICAQYVAGYKVLPPLMDVNMEAAYTSSLLGSIAGVGWTAGLSSFAAIPFAQSIFYRLNGVGITQQVLSENQKLIANKFNQALGAMQTGFTTTNEAFQKVQDAVNNNAQALSKLASELSNTFGAISASIGDIIQRLDPPEQDAQIDRLINGRLTTLNAFVAQQLVRSESAALSAQLAKDKVNECVKAQSKRSGFCGQGTHIVSFVVNAPNGLYFMHVGYYPSNHIEVVSAYGLCDAANPTNCIAPVNGYFIKTNNTRIVDEWSYTGSSFYAPEPITSLNTKYVAPQVTYQNISTNLPPPLLGNSTGIDFQDELDEFFKNVSTSIPNFGSLTQINTTLLDLTYEMLSLQQVVKALNESYIDLKELGNYTY

SEQ ID NO: 62 - protein, 1273 aa, Artificial Sequence
  mutant spike of MERS-CoV comprising substitution G462Y
VDVGPDSVKSACIEVDIQQTFFDKTWPRPIDVSKADGIIYPQGRTYSNITITYQGLFPYQGDHGDMYVYSAGHATGTTPQKLFVANYSQDVKQFANGFVVRIGAAANSTGTVIISPSTSATIRKIYPAFMLGSSVGNFSDGKMGRFFNHTLVLLPDGCGTLLRAFYCILEPRSGNHCPAGNSYTSFATYHTPATDCSDGNYNRNASLNSFKEYFNLRNCTFMYTYNITEDEILEWFGITQTAQGVHLFSSRYVDLYGGNMFQFATLPVYDTIKYYSIIPHSIRSIQSDRKAWAAFYVYKLQPLTFLLDFSVDGYIRRAIDCGFNDLSQLHCSYESFDVESGVYSVSSFEAKPSGSVVEQAEGVECDFSPLLSGTPPQVYNFKRLVFTNCNYNLTKLLSLFSVNDFTCSQISPAAIASNCYSSLILDYFSYPLSMKSDLSVSSAYPISQFNYKQSFSNPTCLILATVPHNLTTITKPLKYSYINKCSRLLSDDRTEVPQLVNANQYSPCVSIVPSTVWEDGDYYRKQLSPLEGGGWLVASGSTVAMTEQLQMGFGITVQYGTDTNSVCPKLEFANDTKIASQLGNCVEYSLYGVSGRGVFQNCTAVGVRQQRFVYDAYQNLVGYYSDDGNYYCLRACVSVPVSVIYDKETKTHATLFGSVACEHISSTMSQYSRSTRSMLKRRDSTYGPLQTPVGCVLGLVNSSLFVEDCKLPLGQSLCALPDTPSTLTPASVGSVPGEMRLASIAFNHPIQVDQLNSSYFKLSIPTNFSFGVTQEYIQTTIQKVTVDCKQYVCNGFQKCEQLLREYGQFCSKINQALHGANLRQDDSVRNLFASVKSSQSSPIIPGFGGDFNLTLLEPVSISTGSRSARSAIEDLLFDKVTIADPGYMQGYDDCMQQGPASARDLICAQYVAGYKVLPPLMDVNMEAAYTSSLLGSIAGVGWTAGLSSFAAIPFAQSIFYRLNGVGITQQVLSENQKLIANKFNQALGAMQTGFTTTNEAFQKVQDAVNNNAQALSKLASELSNTFGAISASIGDIIQRLDPPEQDAQIDRLINGRLTTLNAFVAQQLVRSESAALSAQLAKDKVNECVKAQSKRSGFCGQGTHIVSFVVNAPNGLYFMHVGYYPSNHIEVVSAYGLCDAANPTNCIAPVNGYFIKTNNTRIVDEWSYTGSSFYAPEPITSLNTKYVAPQVTYQNISTNLPPPLLGNSTGIDFQDELDEFFKNVSTSIPNFGSLTQINTTLLDLTYEMLSLQQVVKALNESYIDLKELGNYTY

SEQ ID NO: 63 - protein, 1273 aa, Artificial Sequence
  mutant spike of MERS-CoV comprising substitution G462F
VDVGPDSVKSACIEVDIQQTFFDKTWPRPIDVSKADGIIYPQGRTYSNITITYQGLFPYQGDHGDMYVYSAGHATGTTPQKLFVANYSQDVKQFANGFVVRIGAAANSTGTVIISPSTSATIRKIYPAFMLGSSVGNFSDGKMGRFFNHTLVLLPDGCGTLLRAFYCILEPRSGNHCPAGNSYTSFATYHTPATDCSDGNYNRNASLNSFKEYFNLRNCTFMYTYNITEDEILEWFGITQTAQGVHLFSSRYVDLYGGNMFQFATLPVYDTIKYYSIIPHSIRSIQSDRKAWAAFYVYKLQPLTFLLDFSVDGYIRRAIDCGFNDLSQLHCSYESFDVESGVYSVSSFEAKPSGSVVEQAEGVECDFSPLLSGTPPQVYNFKRLVFTNCNYNLTKLLSLFSVNDFTCSQISPAAIASNCYSSLILDYFSYPLSMKSDLSVSSAFPISQFNYKQSFSNPTCLILATVPHNLTTITKPLKYSYINKCSRLLSDDRTEVPQLVNANQYSPCVSIVPSTVWEDGDYYRKQLSPLEGGGWLVASGSTVAMTEQLQMGFGITVQYGTDTNSVCPKLEFANDTKIASQLGNCVEYSLYGVSGRGVFQNCTAVGVRQQRFVYDAYQNLVGYYSDDGNYYCLRACVSVPVSVIYDKETKTHATLFGSVACEHISSTMSQYSRSTRSMLKRRDSTYGPLQTPVGCVLGLVNSSLFVEDCKLPLGQSLCALPDTPSTLTPASVGSVPGEMRLASIAFNHPIQVDQLNSSYFKLSIPTNFSFGVTQEYIQTTIQKVTVDCKQYVCNGFQKCEQLLREYGQFCSKINQALHGANLRQDDSVRNLFASVKSSQSSPIIPGFGGDFNLTLLEPVSISTGSRSARSAIEDLLFDKVTIADPGYMQGYDDCMQQGPASARDLICAQYVAGYKVLPPLMDVNMEAAYTSSLLGSIAGVGWTAGLSSFAAIPFAQSIFYRLNGVGITQQVLSENQKLIANKFNQALGAMQTGFTTTNEAFQKVQDAVNNNAQALSKLASELSNTFGAISASIGDIIQRLDPPEQDAQIDRLINGRLTTLNAFVAQQLVRSESAALSAQLAKDKVNECVKAQSKRSGFCGQGTHIVSFVVNAPNGLYFMHVGYYPSNHIEVVSAYGLCDAANPTNCIAPVNGYFIKTNNTRIVDEWSYTGSSFYAPEPITSLNTKYVAPQVTYQNISTNLPPPLLGNSTGIDFQDELDEFFKNVSTSIPNFGSLTQINTTLLDLTYEMLSLQQVVKALNESYIDLKELGNYTY

SEQ ID NO: 64 - protein, 1273 aa, Artificial Sequence
  mutant spike of MERS-CoV comprising substitution S498W
VDVGPDSVKSACIEVDIQQTFFDKTWPRPIDVSKADGIIYPQGRTYSNITITYQGLFPYQGDHGDMYVYSAGHATGTTPQKLFVANYSQDVKQFANGFVVRIGAAANSTGTVIISPSTSATIRKIYPAFMLGSSVGNFSDGKMGRFFNHTLVLLPDGCGTLLRAFYCILEPRSGNHCPAGNSYTSFATYHTPATDCSDGNYNRNASLNSFKEYFNLRNCTFMYTYNITEDEILEWFGITQTAQGVHLFSSRYVDLYGGNMFQFATLPVYDTIKYYSIIPHSIRSIQSDRKAWAAFYVYKLQPLTFLLDFSVDGYIRRAIDCGFNDLSQLHCSYESFDVESGVYSVSSFEAKPSGSVVEQAEGVECDFSPLLSGTPPQVYNFKRLVFTNCNYNLTKLLSLFSVNDFTCSQISPAAIASNCYSSLILDYFSYPLSMKSDLSVSSAGPISQFNYKQSFSNPTCLILATVPHNLTTITKPLKYWYINKCSRLLSDDRTEVPQLVNANQYSPCVSIVPSTVWEDGDYYRKQLSPLEGGGWLVASGSTVAMTEQLQMGFGITVQYGTDTNSVCPKLEFANDTKIASQLGNCVEYSLYGVSGRGVFQNCTAVGVRQQRFVYDAYQNLVGYYSDDGNYYCLRACVSVPVSVIYDKETKTHATLFGSVACEHISSTMSQYSRSTRSMLKRRDSTYGPLQTPVGCVLGLVNSSLFVEDCKLPLGQSLCALPDTPSTLTPASVGSVPGEMRLASIAFNHPIQVDQLNSSYFKLSIPTNFSFGVTQEYIQTTIQKVTVDCKQYVCNGFQKCEQLLREYGQFCSKINQALHGANLRQDDSVRNLFASVKSSQSSPIIPGFGGDFNLTLLEPVSISTGSRSARSAIEDLLFDKVTIADPGYMQGYDDCMQQGPASARDLICAQYVAGYKVLPPLMDVNMEAAYTSSLLGSIAGVGWTAGLSSFAAIPFAQSIFYRLNGVGITQQVLSENQKLIANKFNQALGAMQTGFTTTNEAFQKVQDAVNNNAQALSKLASELSNTFGAISASIGDIIQRLDPPEQDAQIDRLINGRLTTLNAFVAQQLVRSESAALSAQLAKDKVNECVKAQSKRSGFCGQGTHIVSFVVNAPNGLYFMHVGYYPSNHIEVVSAYGLCDAANPTNCIAPVNGYFIKTNNTRIVDEWSYTGSSFYAPEPITSLNTKYVAPQVTYQNISTNLPPPLLGNSTGIDFQDELDEFFKNVSTSIPNFGSLTQINTTLLDLTYEMLSLQQVVKALNESYIDLKELGNYTY

SEQ ID NO: 65 - protein, 1273 aa, Artificial Sequence
  mutant spike of MERS-CoV comprising substitution S504W
VDVGPDSVKSACIEVDIQQTFFDKTWPRPIDVSKADGIIYPQGRTYSNITITYQGLFPYQGDHGDMYVYSAGHATGTTPQKLFVANYSQDVKQFANGFVVRIGAAANSTGTVIISPSTSATIRKIYPAFMLGSSVGNFSDGKMGRFFNHTLVLLPDGCGTLLRAFYCILEPRSGNHCPAGNSYTSFATYHTPATDCSDGNYNRNASLNSFKEYFNLRNCTFMYTYNITEDEILEWFGITQTAQGVHLFSSRYVDLYGGNMFQFATLPVYDTIKYYSIIPHSIRSIQSDRKAWAAFYVYKLQPLTFLLDFSVDGYIRRAIDCGFNDLSQLHCSYESFDVESGVYSVSSFEAKPSGSVVEQAEGVECDFSPLLSGTPPQVYNFKRLVFTNCNYNLTKLLSLFSVNDFTCSQISPAAIASNCYSSLILDYFSYPLSMKSDLSVSSAGPISQFNYKQSFSNPTCLILATVPHNLTTITKPLKYSYINKCWRLLSDDRTEVPQLVNANQYSPCVSIVPSTVWEDGDYYRKQLSPLEGGGWLVASGSTVAMTEQLQMGFGITVQYGTDTNSVCPKLEFANDTKIASQLGNCVEYSLYGVSGRGVFQNCTAVGVRQQRFVYDAYQNLVGYYSDDGNYYCLRACVSVPVSVIYDKETKTHATLFGSVACEHISSTMSQYSRSTRSMLKRRDSTYGPLQTPVGCVLGLVNSSLFVEDCKLPLGQSLCALPDTPSTLTPASVGSVPGEMRLASIAFNHPIQVDQLNSSYFKLSIPTNFSFGVTQEYIQTTIQKVTVDCKQYVCNGFQKCEQLLREYGQFCSKINQALHGANLRQDDSVRNLFASVKSSQSSPIIPGFGGDFNLTLLEPVSISTGSRSARSAIEDLLFDKVTIADPGYMQGYDDCMQQGPASARDLICAQYVAGYKVLPPLMDVNMEAAYTSSLLGSIAGVGWTAGLSSFAAIPFAQSIFYRLNGVGITQQVLSENQKLIANKFNQALGAMQTGFTTTNEAFQKVQDAVNNNAQALSKLASELSNTFGAISASIGDIIQRLDPPEQDAQIDRLINGRLTTLNAFVAQQLVRSESAALSAQLAKDKVNECVKAQSKRSGFCGQGTHIVSFVVNAPNGLYFMHVGYYPSNHIEVVSAYGLCDAANPTNCIAPVNGYFIKTNNTRIVDEWSYTGSSFYAPEPITSLNTKYVAPQVTYQNISTNLPPPLLGNSTGIDFQDELDEFFKNVSTSIPNFGSLTQINTTLLDLTYEMLSLQQVVKALNESYIDLKELGNYTY

SEQ ID NO: 66 - protein, 1273 aa, Artificial Sequence
  mutant spike of MERS-CoV comprising substitution L506R
VDVGPDSVKSACIEVDIQQTFFDKTWPRPIDVSKADGIIYPQGRTYSNITITYQGLFPYQGDHGDMYVYSAGHATGTTPQKLFVANYSQDVKQFANGFVVRIGAAANSTGTVIISPSTSATIRKIYPAFMLGSSVGNFSDGKMGRFFNHTLVLLPDGCGTLLRAFYCILEPRSGNHCPAGNSYTSFATYHTPATDCSDGNYNRNASLNSFKEYFNLRNCTFMYTYNITEDEILEWFGITQTAQGVHLFSSRYVDLYGGNMFQFATLPVYDTIKYYSIIPHSIRSIQSDRKAWAAFYVYKLQPLTFLLDFSVDGYIRRAIDCGFNDLSQLHCSYESFDVESGVYSVSSFEAKPSGSVVEQAEGVECDFSPLLSGTPPQVYNFKRLVFTNCNYNLTKLLSLFSVNDFTCSQISPAAIASNCYSSLILDYFSYPLSMKSDLSVSSAGPISQFNYKQSFSNPTCLILATVPHNLTTITKPLKYSYINKCSRRLSDDRTEVPQLVNANQYSPCVSIVPSTVWEDGDYYRKQLSPLEGGGWLVASGSTVAMTEQLQMGFGITVQYGTDTNSVCPKLEFANDTKIASQLGNCVEYSLYGVSGRGVFQNCTAVGVRQQRFVYDAYQNLVGYYSDDGNYYCLRACVSVPVSVIYDKETKTHATLFGSVACEHISSTMSQYSRSTRSMLKRRDSTYGPLQTPVGCVLGLVNSSLFVEDCKLPLGQSLCALPDTPSTLTPASVGSVPGEMRLASIAFNHPIQVDQLNSSYFKLSIPTNFSFGVTQEYIQTTIQKVTVDCKQYVCNGFQKCEQLLREYGQFCSKINQALHGANLRQDDSVRNLFASVKSSQSSPIIPGFGGDFNLTLLEPVSISTGSRSARSAIEDLLFDKVTIADPGYMQGYDDCMQQGPASARDLICAQYVAGYKVLPPLMDVNMEAAYTSSLLGSIAGVGWTAGLSSFAAIPFAQSIFYRLNGVGITQQVLSENQKLIANKFNQALGAMQTGFTTTNEAFQKVQDAVNNNAQALSKLASELSNTFGAISASIGDIIQRLDPPEQDAQIDRLINGRLTTLNAFVAQQLVRSESAALSAQLAKDKVNECVKAQSKRSGFCGQGTHIVSFVVNAPNGLYFMHVGYYPSNHIEVVSAYGLCDAANPTNCIAPVNGYFIKTNNTRIVDEWSYTGSSFYAPEPITSLNTKYVAPQVTYQNISTNLPPPLLGNSTGIDFQDELDEFFKNVSTSIPNFGSLTQINTTLLDLTYEMLSLQQVVKALNESYIDLKELGNYTY

SEQ ID NO: 67 - protein, 1273 aa, Artificial Sequence
  mutant spike of MERS-CoV comprising substitution L506W
VDVGPDSVKSACIEVDIQQTFFDKTWPRPIDVSKADGIIYPQGRTYSNITITYQGLFPYQGDHGDMYVYSAGHATGTTPQKLFVANYSQDVKQFANGFVVRIGAAANSTGTVIISPSTSATIRKIYPAFMLGSSVGNFSDGKMGRFFNHTLVLLPDGCGTLLRAFYCILEPRSGNHCPAGNSYTSFATYHTPATDCSDGNYNRNASLNSFKEYFNLRNCTFMYTYNITEDEILEWFGITQTAQGVHLFSSRYVDLYGGNMFQFATLPVYDTIKYYSIIPHSIRSIQSDRKAWAAFYVYKLQPLTFLLDFSVDGYIRRAIDCGFNDLSQLHCSYESFDVESGVYSVSSFEAKPSGSVVEQAEGVECDFSPLLSGTPPQVYNFKRLVFTNCNYNLTKLLSLFSVNDFTCSQISPAAIASNCYSSLILDYFSYPLSMKSDLSVSSAGPISQFNYKQSFSNPTCLILATVPHNLTTITKPLKYSYINKCSRWLSDDRTEVPQLVNANQYSPCVSIVPSTVWEDGDYYRKQLSPLEGGGWLVASGSTVAMTEQLQMGFGITVQYGTDTNSVCPKLEFANDTKIASQLGNCVEYSLYGVSGRGVFQNCTAVGVRQQRFVYDAYQNLVGYYSDDGNYYCLRACVSVPVSVIYDKETKTHATLFGSVACEHISSTMSQYSRSTRSMLKRRDSTYGPLQTPVGCVLGLVNSSLFVEDCKLPLGQSLCALPDTPSTLTPASVGSVPGEMRLASIAFNHPIQVDQLNSSYFKLSIPTNFSFGVTQEYIQTTIQKVTVDCKQYVCNGFQKCEQLLREYGQFCSKINQALHGANLRQDDSVRNLFASVKSSQSSPIIPGFGGDFNLTLLEPVSISTGSRSARSAIEDLLFDKVTIADPGYMQGYDDCMQQGPASARDLICAQYVAGYKVLPPLMDVNMEAAYTSSLLGSIAGVGWTAGLSSFAAIPFAQSIFYRLNGVGITQQVLSENQKLIANKFNQALGAMQTGFTTTNEAFQKVQDAVNNNAQALSKLASELSNTFGAISASIGDIIQRLDPPEQDAQIDRLINGRLTTLNAFVAQQLVRSESAALSAQLAKDKVNECVKAQSKRSGFCGQGTHIVSFVVNAPNGLYFMHVGYYPSNHIEVVSAYGLCDAANPTNCIAPVNGYFIKTNNTRIVDEWSYTGSSFYAPEPITSLNTKYVAPQVTYQNISTNLPPPLLGNSTGIDFQDELDEFFKNVSTSIPNFGSLTQINTTLLDLTYEMLSLQQVVKALNESYIDLKELGNYTY

SEQ ID NO: 68 - protein, 1273 aa, Artificial Sequence
  mutant spike of MERS-CoV comprising substitution L506Y
VDVGPDSVKSACIEVDIQQTFFDKTWPRPIDVSKADGIIYPQGRTYSNITITYQGLFPYQGDHGDMYVYSAGHATGTTPQKLFVANYSQDVKQFANGFVVRIGAAANSTGTVIISPSTSATIRKIYPAFMLGSSVGNFSDGKMGRFFNHTLVLLPDGCGTLLRAFYCILEPRSGNHCPAGNSYTSFATYHTPATDCSDGNYNRNASLNSFKEYFNLRNCTFMYTYNITEDEILEWFGITQTAQGVHLFSSRYVDLYGGNMFQFATLPVYDTIKYYSIIPHSIRSIQSDRKAWAAFYVYKLQPLTFLLDFSVDGYIRRAIDCGFNDLSQLHCSYESFDVESGVYSVSSFEAKPSGSVVEQAEGVECDFSPLLSGTPPQVYNFKRLVFTNCNYNLTKLLSLFSVNDFTCSQISPAAIASNCYSSLILDYFSYPLSMKSDLSVSSAGPISQFNYKQSFSNPTCLILATVPHNLTTITKPLKYSYINKCSRYLSDDRTEVPQLVNANQYSPCVSIVPSTVWEDGDYYRKQLSPLEGGGWLVASGSTVAMTEQLQMGFGITVQYGTDTNSVCPKLEFANDTKIASQLGNCVEYSLYGVSGRGVFQNCTAVGVRQQRFVYDAYQNLVGYYSDDGNYYCLRACVSVPVSVIYDKETKTHATLFGSVACEHISSTMSQYSRSTRSMLKRRDSTYGPLQTPVGCVLGLVNSSLFVEDCKLPLGQSLCALPDTPSTLTPASVGSVPGEMRLASIAFNHPIQVDQLNSSYFKLSIPTNFSFGVTQEYIQTTIQKVTVDCKQYVCNGFQKCEQLLREYGQFCSKINQALHGANLRQDDSVRNLFASVKSSQSSPIIPGFGGDFNLTLLEPVSISTGSRSARSAIEDLLFDKVTIADPGYMQGYDDCMQQGPASARDLICAQYVAGYKVLPPLMDVNMEAAYTSSLLGSIAGVGWTAGLSSFAAIPFAQSIFYRLNGVGITQQVLSENQKLIANKFNQALGAMQTGFTTTNEAFQKVQDAVNNNAQALSKLASELSNTFGAISASIGDIIQRLDPPEQDAQIDRLINGRLTTLNAFVAQQLVRSESAALSAQLAKDKVNECVKAQSKRSGFCGQGTHIVSFVVNAPNGLYFMHVGYYPSNHIEVVSAYGLCDAANPTNCIAPVNGYFIKTNNTRIVDEWSYTGSSFYAPEPITSLNTKYVAPQVTYQNISTNLPPPLLGNSTGIDFQDELDEFFKNVSTSIPNFGSLTQINTTLLDLTYEMLSLQQVVKALNESYIDLKELGNYTY

SEQ ID NO: 69 - protein, 1273 aa, Artificial Sequence
  mutant spike of MERS-CoV comprising substitution L506H
VDVGPDSVKSACIEVDIQQTFFDKTWPRPIDVSKADGIIYPQGRTYSNITITYQGLFPYQGDHGDMYVYSAGHATGTTPQKLFVANYSQDVKQFANGFVVRIGAAANSTGTVIISPSTSATIRKIYPAFMLGSSVGNFSDGKMGRFFNHTLVLLPDGCGTLLRAFYCILEPRSGNHCPAGNSYTSFATYHTPATDCSDGNYNRNASLNSFKEYFNLRNCTFMYTYNITEDEILEWFGITQTAQGVHLFSSRYVDLYGGNMFQFATLPVYDTIKYYSIIPHSIRSIQSDRKAWAAFYVYKLQPLTFLLDFSVDGYIRRAIDCGFNDLSQLHCSYESFDVESGVYSVSSFEAKPSGSVVEQAEGVECDFSPLLSGTPPQVYNFKRLVFTNCNYNLTKLLSLFSVNDFTCSQISPAAIASNCYSSLILDYFSYPLSMKSDLSVSSAGPISQFNYKQSFSNPTCLILATVPHNLTTITKPLKYSYINKCSRHLSDDRTEVPQLVNANQYSPCVSIVPSTVWEDGDYYRKQLSPLEGGGWLVASGSTVAMTEQLQMGFGITVQYGTDTNSVCPKLEFANDTKIASQLGNCVEYSLYGVSGRGVFQNCTAVGVRQQRFVYDAYQNLVGYYSDDGNYYCLRACVSVPVSVIYDKETKTHATLFGSVACEHISSTMSQYSRSTRSMLKRRDSTYGPLQTPVGCVLGLVNSSLFVEDCKLPLGQSLCALPDTPSTLTPASVGSVPGEMRLASIAFNHPIQVDQLNSSYFKLSIPTNFSFGVTQEYIQTTIQKVTVDCKQYVCNGFQKCEQLLREYGQFCSKINQALHGANLRQDDSVRNLFASVKSSQSSPIIPGFGGDFNLTLLEPVSISTGSRSARSAIEDLLFDKVTIADPGYMQGYDDCMQQGPASARDLICAQYVAGYKVLPPLMDVNMEAAYTSSLLGSIAGVGWTAGLSSFAAIPFAQSIFYRLNGVGITQQVLSENQKLIANKFNQALGAMQTGFTTTNEAFQKVQDAVNNNAQALSKLASELSNTFGAISASIGDIIQRLDPPEQDAQIDRLINGRLTTLNAFVAQQLVRSESAALSAQLAKDKVNECVKAQSKRSGFCGQGTHIVSFVVNAPNGLYFMHVGYYPSNHIEVVSAYGLCDAANPTNCIAPVNGYFIKTNNTRIVDEWSYTGSSFYAPEPITSLNTKYVAPQVTYQNISTNLPPPLLGNSTGIDFQDELDEFFKNVSTSIPNFGSLTQINTTLLDLTYEMLSLQQVVKALNESYIDLKELGNYTY

SEQ ID NO: 70 - protein, 1273 aa, Artificial Sequence
  mutant spike of MERS-CoV comprising substitution G538H
VDVGPDSVKSACIEVDIQQTFFDKTWPRPIDVSKADGIIYPQGRTYSNITITYQGLFPYQGDHGDMYVYSAGHATGTTPQKLFVANYSQDVKQFANGFVVRIGAAANSTGTVIISPSTSATIRKIYPAFMLGSSVGNFSDGKMGRFFNHTLVLLPDGCGTLLRAFYCILEPRSGNHCPAGNSYTSFATYHTPATDCSDGNYNRNASLNSFKEYFNLRNCTFMYTYNITEDEILEWFGITQTAQGVHLFSSRYVDLYGGNMFQFATLPVYDTIKYYSIIPHSIRSIQSDRKAWAAFYVYKLQPLTFLLDFSVDGYIRRAIDCGFNDLSQLHCSYESFDVESGVYSVSSFEAKPSGSVVEQAEGVECDFSPLLSGTPPQVYNFKRLVFTNCNYNLTKLLSLFSVNDFTCSQISPAAIASNCYSSLILDYFSYPLSMKSDLSVSSAGPISQFNYKQSFSNPTCLILATVPHNLTTITKPLKYSYINKCSRLLSDDRTEVPQLVNANQYSPCVSIVPSTVWEDHDYYRKQLSPLEGGGWLVASGSTVAMTEQLQMGFGITVQYGTDTNSVCPKLEFANDTKIASQLGNCVEYSLYGVSGRGVFQNCTAVGVRQQRFVYDAYQNLVGYYSDDGNYYCLRACVSVPVSVIYDKETKTHATLFGSVACEHISSTMSQYSRSTRSMLKRRDSTYGPLQTPVGCVLGLVNSSLFVEDCKLPLGQSLCALPDTPSTLTPASVGSVPGEMRLASIAFNHPIQVDQLNSSYFKLSIPTNFSFGVTQEYIQTTIQKVTVDCKQYVCNGFQKCEQLLREYGQFCSKINQALHGANLRQDDSVRNLFASVKSSQSSPIIPGFGGDFNLTLLEPVSISTGSRSARSAIEDLLFDKVTIADPGYMQGYDDCMQQGPASARDLICAQYVAGYKVLPPLMDVNMEAAYTSSLLGSIAGVGWTAGLSSFAAIPFAQSIFYRLNGVGITQQVLSENQKLIANKFNQALGAMQTGFTTTNEAFQKVQDAVNNNAQALSKLASELSNTFGAISASIGDIIQRLDPPEQDAQIDRLINGRLTTLNAFVAQQLVRSESAALSAQLAKDKVNECVKAQSKRSGFCGQGTHIVSFVVNAPNGLYFMHVGYYPSNHIEVVSAYGLCDAANPTNCIAPVNGYFIKTNNTRIVDEWSYTGSSFYAPEPITSLNTKYVAPQVTYQNISTNLPPPLLGNSTGIDFQDELDEFFKNVSTSIPNFGSLTQINTTLLDLTYEMLSLQQVVKALNESYIDLKELGNYTY

SEQ ID NO: 71 - protein, 1273 aa, Artificial Sequence
  mutant spike of MERS-CoV comprising substitution G538W
VDVGPDSVKSACIEVDIQQTFFDKTWPRPIDVSKADGIIYPQGRTYSNITITYQGLFPYQGDHGDMYVYSAGHATGTTPQKLFVANYSQDVKQFANGFVVRIGAAANSTGTVIISPSTSATIRKIYPAFMLGSSVGNFSDGKMGRFFNHTLVLLPDGCGTLLRAFYCILEPRSGNHCPAGNSYTSFATYHTPATDCSDGNYNRNASLNSFKEYFNLRNCTFMYTYNITEDEILEWFGITQTAQGVHLFSSRYVDLYGGNMFQFATLPVYDTIKYYSIIPHSIRSIQSDRKAWAAFYVYKLQPLTFLLDFSVDGYIRRAIDCGFNDLSQLHCSYESFDVESGVYSVSSFEAKPSGSVVEQAEGVECDFSPLLSGTPPQVYNFKRLVFTNCNYNLTKLLSLFSVNDFTCSQISPAAIASNCYSSLILDYFSYPLSMKSDLSVSSAGPISQFNYKQSFSNPTCLILATVPHNLTTITKPLKYSYINKCSRLLSDDRTEVPQLVNANQYSPCVSIVPSTVWEDWDYYRKQLSPLEGGGWLVASGSTVAMTEQLQMGFGITVQYGTDTNSVCPKLEFANDTKIASQLGNCVEYSLYGVSGRGVFQNCTAVGVRQQRFVYDAYQNLVGYYSDDGNYYCLRACVSVPVSVIYDKETKTHATLFGSVACEHISSTMSQYSRSTRSMLKRRDSTYGPLQTPVGCVLGLVNSSLFVEDCKLPLGQSLCALPDTPSTLTPASVGSVPGEMRLASIAFNHPIQVDQLNSSYFKLSIPTNFSFGVTQEYIQTTIQKVTVDCKQYVCNGFQKCEQLLREYGQFCSKINQALHGANLRQDDSVRNLFASVKSSQSSPIIPGFGGDFNLTLLEPVSISTGSRSARSAIEDLLFDKVTIADPGYMQGYDDCMQQGPASARDLICAQYVAGYKVLPPLMDVNMEAAYTSSLLGSIAGVGWTAGLSSFAAIPFAQSIFYRLNGVGITQQVLSENQKLIANKFNQALGAMQTGFTTTNEAFQKVQDAVNNNAQALSKLASELSNTFGAISASIGDIIQRLDPPEQDAQIDRLINGRLTTLNAFVAQQLVRSESAALSAQLAKDKVNECVKAQSKRSGFCGQGTHIVSFVVNAPNGLYFMHVGYYPSNHIEVVSAYGLCDAANPTNCIAPVNGYFIKTNNTRIVDEWSYTGSSFYAPEPITSLNTKYVAPQVTYQNISTNLPPPLLGNSTGIDFQDELDEFFKNVSTSIPNFGSLTQINTTLLDLTYEMLSLQQVVKALNESYIDLKELGNYTY

SEQ ID NO: 72 - protein, 1273 aa, Artificial Sequence
  mutant spike of MERS-CoV comprising substitution G538E
VDVGPDSVKSACIEVDIQQTFFDKTWPRPIDVSKADGIIYPQGRTYSNITITYQGLFPYQGDHGDMYVYSAGHATGTTPQKLFVANYSQDVKQFANGFVVRIGAAANSTGTVIISPSTSATIRKIYPAFMLGSSVGNFSDGKMGRFFNHTLVLLPDGCGTLLRAFYCILEPRSGNHCPAGNSYTSFATYHTPATDCSDGNYNRNASLNSFKEYFNLRNCTFMYTYNITEDEILEWFGITQTAQGVHLFSSRYVDLYGGNMFQFATLPVYDTIKYYSIIPHSIRSIQSDRKAWAAFYVYKLQPLTFLLDFSVDGYIRRAIDCGFNDLSQLHCSYESFDVESGVYSVSSFEAKPSGSVVEQAEGVECDFSPLLSGTPPQVYNFKRLVFTNCNYNLTKLLSLFSVNDFTCSQISPAAIASNCYSSLILDYFSYPLSMKSDLSVSSAGPISQFNYKQSFSNPTCLILATVPHNLTTITKPLKYSYINKCSRLLSDDRTEVPQLVNANQYSPCVSIVPSTVWEDEDYYRKQLSPLEGGGWLVASGSTVAMTEQLQMGFGITVQYGTDTNSVCPKLEFANDTKIASQLGNCVEYSLYGVSGRGVFQNCTAVGVRQQRFVYDAYQNLVGYYSDDGNYYCLRACVSVPVSVIYDKETKTHATLFGSVACEHISSTMSQYSRSTRSMLKRRDSTYGPLQTPVGCVLGLVNSSLFVEDCKLPLGQSLCALPDTPSTLTPASVGSVPGEMRLASIAFNHPIQVDQLNSSYFKLSIPTNFSFGVTQEYIQTTIQKVTVDCKQYVCNGFQKCEQLLREYGQFCSKINQALHGANLRQDDSVRNLFASVKSSQSSPIIPGFGGDFNLTLLEPVSISTGSRSARSAIEDLLFDKVTIADPGYMQGYDDCMQQGPASARDLICAQYVAGYKVLPPLMDVNMEAAYTSSLLGSIAGVGWTAGLSSFAAIPFAQSIFYRLNGVGITQQVLSENQKLIANKFNQALGAMQTGFTTTNEAFQKVQDAVNNNAQALSKLASELSNTFGAISASIGDIIQRLDPPEQDAQIDRLINGRLTTLNAFVAQQLVRSESAALSAQLAKDKVNECVKAQSKRSGFCGQGTHIVSFVVNAPNGLYFMHVGYYPSNHIEVVSAYGLCDAANPTNCIAPVNGYFIKTNNTRIVDEWSYTGSSFYAPEPITSLNTKYVAPQVTYQNISTNLPPPLLGNSTGIDFQDELDEFFKNVSTSIPNFGSLTQINTTLLDLTYEMLSLQQVVKALNESYIDLKELGNYTY

SEQ ID NO: 73 - protein, 1273 aa, Artificial Sequence
  mutant spike of MERS-CoV comprising substitution G538K
VDVGPDSVKSACIEVDIQQTFFDKTWPRPIDVSKADGIIYPQGRTYSNITITYQGLFPYQGDHGDMYVYSAGHATGTTPQKLFVANYSQDVKQFANGFVVRIGAAANSTGTVIISPSTSATIRKIYPAFMLGSSVGNFSDGKMGRFFNHTLVLLPDGCGTLLRAFYCILEPRSGNHCPAGNSYTSFATYHTPATDCSDGNYNRNASLNSFKEYFNLRNCTFMYTYNITEDEILEWFGITQTAQGVHLFSSRYVDLYGGNMFQFATLPVYDTIKYYSIIPHSIRSIQSDRKAWAAFYVYKLQPLTFLLDFSVDGYIRRAIDCGFNDLSQLHCSYESFDVESGVYSVSSFEAKPSGSVVEQAEGVECDFSPLLSGTPPQVYNFKRLVFTNCNYNLTKLLSLFSVNDFTCSQISPAAIASNCYSSLILDYFSYPLSMKSDLSVSSAGPISQFNYKQSFSNPTCLILATVPHNLTTITKPLKYSYINKCSRLLSDDRTEVPQLVNANQYSPCVSIVPSTVWEDKDYYRKQLSPLEGGGWLVASGSTVAMTEQLQMGFGITVQYGTDTNSVCPKLEFANDTKIASQLGNCVEYSLYGVSGRGVFQNCTAVGVRQQRFVYDAYQNLVGYYSDDGNYYCLRACVSVPVSVIYDKETKTHATLFGSVACEHISSTMSQYSRSTRSMLKRRDSTYGPLQTPVGCVLGLVNSSLFVEDCKLPLGQSLCALPDTPSTLTPASVGSVPGEMRLASIAFNHPIQVDQLNSSYFKLSIPTNFSFGVTQEYIQTTIQKVTVDCKQYVCNGFQKCEQLLREYGQFCSKINQALHGANLRQDDSVRNLFASVKSSQSSPIIPGFGGDFNLTLLEPVSISTGSRSARSAIEDLLFDKVTIADPGYMQGYDDCMQQGPASARDLICAQYVAGYKVLPPLMDVNMEAAYTSSLLGSIAGVGWTAGLSSFAAIPFAQSIFYRLNGVGITQQVLSENQKLIANKFNQALGAMQTGFTTTNEAFQKVQDAVNNNAQALSKLASELSNTFGAISASIGDIIQRLDPPEQDAQIDRLINGRLTTLNAFVAQQLVRSESAALSAQLAKDKVNECVKAQSKRSGFCGQGTHIVSFVVNAPNGLYFMHVGYYPSNHIEVVSAYGLCDAANPTNCIAPVNGYFIKTNNTRIVDEWSYTGSSFYAPEPITSLNTKYVAPQVTYQNISTNLPPPLLGNSTGIDFQDELDEFFKNVSTSIPNFGSLTQINTTLLDLTYEMLSLQQVVKALNESYIDLKELGNYTY

SEQ ID NO: 74 - protein, 1273 aa, Artificial Sequence
  mutant spike of MERS-CoV comprising substitution G538F
VDVGPDSVKSACIEVDIQQTFFDKTWPRPIDVSKADGIIYPQGRTYSNITITYQGLFPYQGDHGDMYVYSAGHATGTTPQKLFVANYSQDVKQFANGFVVRIGAAANSTGTVIISPSTSATIRKIYPAFMLGSSVGNFSDGKMGRFFNHTLVLLPDGCGTLLRAFYCILEPRSGNHCPAGNSYTSFATYHTPATDCSDGNYNRNASLNSFKEYFNLRNCTFMYTYNITEDEILEWFGITQTAQGVHLFSSRYVDLYGGNMFQFATLPVYDTIKYYSIIPHSIRSIQSDRKAWAAFYVYKLQPLTFLLDFSVDGYIRRAIDCGFNDLSQLHCSYESFDVESGVYSVSSFEAKPSGSVVEQAEGVECDFSPLLSGTPPQVYNFKRLVFTNCNYNLTKLLSLFSVNDFTCSQISPAAIASNCYSSLILDYFSYPLSMKSDLSVSSAGPISQFNYKQSFSNPTCLILATVPHNLTTITKPLKYSYINKCSRLLSDDRTEVPQLVNANQYSPCVSIVPSTVWEDFDYYRKQLSPLEGGGWLVASGSTVAMTEQLQMGFGITVQYGTDTNSVCPKLEFANDTKIASQLGNCVEYSLYGVSGRGVFQNCTAVGVRQQRFVYDAYQNLVGYYSDDGNYYCLRACVSVPVSVIYDKETKTHATLFGSVACEHISSTMSQYSRSTRSMLKRRDSTYGPLQTPVGCVLGLVNSSLFVEDCKLPLGQSLCALPDTPSTLTPASVGSVPGEMRLASIAFNHPIQVDQLNSSYFKLSIPTNFSFGVTQEYIQTTIQKVTVDCKQYVCNGFQKCEQLLREYGQFCSKINQALHGANLRQDDSVRNLFASVKSSQSSPIIPGFGGDFNLTLLEPVSISTGSRSARSAIEDLLFDKVTIADPGYMQGYDDCMQQGPASARDLICAQYVAGYKVLPPLMDVNMEAAYTSSLLGSIAGVGWTAGLSSFAAIPFAQSIFYRLNGVGITQQVLSENQKLIANKFNQALGAMQTGFTTTNEAFQKVQDAVNNNAQALSKLASELSNTFGAISASIGDIIQRLDPPEQDAQIDRLINGRLTTLNAFVAQQLVRSESAALSAQLAKDKVNECVKAQSKRSGFCGQGTHIVSFVVNAPNGLYFMHVGYYPSNHIEVVSAYGLCDAANPTNCIAPVNGYFIKTNNTRIVDEWSYTGSSFYAPEPITSLNTKYVAPQVTYQNISTNLPPPLLGNSTGIDFQDELDEFFKNVSTSIPNFGSLTQINTTLLDLTYEMLSLQQVVKALNESYIDLKELGNYTY

SEQ ID NO: 75 - protein, 1273 aa, Artificial Sequence
  mutant spike of MERS-CoV comprising substitution G538L
VDVGPDSVKSACIEVDIQQTFFDKTWPRPIDVSKADGIIYPQGRTYSNITITYQGLFPYQGDHGDMYVYSAGHATGTTPQKLFVANYSQDVKQFANGFVVRIGAAANSTGTVIISPSTSATIRKIYPAFMLGSSVGNFSDGKMGRFFNHTLVLLPDGCGTLLRAFYCILEPRSGNHCPAGNSYTSFATYHTPATDCSDGNYNRNASLNSFKEYFNLRNCTFMYTYNITEDEILEWFGITQTAQGVHLFSSRYVDLYGGNMFQFATLPVYDTIKYYSIIPHSIRSIQSDRKAWAAFYVYKLQPLTFLLDFSVDGYIRRAIDCGFNDLSQLHCSYESFDVESGVYSVSSFEAKPSGSVVEQAEGVECDFSPLLSGTPPQVYNFKRLVFTNCNYNLTKLLSLFSVNDFTCSQISPAAIASNCYSSLILDYFSYPLSMKSDLSVSSAGPISQFNYKQSFSNPTCLILATVPHNLTTITKPLKYSYINKCSRLLSDDRTEVPQLVNANQYSPCVSIVPSTVWEDLDYYRKQLSPLEGGGWLVASGSTVAMTEQLQMGFGITVQYGTDTNSVCPKLEFANDTKIASQLGNCVEYSLYGVSGRGVFQNCTAVGVRQQRFVYDAYQNLVGYYSDDGNYYCLRACVSVPVSVIYDKETKTHATLFGSVACEHISSTMSQYSRSTRSMLKRRDSTYGPLQTPVGCVLGLVNSSLFVEDCKLPLGQSLCALPDTPSTLTPASVGSVPGEMRLASIAFNHPIQVDQLNSSYFKLSIPTNFSFGVTQEYIQTTIQKVTVDCKQYVCNGFQKCEQLLREYGQFCSKINQALHGANLRQDDSVRNLFASVKSSQSSPIIPGFGGDFNLTLLEPVSISTGSRSARSAIEDLLFDKVTIADPGYMQGYDDCMQQGPASARDLICAQYVAGYKVLPPLMDVNMEAAYTSSLLGSIAGVGWTAGLSSFAAIPFAQSIFYRLNGVGITQQVLSENQKLIANKFNQALGAMQTGFTTTNEAFQKVQDAVNNNAQALSKLASELSNTFGAISASIGDIIQRLDPPEQDAQIDRLINGRLTTLNAFVAQQLVRSESAALSAQLAKDKVNECVKAQSKRSGFCGQGTHIVSFVVNAPNGLYFMHVGYYPSNHIEVVSAYGLCDAANPTNCIAPVNGYFIKTNNTRIVDEWSYTGSSFYAPEPITSLNTKYVAPQVTYQNISTNLPPPLLGNSTGIDFQDELDEFFKNVSTSIPNFGSLTQINTTLLDLTYEMLSLQQVVKALNESYIDLKELGNYTY

SEQ ID NO: 76 - protein, 1273 aa, Artificial Sequence
  mutant spike of MERS-CoV comprising substitution G538S
VDVGPDSVKSACIEVDIQQTFFDKTWPRPIDVSKADGIIYPQGRTYSNITITYQGLFPYQGDHGDMYVYSAGHATGTTPQKLFVANYSQDVKQFANGFVVRIGAAANSTGTVIISPSTSATIRKIYPAFMLGSSVGNFSDGKMGRFFNHTLVLLPDGCGTLLRAFYCILEPRSGNHCPAGNSYTSFATYHTPATDCSDGNYNRNASLNSFKEYFNLRNCTFMYTYNITEDEILEWFGITQTAQGVHLFSSRYVDLYGGNMFQFATLPVYDTIKYYSIIPHSIRSIQSDRKAWAAFYVYKLQPLTFLLDFSVDGYIRRAIDCGFNDLSQLHCSYESFDVESGVYSVSSFEAKPSGSVVEQAEGVECDFSPLLSGTPPQVYNFKRLVFTNCNYNLTKLLSLFSVNDFTCSQISPAAIASNCYSSLILDYFSYPLSMKSDLSVSSAGPISQFNYKQSFSNPTCLILATVPHNLTTITKPLKYSYINKCSRLLSDDRTEVPQLVNANQYSPCVSIVPSTVWEDSDYYRKQLSPLEGGGWLVASGSTVAMTEQLQMGFGITVQYGTDTNSVCPKLEFANDTKIASQLGNCVEYSLYGVSGRGVFQNCTAVGVRQQRFVYDAYQNLVGYYSDDGNYYCLRACVSVPVSVIYDKETKTHATLFGSVACEHISSTMSQYSRSTRSMLKRRDSTYGPLQTPVGCVLGLVNSSLFVEDCKLPLGQSLCALPDTPSTLTPASVGSVPGEMRLASIAFNHPIQVDQLNSSYFKLSIPTNFSFGVTQEYIQTTIQKVTVDCKQYVCNGFQKCEQLLREYGQFCSKINQALHGANLRQDDSVRNLFASVKSSQSSPIIPGFGGDFNLTLLEPVSISTGSRSARSAIEDLLFDKVTIADPGYMQGYDDCMQQGPASARDLICAQYVAGYKVLPPLMDVNMEAAYTSSLLGSIAGVGWTAGLSSFAAIPFAQSIFYRLNGVGITQQVLSENQKLIANKFNQALGAMQTGFTTTNEAFQKVQDAVNNNAQALSKLASELSNTFGAISASIGDIIQRLDPPEQDAQIDRLINGRLTTLNAFVAQQLVRSESAALSAQLAKDKVNECVKAQSKRSGFCGQGTHIVSFVVNAPNGLYFMHVGYYPSNHIEVVSAYGLCDAANPTNCIAPVNGYFIKTNNTRIVDEWSYTGSSFYAPEPITSLNTKYVAPQVTYQNISTNLPPPLLGNSTGIDFQDELDEFFKNVSTSIPNFGSLTQINTTLLDLTYEMLSLQQVVKALNESYIDLKELGNYTY

SEQ ID NO: 77 - protein, 1273 aa, Artificial Sequence
  mutant spike of MERS-CoV comprising substitution G538Y
VDVGPDSVKSACIEVDIQQTFFDKTWPRPIDVSKADGIIYPQGRTYSNITITYQGLFPYQGDHGDMYVYSAGHATGTTPQKLFVANYSQDVKQFANGFVVRIGAAANSTGTVIISPSTSATIRKIYPAFMLGSSVGNFSDGKMGRFFNHTLVLLPDGCGTLLRAFYCILEPRSGNHCPAGNSYTSFATYHTPATDCSDGNYNRNASLNSFKEYFNLRNCTFMYTYNITEDEILEWFGITQTAQGVHLFSSRYVDLYGGNMFQFATLPVYDTIKYYSIIPHSIRSIQSDRKAWAAFYVYKLQPLTFLLDFSVDGYIRRAIDCGFNDLSQLHCSYESFDVESGVYSVSSFEAKPSGSVVEQAEGVECDFSPLLSGTPPQVYNFKRLVFTNCNYNLTKLLSLFSVNDFTCSQISPAAIASNCYSSLILDYFSYPLSMKSDLSVSSAGPISQFNYKQSFSNPTCLILATVPHNLTTITKPLKYSYINKCSRLLSDDRTEVPQLVNANQYSPCVSIVPSTVWEDYDYYRKQLSPLEGGGWLVASGSTVAMTEQLQMGFGITVQYGTDTNSVCPKLEFANDTKIASQLGNCVEYSLYGVSGRGVFQNCTAVGVRQQRFVYDAYQNLVGYYSDDGNYYCLRACVSVPVSVIYDKETKTHATLFGSVACEHISSTMSQYSRSTRSMLKRRDSTYGPLQTPVGCVLGLVNSSLFVEDCKLPLGQSLCALPDTPSTLTPASVGSVPGEMRLASIAFNHPIQVDQLNSSYFKLSIPTNFSFGVTQEYIQTTIQKVTVDCKQYVCNGFQKCEQLLREYGQFCSKINQALHGANLRQDDSVRNLFASVKSSQSSPIIPGFGGDFNLTLLEPVSISTGSRSARSAIEDLLFDKVTIADPGYMQGYDDCMQQGPASARDLICAQYVAGYKVLPPLMDVNMEAAYTSSLLGSIAGVGWTAGLSSFAAIPFAQSIFYRLNGVGITQQVLSENQKLIANKFNQALGAMQTGFTTTNEAFQKVQDAVNNNAQALSKLASELSNTFGAISASIGDIIQRLDPPEQDAQIDRLINGRLTTLNAFVAQQLVRSESAALSAQLAKDKVNECVKAQSKRSGFCGQGTHIVSFVVNAPNGLYFMHVGYYPSNHIEVVSAYGLCDAANPTNCIAPVNGYFIKTNNTRIVDEWSYTGSSFYAPEPITSLNTKYVAPQVTYQNISTNLPPPLLGNSTGIDFQDELDEFFKNVSTSIPNFGSLTQINTTLLDLTYEMLSLQQVVKALNESYIDLKELGNYTY

SEQ ID NO: 78 - protein, 1273 aa, Artificial Sequence
  mutant spike of MERS-CoV comprising substitution G538C
VDVGPDSVKSACIEVDIQQTFFDKTWPRPIDVSKADGIIYPQGRTYSNITITYQGLFPYQGDHGDMYVYSAGHATGTTPQKLFVANYSQDVKQFANGFVVRIGAAANSTGTVIISPSTSATIRKIYPAFMLGSSVGNFSDGKMGRFFNHTLVLLPDGCGTLLRAFYCILEPRSGNHCPAGNSYTSFATYHTPATDCSDGNYNRNASLNSFKEYFNLRNCTFMYTYNITEDEILEWFGITQTAQGVHLFSSRYVDLYGGNMFQFATLPVYDTIKYYSIIPHSIRSIQSDRKAWAAFYVYKLQPLTFLLDFSVDGYIRRAIDCGFNDLSQLHCSYESFDVESGVYSVSSFEAKPSGSVVEQAEGVECDFSPLLSGTPPQVYNFKRLVFTNCNYNLTKLLSLFSVNDFTCSQISPAAIASNCYSSLILDYFSYPLSMKSDLSVSSAGPISQFNYKQSFSNPTCLILATVPHNLTTITKPLKYSYINKCSRLLSDDRTEVPQLVNANQYSPCVSIVPSTVWEDCDYYRKQLSPLEGGGWLVASGSTVAMTEQLQMGFGITVQYGTDTNSVCPKLEFANDTKIASQLGNCVEYSLYGVSGRGVFQNCTAVGVRQQRFVYDAYQNLVGYYSDDGNYYCLRACVSVPVSVIYDKETKTHATLFGSVACEHISSTMSQYSRSTRSMLKRRDSTYGPLQTPVGCVLGLVNSSLFVEDCKLPLGQSLCALPDTPSTLTPASVGSVPGEMRLASIAFNHPIQVDQLNSSYFKLSIPTNFSFGVTQEYIQTTIQKVTVDCKQYVCNGFQKCEQLLREYGQFCSKINQALHGANLRQDDSVRNLFASVKSSQSSPIIPGFGGDFNLTLLEPVSISTGSRSARSAIEDLLFDKVTIADPGYMQGYDDCMQQGPASARDLICAQYVAGYKVLPPLMDVNMEAAYTSSLLGSIAGVGWTAGLSSFAAIPFAQSIFYRLNGVGITQQVLSENQKLIANKFNQALGAMQTGFTTTNEAFQKVQDAVNNNAQALSKLASELSNTFGAISASIGDIIQRLDPPEQDAQIDRLINGRLTTLNAFVAQQLVRSESAALSAQLAKDKVNECVKAQSKRSGFCGQGTHIVSFVVNAPNGLYFMHVGYYPSNHIEVVSAYGLCDAANPTNCIAPVNGYFIKTNNTRIVDEWSYTGSSFYAPEPITSLNTKYVAPQVTYQNISTNLPPPLLGNSTGIDFQDELDEFFKNVSTSIPNFGSLTQINTTLLDLTYEMLSLQQVVKALNESYIDLKELGNYTY

SEQ ID NO: 79 - protein, 1273 aa, Artificial Sequence
  mutant spike of MERS-CoV comprising substitution G538P
VDVGPDSVKSACIEVDIQQTFFDKTWPRPIDVSKADGIIYPQGRTYSNITITYQGLFPYQGDHGDMYVYSAGHATGTTPQKLFVANYSQDVKQFANGFVVRIGAAANSTGTVIISPSTSATIRKIYPAFMLGSSVGNFSDGKMGRFFNHTLVLLPDGCGTLLRAFYCILEPRSGNHCPAGNSYTSFATYHTPATDCSDGNYNRNASLNSFKEYFNLRNCTFMYTYNITEDEILEWFGITQTAQGVHLFSSRYVDLYGGNMFQFATLPVYDTIKYYSIIPHSIRSIQSDRKAWAAFYVYKLQPLTFLLDFSVDGYIRRAIDCGFNDLSQLHCSYESFDVESGVYSVSSFEAKPSGSVVEQAEGVECDFSPLLSGTPPQVYNFKRLVFTNCNYNLTKLLSLFSVNDFTCSQISPAAIASNCYSSLILDYFSYPLSMKSDLSVSSAGPISQFNYKQSFSNPTCLILATVPHNLTTITKPLKYSYINKCSRLLSDDRTEVPQLVNANQYSPCVSIVPSTVWEDPDYYRKQLSPLEGGGWLVASGSTVAMTEQLQMGFGITVQYGTDTNSVCPKLEFANDTKIASQLGNCVEYSLYGVSGRGVFQNCTAVGVRQQRFVYDAYQNLVGYYSDDGNYYCLRACVSVPVSVIYDKETKTHATLFGSVACEHISSTMSQYSRSTRSMLKRRDSTYGPLQTPVGCVLGLVNSSLFVEDCKLPLGQSLCALPDTPSTLTPASVGSVPGEMRLASIAFNHPIQVDQLNSSYFKLSIPTNFSFGVTQEYIQTTIQKVTVDCKQYVCNGFQKCEQLLREYGQFCSKINQALHGANLRQDDSVRNLFASVKSSQSSPIIPGFGGDFNLTLLEPVSISTGSRSARSAIEDLLFDKVTIADPGYMQGYDDCMQQGPASARDLICAQYVAGYKVLPPLMDVNMEAAYTSSLLGSIAGVGWTAGLSSFAAIPFAQSIFYRLNGVGITQQVLSENQKLIANKFNQALGAMQTGFTTTNEAFQKVQDAVNNNAQALSKLASELSNTFGAISASIGDIIQRLDPPEQDAQIDRLINGRLTTLNAFVAQQLVRSESAALSAQLAKDKVNECVKAQSKRSGFCGQGTHIVSFVVNAPNGLYFMHVGYYPSNHIEVVSAYGLCDAANPTNCIAPVNGYFIKTNNTRIVDEWSYTGSSFYAPEPITSLNTKYVAPQVTYQNISTNLPPPLLGNSTGIDFQDELDEFFKNVSTSIPNFGSLTQINTTLLDLTYEMLSLQQVVKALNESYIDLKELGNYTY

SEQ ID NO: 80 - protein, 1273 aa, Artificial Sequence
  mutant spike of MERS-CoV comprising substitution G538Q
VDVGPDSVKSACIEVDIQQTFFDKTWPRPIDVSKADGIIYPQGRTYSNITITYQGLFPYQGDHGDMYVYSAGHATGTTPQKLFVANYSQDVKQFANGFVVRIGAAANSTGTVIISPSTSATIRKIYPAFMLGSSVGNFSDGKMGRFFNHTLVLLPDGCGTLLRAFYCILEPRSGNHCPAGNSYTSFATYHTPATDCSDGNYNRNASLNSFKEYFNLRNCTFMYTYNITEDEILEWFGITQTAQGVHLFSSRYVDLYGGNMFQFATLPVYDTIKYYSIIPHSIRSIQSDRKAWAAFYVYKLQPLTFLLDFSVDGYIRRAIDCGFNDLSQLHCSYESFDVESGVYSVSSFEAKPSGSVVEQAEGVECDFSPLLSGTPPQVYNFKRLVFTNCNYNLTKLLSLFSVNDFTCSQISPAAIASNCYSSLILDYFSYPLSMKSDLSVSSAGPISQFNYKQSFSNPTCLILATVPHNLTTITKPLKYSYINKCSRLLSDDRTEVPQLVNANQYSPCVSIVPSTVWEDQDYYRKQLSPLEGGGWLVASGSTVAMTEQLQMGFGITVQYGTDTNSVCPKLEFANDTKIASQLGNCVEYSLYGVSGRGVFQNCTAVGVRQQRFVYDAYQNLVGYYSDDGNYYCLRACVSVPVSVIYDKETKTHATLFGSVACEHISSTMSQYSRSTRSMLKRRDSTYGPLQTPVGCVLGLVNSSLFVEDCKLPLGQSLCALPDTPSTLTPASVGSVPGEMRLASIAFNHPIQVDQLNSSYFKLSIPTNFSFGVTQEYIQTTIQKVTVDCKQYVCNGFQKCEQLLREYGQFCSKINQALHGANLRQDDSVRNLFASVKSSQSSPIIPGFGGDFNLTLLEPVSISTGSRSARSAIEDLLFDKVTIADPGYMQGYDDCMQQGPASARDLICAQYVAGYKVLPPLMDVNMEAAYTSSLLGSIAGVGWTAGLSSFAAIPFAQSIFYRLNGVGITQQVLSENQKLIANKFNQALGAMQTGFTTTNEAFQKVQDAVNNNAQALSKLASELSNTFGAISASIGDIIQRLDPPEQDAQIDRLINGRLTTLNAFVAQQLVRSESAALSAQLAKDKVNECVKAQSKRSGFCGQGTHIVSFVVNAPNGLYFMHVGYYPSNHIEVVSAYGLCDAANPTNCIAPVNGYFIKTNNTRIVDEWSYTGSSFYAPEPITSLNTKYVAPQVTYQNISTNLPPPLLGNSTGIDFQDELDEFFKNVSTSIPNFGSLTQINTTLLDLTYEMLSLQQVVKALNESYIDLKELGNYTY

SEQ ID NO: 81 - protein, 1273 aa, Artificial Sequence
  mutant spike of MERS-CoV comprising substitution G538I
VDVGPDSVKSACIEVDIQQTFFDKTWPRPIDVSKADGIIYPQGRTYSNITITYQGLFPYQGDHGDMYVYSAGHATGTTPQKLFVANYSQDVKQFANGFVVRIGAAANSTGTVIISPSTSATIRKIYPAFMLGSSVGNFSDGKMGRFFNHTLVLLPDGCGTLLRAFYCILEPRSGNHCPAGNSYTSFATYHTPATDCSDGNYNRNASLNSFKEYFNLRNCTFMYTYNITEDEILEWFGITQTAQGVHLFSSRYVDLYGGNMFQFATLPVYDTIKYYSIIPHSIRSIQSDRKAWAAFYVYKLQPLTFLLDFSVDGYIRRAIDCGFNDLSQLHCSYESFDVESGVYSVSSFEAKPSGSVVEQAEGVECDFSPLLSGTPPQVYNFKRLVFTNCNYNLTKLLSLFSVNDFTCSQISPAAIASNCYSSLILDYFSYPLSMKSDLSVSSAGPISQFNYKQSFSNPTCLILATVPHNLTTITKPLKYSYINKCSRLLSDDRTEVPQLVNANQYSPCVSIVPSTVWEDIDYYRKQLSPLEGGGWLVASGSTVAMTEQLQMGFGITVQYGTDTNSVCPKLEFANDTKIASQLGNCVEYSLYGVSGRGVFQNCTAVGVRQQRFVYDAYQNLVGYYSDDGNYYCLRACVSVPVSVIYDKETKTHATLFGSVACEHISSTMSQYSRSTRSMLKRRDSTYGPLQTPVGCVLGLVNSSLFVEDCKLPLGQSLCALPDTPSTLTPASVGSVPGEMRLASIAFNHPIQVDQLNSSYFKLSIPTNFSFGVTQEYIQTTIQKVTVDCKQYVCNGFQKCEQLLREYGQFCSKINQALHGANLRQDDSVRNLFASVKSSQSSPIIPGFGGDFNLTLLEPVSISTGSRSARSAIEDLLFDKVTIADPGYMQGYDDCMQQGPASARDLICAQYVAGYKVLPPLMDVNMEAAYTSSLLGSIAGVGWTAGLSSFAAIPFAQSIFYRLNGVGITQQVLSENQKLIANKFNQALGAMQTGFTTTNEAFQKVQDAVNNNAQALSKLASELSNTFGAISASIGDIIQRLDPPEQDAQIDRLINGRLTTLNAFVAQQLVRSESAALSAQLAKDKVNECVKAQSKRSGFCGQGTHIVSFVVNAPNGLYFMHVGYYPSNHIEVVSAYGLCDAANPTNCIAPVNGYFIKTNNTRIVDEWSYTGSSFYAPEPITSLNTKYVAPQVTYQNISTNLPPPLLGNSTGIDFQDELDEFFKNVSTSIPNFGSLTQINTTLLDLTYEMLSLQQVVKALNESYIDLKELGNYTY

SEQ ID NO: 82 - protein, 1273 aa, Artificial Sequence
  mutant spike of MERS-CoV comprising substitution G538M
VDVGPDSVKSACIEVDIQQTFFDKTWPRPIDVSKADGIIYPQGRTYSNITITYQGLFPYQGDHGDMYVYSAGHATGTTPQKLFVANYSQDVKQFANGFVVRIGAAANSTGTVIISPSTSATIRKIYPAFMLGSSVGNFSDGKMGRFFNHTLVLLPDGCGTLLRAFYCILEPRSGNHCPAGNSYTSFATYHTPATDCSDGNYNRNASLNSFKEYFNLRNCTFMYTYNITEDEILEWFGITQTAQGVHLFSSRYVDLYGGNMFQFATLPVYDTIKYYSIIPHSIRSIQSDRKAWAAFYVYKLQPLTFLLDFSVDGYIRRAIDCGFNDLSQLHCSYESFDVESGVYSVSSFEAKPSGSVVEQAEGVECDFSPLLSGTPPQVYNFKRLVFTNCNYNLTKLLSLFSVNDFTCSQISPAAIASNCYSSLILDYFSYPLSMKSDLSVSSAGPISQFNYKQSFSNPTCLILATVPHNLTTITKPLKYSYINKCSRLLSDDRTEVPQLVNANQYSPCVSIVPSTVWEDMDYYRKQLSPLEGGGWLVASGSTVAMTEQLQMGFGITVQYGTDTNSVCPKLEFANDTKIASQLGNCVEYSLYGVSGRGVFQNCTAVGVRQQRFVYDAYQNLVGYYSDDGNYYCLRACVSVPVSVIYDKETKTHATLFGSVACEHISSTMSQYSRSTRSMLKRRDSTYGPLQTPVGCVLGLVNSSLFVEDCKLPLGQSLCALPDTPSTLTPASVGSVPGEMRLASIAFNHPIQVDQLNSSYFKLSIPTNFSFGVTQEYIQTTIQKVTVDCKQYVCNGFQKCEQLLREYGQFCSKINQALHGANLRQDDSVRNLFASVKSSQSSPIIPGFGGDFNLTLLEPVSISTGSRSARSAIEDLLFDKVTIADPGYMQGYDDCMQQGPASARDLICAQYVAGYKVLPPLMDVNMEAAYTSSLLGSIAGVGWTAGLSSFAAIPFAQSIFYRLNGVGITQQVLSENQKLIANKFNQALGAMQTGFTTTNEAFQKVQDAVNNNAQALSKLASELSNTFGAISASIGDIIQRLDPPEQDAQIDRLINGRLTTLNAFVAQQLVRSESAALSAQLAKDKVNECVKAQSKRSGFCGQGTHIVSFVVNAPNGLYFMHVGYYPSNHIEVVSAYGLCDAANPTNCIAPVNGYFIKTNNTRIVDEWSYTGSSFYAPEPITSLNTKYVAPQVTYQNISTNLPPPLLGNSTGIDFQDELDEFFKNVSTSIPNFGSLTQINTTLLDLTYEMLSLQQVVKALNESYIDLKELGNYTY

SEQ ID NO: 83 - protein, 1273 aa, Artificial Sequence
  mutant spike of MERS-CoV comprising substitution G538T
VDVGPDSVKSACIEVDIQQTFFDKTWPRPIDVSKADGIIYPQGRTYSNITITYQGLFPYQGDHGDMYVYSAGHATGTTPQKLFVANYSQDVKQFANGFVVRIGAAANSTGTVIISPSTSATIRKIYPAFMLGSSVGNFSDGKMGRFFNHTLVLLPDGCGTLLRAFYCILEPRSGNHCPAGNSYTSFATYHTPATDCSDGNYNRNASLNSFKEYFNLRNCTFMYTYNITEDEILEWFGITQTAQGVHLFSSRYVDLYGGNMFQFATLPVYDTIKYYSIIPHSIRSIQSDRKAWAAFYVYKLQPLTFLLDFSVDGYIRRAIDCGFNDLSQLHCSYESFDVESGVYSVSSFEAKPSGSVVEQAEGVECDFSPLLSGTPPQVYNFKRLVFTNCNYNLTKLLSLFSVNDFTCSQISPAAIASNCYSSLILDYFSYPLSMKSDLSVSSAGPISQFNYKQSFSNPTCLILATVPHNLTTITKPLKYSYINKCSRLLSDDRTEVPQLVNANQYSPCVSIVPSTVWEDTDYYRKQLSPLEGGGWLVASGSTVAMTEQLQMGFGITVQYGTDTNSVCPKLEFANDTKIASQLGNCVEYSLYGVSGRGVFQNCTAVGVRQQRFVYDAYQNLVGYYSDDGNYYCLRACVSVPVSVIYDKETKTHATLFGSVACEHISSTMSQYSRSTRSMLKRRDSTYGPLQTPVGCVLGLVNSSLFVEDCKLPLGQSLCALPDTPSTLTPASVGSVPGEMRLASIAFNHPIQVDQLNSSYFKLSIPTNFSFGVTQEYIQTTIQKVTVDCKQYVCNGFQKCEQLLREYGQFCSKINQALHGANLRQDDSVRNLFASVKSSQSSPIIPGFGGDFNLTLLEPVSISTGSRSARSAIEDLLFDKVTIADPGYMQGYDDCMQQGPASARDLICAQYVAGYKVLPPLMDVNMEAAYTSSLLGSIAGVGWTAGLSSFAAIPFAQSIFYRLNGVGITQQVLSENQKLIANKFNQALGAMQTGFTTTNEAFQKVQDAVNNNAQALSKLASELSNTFGAISASIGDIIQRLDPPEQDAQIDRLINGRLTTLNAFVAQQLVRSESAALSAQLAKDKVNECVKAQSKRSGFCGQGTHIVSFVVNAPNGLYFMHVGYYPSNHIEVVSAYGLCDAANPTNCIAPVNGYFIKTNNTRIVDEWSYTGSSFYAPEPITSLNTKYVAPQVTYQNISTNLPPPLLGNSTGIDFQDELDEFFKNVSTSIPNFGSLTQINTTLLDLTYEMLSLQQVVKALNESYIDLKELGNYTY

SEQ ID NO: 84 - protein, 1273 aa, Artificial Sequence
  mutant spike of MERS-CoV comprising substitution G538N
VDVGPDSVKSACIEVDIQQTFFDKTWPRPIDVSKADGIIYPQGRTYSNITITYQGLFPYQGDHGDMYVYSAGHATGTTPQKLFVANYSQDVKQFANGFVVRIGAAANSTGTVIISPSTSATIRKIYPAFMLGSSVGNFSDGKMGRFFNHTLVLLPDGCGTLLRAFYCILEPRSGNHCPAGNSYTSFATYHTPATDCSDGNYNRNASLNSFKEYFNLRNCTFMYTYNITEDEILEWFGITQTAQGVHLFSSRYVDLYGGNMFQFATLPVYDTIKYYSIIPHSIRSIQSDRKAWAAFYVYKLQPLTFLLDFSVDGYIRRAIDCGFNDLSQLHCSYESFDVESGVYSVSSFEAKPSGSVVEQAEGVECDFSPLLSGTPPQVYNFKRLVFTNCNYNLTKLLSLFSVNDFTCSQISPAAIASNCYSSLILDYFSYPLSMKSDLSVSSAGPISQFNYKQSFSNPTCLILATVPHNLTTITKPLKYSYINKCSRLLSDDRTEVPQLVNANQYSPCVSIVPSTVWEDNDYYRKQLSPLEGGGWLVASGSTVAMTEQLQMGFGITVQYGTDTNSVCPKLEFANDTKIASQLGNCVEYSLYGVSGRGVFQNCTAVGVRQQRFVYDAYQNLVGYYSDDGNYYCLRACVSVPVSVIYDKETKTHATLFGSVACEHISSTMSQYSRSTRSMLKRRDSTYGPLQTPVGCVLGLVNSSLFVEDCKLPLGQSLCALPDTPSTLTPASVGSVPGEMRLASIAFNHPIQVDQLNSSYFKLSIPTNFSFGVTQEYIQTTIQKVTVDCKQYVCNGFQKCEQLLREYGQFCSKINQALHGANLRQDDSVRNLFASVKSSQSSPIIPGFGGDFNLTLLEPVSISTGSRSARSAIEDLLFDKVTIADPGYMQGYDDCMQQGPASARDLICAQYVAGYKVLPPLMDVNMEAAYTSSLLGSIAGVGWTAGLSSFAAIPFAQSIFYRLNGVGITQQVLSENQKLIANKFNQALGAMQTGFTTTNEAFQKVQDAVNNNAQALSKLASELSNTFGAISASIGDIIQRLDPPEQDAQIDRLINGRLTTLNAFVAQQLVRSESAALSAQLAKDKVNECVKAQSKRSGFCGQGTHIVSFVVNAPNGLYFMHVGYYPSNHIEVVSAYGLCDAANPTNCIAPVNGYFIKTNNTRIVDEWSYTGSSFYAPEPITSLNTKYVAPQVTYQNISTNLPPPLLGNSTGIDFQDELDEFFKNVSTSIPNFGSLTQINTTLLDLTYEMLSLQQVVKALNESYIDLKELGNYTY

SEQ ID NO: 85 - protein, 1273 aa, Artificial Sequence
  mutant spike of MERS-CoV comprising substitution G538R
VDVGPDSVKSACIEVDIQQTFFDKTWPRPIDVSKADGIIYPQGRTYSNITITYQGLFPYQGDHGDMYVYSAGHATGTTPQKLFVANYSQDVKQFANGFVVRIGAAANSTGTVIISPSTSATIRKIYPAFMLGSSVGNFSDGKMGRFFNHTLVLLPDGCGTLLRAFYCILEPRSGNHCPAGNSYTSFATYHTPATDCSDGNYNRNASLNSFKEYFNLRNCTFMYTYNITEDEILEWFGITQTAQGVHLFSSRYVDLYGGNMFQFATLPVYDTIKYYSIIPHSIRSIQSDRKAWAAFYVYKLQPLTFLLDFSVDGYIRRAIDCGFNDLSQLHCSYESFDVESGVYSVSSFEAKPSGSVVEQAEGVECDFSPLLSGTPPQVYNFKRLVFTNCNYNLTKLLSLFSVNDFTCSQISPAAIASNCYSSLILDYFSYPLSMKSDLSVSSAGPISQFNYKQSFSNPTCLILATVPHNLTTITKPLKYSYINKCSRLLSDDRTEVPQLVNANQYSPCVSIVPSTVWEDRDYYRKQLSPLEGGGWLVASGSTVAMTEQLQMGFGITVQYGTDTNSVCPKLEFANDTKIASQLGNCVEYSLYGVSGRGVFQNCTAVGVRQQRFVYDAYQNLVGYYSDDGNYYCLRACVSVPVSVIYDKETKTHATLFGSVACEHISSTMSQYSRSTRSMLKRRDSTYGPLQTPVGCVLGLVNSSLFVEDCKLPLGQSLCALPDTPSTLTPASVGSVPGEMRLASIAFNHPIQVDQLNSSYFKLSIPTNFSFGVTQEYIQTTIQKVTVDCKQYVCNGFQKCEQLLREYGQFCSKINQALHGANLRQDDSVRNLFASVKSSQSSPIIPGFGGDFNLTLLEPVSISTGSRSARSAIEDLLFDKVTIADPGYMQGYDDCMQQGPASARDLICAQYVAGYKVLPPLMDVNMEAAYTSSLLGSIAGVGWTAGLSSFAAIPFAQSIFYRLNGVGITQQVLSENQKLIANKFNQALGAMQTGFTTTNEAFQKVQDAVNNNAQALSKLASELSNTFGAISASIGDIIQRLDPPEQDAQIDRLINGRLTTLNAFVAQQLVRSESAALSAQLAKDKVNECVKAQSKRSGFCGQGTHIVSFVVNAPNGLYFMHVGYYPSNHIEVVSAYGLCDAANPTNCIAPVNGYFIKTNNTRIVDEWSYTGSSFYAPEPITSLNTKYVAPQVTYQNISTNLPPPLLGNSTGIDFQDELDEFFKNVSTSIPNFGSLTQINTTLLDLTYEMLSLQQVVKALNESYIDLKELGNYTY

SEQ ID NO: 86 - protein, 1273 aa, Artificial Sequence
  mutant spike of MERS-CoV comprising substitution G538V
VDVGPDSVKSACIEVDIQQTFFDKTWPRPIDVSKADGIIYPQGRTYSNITITYQGLFPYQGDHGDMYVYSAGHATGTTPQKLFVANYSQDVKQFANGFVVRIGAAANSTGTVIISPSTSATIRKIYPAFMLGSSVGNFSDGKMGRFFNHTLVLLPDGCGTLLRAFYCILEPRSGNHCPAGNSYTSFATYHTPATDCSDGNYNRNASLNSFKEYFNLRNCTFMYTYNITEDEILEWFGITQTAQGVHLFSSRYVDLYGGNMFQFATLPVYDTIKYYSIIPHSIRSIQSDRKAWAAFYVYKLQPLTFLLDFSVDGYIRRAIDCGFNDLSQLHCSYESFDVESGVYSVSSFEAKPSGSVVEQAEGVECDFSPLLSGTPPQVYNFKRLVFTNCNYNLTKLLSLFSVNDFTCSQISPAAIASNCYSSLILDYFSYPLSMKSDLSVSSAGPISQFNYKQSFSNPTCLILATVPHNLTTITKPLKYSYINKCSRLLSDDRTEVPQLVNANQYSPCVSIVPSTVWEDVDYYRKQLSPLEGGGWLVASGSTVAMTEQLQMGFGITVQYGTDTNSVCPKLEFANDTKIASQLGNCVEYSLYGVSGRGVFQNCTAVGVRQQRFVYDAYQNLVGYYSDDGNYYCLRACVSVPVSVIYDKETKTHATLFGSVACEHISSTMSQYSRSTRSMLKRRDSTYGPLQTPVGCVLGLVNSSLFVEDCKLPLGQSLCALPDTPSTLTPASVGSVPGEMRLASIAFNHPIQVDQLNSSYFKLSIPTNFSFGVTQEYIQTTIQKVTVDCKQYVCNGFQKCEQLLREYGQFCSKINQALHGANLRQDDSVRNLFASVKSSQSSPIIPGFGGDFNLTLLEPVSISTGSRSARSAIEDLLFDKVTIADPGYMQGYDDCMQQGPASARDLICAQYVAGYKVLPPLMDVNMEAAYTSSLLGSIAGVGWTAGLSSFAAIPFAQSIFYRLNGVGITQQVLSENQKLIANKFNQALGAMQTGFTTTNEAFQKVQDAVNNNAQALSKLASELSNTFGAISASIGDIIQRLDPPEQDAQIDRLINGRLTTLNAFVAQQLVRSESAALSAQLAKDKVNECVKAQSKRSGFCGQGTHIVSFVVNAPNGLYFMHVGYYPSNHIEVVSAYGLCDAANPTNCIAPVNGYFIKTNNTRIVDEWSYTGSSFYAPEPITSLNTKYVAPQVTYQNISTNLPPPLLGNSTGIDFQDELDEFFKNVSTSIPNFGSLTQINTTLLDLTYEMLSLQQVVKALNESYIDLKELGNYTY

SEQ ID NO: 87 - protein, 1273 aa, Artificial Sequence
  mutant spike of MERS-CoV comprising substitution G538A
VDVGPDSVKSACIEVDIQQTFFDKTWPRPIDVSKADGIIYPQGRTYSNITITYQGLFPYQGDHGDMYVYSAGHATGTTPQKLFVANYSQDVKQFANGFVVRIGAAANSTGTVIISPSTSATIRKIYPAFMLGSSVGNFSDGKMGRFFNHTLVLLPDGCGTLLRAFYCILEPRSGNHCPAGNSYTSFATYHTPATDCSDGNYNRNASLNSFKEYFNLRNCTFMYTYNITEDEILEWFGITQTAQGVHLFSSRYVDLYGGNMFQFATLPVYDTIKYYSIIPHSIRSIQSDRKAWAAFYVYKLQPLTFLLDFSVDGYIRRAIDCGFNDLSQLHCSYESFDVESGVYSVSSFEAKPSGSVVEQAEGVECDFSPLLSGTPPQVYNFKRLVFTNCNYNLTKLLSLFSVNDFTCSQISPAAIASNCYSSLILDYFSYPLSMKSDLSVSSAGPISQFNYKQSFSNPTCLILATVPHNLTTITKPLKYSYINKCSRLLSDDRTEVPQLVNANQYSPCVSIVPSTVWEDADYYRKQLSPLEGGGWLVASGSTVAMTEQLQMGFGITVQYGTDTNSVCPKLEFANDTKIASQLGNCVEYSLYGVSGRGVFQNCTAVGVRQQRFVYDAYQNLVGYYSDDGNYYCLRACVSVPVSVIYDKETKTHATLFGSVACEHISSTMSQYSRSTRSMLKRRDSTYGPLQTPVGCVLGLVNSSLFVEDCKLPLGQSLCALPDTPSTLTPASVGSVPGEMRLASIAFNHPIQVDQLNSSYFKLSIPTNFSFGVTQEYIQTTIQKVTVDCKQYVCNGFQKCEQLLREYGQFCSKINQALHGANLRQDDSVRNLFASVKSSQSSPIIPGFGGDFNLTLLEPVSISTGSRSARSAIEDLLFDKVTIADPGYMQGYDDCMQQGPASARDLICAQYVAGYKVLPPLMDVNMEAAYTSSLLGSIAGVGWTAGLSSFAAIPFAQSIFYRLNGVGITQQVLSENQKLIANKFNQALGAMQTGFTTTNEAFQKVQDAVNNNAQALSKLASELSNTFGAISASIGDIIQRLDPPEQDAQIDRLINGRLTTLNAFVAQQLVRSESAALSAQLAKDKVNECVKAQSKRSGFCGQGTHIVSFVVNAPNGLYFMHVGYYPSNHIEVVSAYGLCDAANPTNCIAPVNGYFIKTNNTRIVDEWSYTGSSFYAPEPITSLNTKYVAPQVTYQNISTNLPPPLLGNSTGIDFQDELDEFFKNVSTSIPNFGSLTQINTTLLDLTYEMLSLQQVVKALNESYIDLKELGNYTY

SEQ ID NO: 88 - protein, 1273 aa, Artificial Sequence
  mutant spike of MERS-CoV comprising substitution G538D
VDVGPDSVKSACIEVDIQQTFFDKTWPRPIDVSKADGIIYPQGRTYSNITITYQGLFPYQGDHGDMYVYSAGHATGTTPQKLFVANYSQDVKQFANGFVVRIGAAANSTGTVIISPSTSATIRKIYPAFMLGSSVGNFSDGKMGRFFNHTLVLLPDGCGTLLRAFYCILEPRSGNHCPAGNSYTSFATYHTPATDCSDGNYNRNASLNSFKEYFNLRNCTFMYTYNITEDEILEWFGITQTAQGVHLFSSRYVDLYGGNMFQFATLPVYDTIKYYSIIPHSIRSIQSDRKAWAAFYVYKLQPLTFLLDFSVDGYIRRAIDCGFNDLSQLHCSYESFDVESGVYSVSSFEAKPSGSVVEQAEGVECDFSPLLSGTPPQVYNFKRLVFTNCNYNLTKLLSLFSVNDFTCSQISPAAIASNCYSSLILDYFSYPLSMKSDLSVSSAGPISQFNYKQSFSNPTCLILATVPHNLTTITKPLKYSYINKCSRLLSDDRTEVPQLVNANQYSPCVSIVPSTVWEDDDYYRKQLSPLEGGGWLVASGSTVAMTEQLQMGFGITVQYGTDTNSVCPKLEFANDTKIASQLGNCVEYSLYGVSGRGVFQNCTAVGVRQQRFVYDAYQNLVGYYSDDGNYYCLRACVSVPVSVIYDKETKTHATLFGSVACEHISSTMSQYSRSTRSMLKRRDSTYGPLQTPVGCVLGLVNSSLFVEDCKLPLGQSLCALPDTPSTLTPASVGSVPGEMRLASIAFNHPIQVDQLNSSYFKLSIPTNFSFGVTQEYIQTTIQKVTVDCKQYVCNGFQKCEQLLREYGQFCSKINQALHGANLRQDDSVRNLFASVKSSQSSPIIPGFGGDFNLTLLEPVSISTGSRSARSAIEDLLFDKVTIADPGYMQGYDDCMQQGPASARDLICAQYVAGYKVLPPLMDVNMEAAYTSSLLGSIAGVGWTAGLSSFAAIPFAQSIFYRLNGVGITQQVLSENQKLIANKFNQALGAMQTGFTTTNEAFQKVQDAVNNNAQALSKLASELSNTFGAISASIGDIIQRLDPPEQDAQIDRLINGRLTTLNAFVAQQLVRSESAALSAQLAKDKVNECVKAQSKRSGFCGQGTHIVSFVVNAPNGLYFMHVGYYPSNHIEVVSAYGLCDAANPTNCIAPVNGYFIKTNNTRIVDEWSYTGSSFYAPEPITSLNTKYVAPQVTYQNISTNLPPPLLGNSTGIDFQDELDEFFKNVSTSIPNFGSLTQINTTLLDLTYEMLSLQQVVKALNESYIDLKELGNYTY

SEQ ID NO: 89 - protein, 1273 aa, Artificial Sequence
  mutant spike of MERS-CoV comprising substitution V555W
VDVGPDSVKSACIEVDIQQTFFDKTWPRPIDVSKADGIIYPQGRTYSNITITYQGLFPYQGDHGDMYVYSAGHATGTTPQKLFVANYSQDVKQFANGFVVRIGAAANSTGTVIISPSTSATIRKIYPAFMLGSSVGNFSDGKMGRFFNHTLVLLPDGCGTLLRAFYCILEPRSGNHCPAGNSYTSFATYHTPATDCSDGNYNRNASLNSFKEYFNLRNCTFMYTYNITEDEILEWFGITQTAQGVHLFSSRYVDLYGGNMFQFATLPVYDTIKYYSIIPHSIRSIQSDRKAWAAFYVYKLQPLTFLLDFSVDGYIRRAIDCGFNDLSQLHCSYESFDVESGVYSVSSFEAKPSGSVVEQAEGVECDFSPLLSGTPPQVYNFKRLVFTNCNYNLTKLLSLFSVNDFTCSQISPAAIASNCYSSLILDYFSYPLSMKSDLSVSSAGPISQFNYKQSFSNPTCLILATVPHNLTTITKPLKYSYINKCSRLLSDDRTEVPQLVNANQYSPCVSIVPSTVWEDGDYYRKQLSPLEGGGWLWASGSTVAMTEQLQMGFGITVQYGTDTNSVCPKLEFANDTKIASQLGNCVEYSLYGVSGRGVFQNCTAVGVRQQRFVYDAYQNLVGYYSDDGNYYCLRACVSVPVSVIYDKETKTHATLFGSVACEHISSTMSQYSRSTRSMLKRRDSTYGPLQTPVGCVLGLVNSSLFVEDCKLPLGQSLCALPDTPSTLTPASVGSVPGEMRLASIAFNHPIQVDQLNSSYFKLSIPTNFSFGVTQEYIQTTIQKVTVDCKQYVCNGFQKCEQLLREYGQFCSKINQALHGANLRQDDSVRNLFASVKSSQSSPIIPGFGGDFNLTLLEPVSISTGSRSARSAIEDLLFDKVTIADPGYMQGYDDCMQQGPASARDLICAQYVAGYKVLPPLMDVNMEAAYTSSLLGSIAGVGWTAGLSSFAAIPFAQSIFYRLNGVGITQQVLSENQKLIANKFNQALGAMQTGFTTTNEAFQKVQDAVNNNAQALSKLASELSNTFGAISASIGDIIQRLDPPEQDAQIDRLINGRLTTLNAFVAQQLVRSESAALSAQLAKDKVNECVKAQSKRSGFCGQGTHIVSFVVNAPNGLYFMHVGYYPSNHIEVVSAYGLCDAANPTNCIAPVNGYFIKTNNTRIVDEWSYTGSSFYAPEPITSLNTKYVAPQVTYQNISTNLPPPLLGNSTGIDFQDELDEFFKNVSTSIPNFGSLTQINTTLLDLTYEMLSLQQVVKALNESYIDLKELGNYTY

SEQ ID NO: 90 - protein, 1273 aa, Artificial Sequence
  mutant spike of MERS-CoV comprising substitution V555Y
VDVGPDSVKSACIEVDIQQTFFDKTWPRPIDVSKADGIIYPQGRTYSNITITYQGLFPYQGDHGDMYVYSAGHATGTTPQKLFVANYSQDVKQFANGFVVRIGAAANSTGTVIISPSTSATIRKIYPAFMLGSSVGNFSDGKMGRFFNHTLVLLPDGCGTLLRAFYCILEPRSGNHCPAGNSYTSFATYHTPATDCSDGNYNRNASLNSFKEYFNLRNCTFMYTYNITEDEILEWFGITQTAQGVHLFSSRYVDLYGGNMFQFATLPVYDTIKYYSIIPHSIRSIQSDRKAWAAFYVYKLQPLTFLLDFSVDGYIRRAIDCGFNDLSQLHCSYESFDVESGVYSVSSFEAKPSGSVVEQAEGVECDFSPLLSGTPPQVYNFKRLVFTNCNYNLTKLLSLFSVNDFTCSQISPAAIASNCYSSLILDYFSYPLSMKSDLSVSSAGPISQFNYKQSFSNPTCLILATVPHNLTTITKPLKYSYINKCSRLLSDDRTEVPQLVNANQYSPCVSIVPSTVWEDGDYYRKQLSPLEGGGWLYASGSTVAMTEQLQMGFGITVQYGTDTNSVCPKLEFANDTKIASQLGNCVEYSLYGVSGRGVFQNCTAVGVRQQRFVYDAYQNLVGYYSDDGNYYCLRACVSVPVSVIYDKETKTHATLFGSVACEHISSTMSQYSRSTRSMLKRRDSTYGPLQTPVGCVLGLVNSSLFVEDCKLPLGQSLCALPDTPSTLTPASVGSVPGEMRLASIAFNHPIQVDQLNSSYFKLSIPTNFSFGVTQEYIQTTIQKVTVDCKQYVCNGFQKCEQLLREYGQFCSKINQALHGANLRQDDSVRNLFASVKSSQSSPIIPGFGGDFNLTLLEPVSISTGSRSARSAIEDLLFDKVTIADPGYMQGYDDCMQQGPASARDLICAQYVAGYKVLPPLMDVNMEAAYTSSLLGSIAGVGWTAGLSSFAAIPFAQSIFYRLNGVGITQQVLSENQKLIANKFNQALGAMQTGFTTTNEAFQKVQDAVNNNAQALSKLASELSNTFGAISASIGDIIQRLDPPEQDAQIDRLINGRLTTLNAFVAQQLVRSESAALSAQLAKDKVNECVKAQSKRSGFCGQGTHIVSFVVNAPNGLYFMHVGYYPSNHIEVVSAYGLCDAANPTNCIAPVNGYFIKTNNTRIVDEWSYTGSSFYAPEPITSLNTKYVAPQVTYQNISTNLPPPLLGNSTGIDFQDELDEFFKNVSTSIPNFGSLTQINTTLLDLTYEMLSLQQVVKALNESYIDLKELGNYTY

SEQ ID NO: 91 - protein, 1273 aa, Artificial Sequence
  mutant spike of MERS-CoV comprising substitution V555F
VDVGPDSVKSACIEVDIQQTFFDKTWPRPIDVSKADGIIYPQGRTYSNITITYQGLFPYQGDHGDMYVYSAGHATGTTPQKLFVANYSQDVKQFANGFVVRIGAAANSTGTVIISPSTSATIRKIYPAFMLGSSVGNFSDGKMGRFFNHTLVLLPDGCGTLLRAFYCILEPRSGNHCPAGNSYTSFATYHTPATDCSDGNYNRNASLNSFKEYFNLRNCTFMYTYNITEDEILEWFGITQTAQGVHLFSSRYVDLYGGNMFQFATLPVYDTIKYYSIIPHSIRSIQSDRKAWAAFYVYKLQPLTFLLDFSVDGYIRRAIDCGFNDLSQLHCSYESFDVESGVYSVSSFEAKPSGSVVEQAEGVECDFSPLLSGTPPQVYNFKRLVFTNCNYNLTKLLSLFSVNDFTCSQISPAAIASNCYSSLILDYFSYPLSMKSDLSVSSAGPISQFNYKQSFSNPTCLILATVPHNLTTITKPLKYSYINKCSRLLSDDRTEVPQLVNANQYSPCVSIVPSTVWEDGDYYRKQLSPLEGGGWLFASGSTVAMTEQLQMGFGITVQYGTDTNSVCPKLEFANDTKIASQLGNCVEYSLYGVSGRGVFQNCTAVGVRQQRFVYDAYQNLVGYYSDDGNYYCLRACVSVPVSVIYDKETKTHATLFGSVACEHISSTMSQYSRSTRSMLKRRDSTYGPLQTPVGCVLGLVNSSLFVEDCKLPLGQSLCALPDTPSTLTPASVGSVPGEMRLASIAFNHPIQVDQLNSSYFKLSIPTNFSFGVTQEYIQTTIQKVTVDCKQYVCNGFQKCEQLLREYGQFCSKINQALHGANLRQDDSVRNLFASVKSSQSSPIIPGFGGDFNLTLLEPVSISTGSRSARSAIEDLLFDKVTIADPGYMQGYDDCMQQGPASARDLICAQYVAGYKVLPPLMDVNMEAAYTSSLLGSIAGVGWTAGLSSFAAIPFAQSIFYRLNGVGITQQVLSENQKLIANKFNQALGAMQTGFTTTNEAFQKVQDAVNNNAQALSKLASELSNTFGAISASIGDIIQRLDPPEQDAQIDRLINGRLTTLNAFVAQQLVRSESAALSAQLAKDKVNECVKAQSKRSGFCGQGTHIVSFVVNAPNGLYFMHVGYYPSNHIEVVSAYGLCDAANPTNCIAPVNGYFIKTNNTRIVDEWSYTGSSFYAPEPITSLNTKYVAPQVTYQNISTNLPPPLLGNSTGIDFQDELDEFFKNVSTSIPNFGSLTQINTTLLDLTYEMLSLQQVVKALNESYIDLKELGNYTY

SEQ ID NO: 92 - protein, 1273 aa, Artificial Sequence
  mutant spike of MERS-CoV comprising substitution V555R
VDVGPDSVKSACIEVDIQQTFFDKTWPRPIDVSKADGIIYPQGRTYSNITITYQGLFPYQGDHGDMYVYSAGHATGTTPQKLFVANYSQDVKQFANGFVVRIGAAANSTGTVIISPSTSATIRKIYPAFMLGSSVGNFSDGKMGRFFNHTLVLLPDGCGTLLRAFYCILEPRSGNHCPAGNSYTSFATYHTPATDCSDGNYNRNASLNSFKEYFNLRNCTFMYTYNITEDEILEWFGITQTAQGVHLFSSRYVDLYGGNMFQFATLPVYDTIKYYSIIPHSIRSIQSDRKAWAAFYVYKLQPLTFLLDFSVDGYIRRAIDCGFNDLSQLHCSYESFDVESGVYSVSSFEAKPSGSVVEQAEGVECDFSPLLSGTPPQVYNFKRLVFTNCNYNLTKLLSLFSVNDFTCSQISPAAIASNCYSSLILDYFSYPLSMKSDLSVSSAGPISQFNYKQSFSNPTCLILATVPHNLTTITKPLKYSYINKCSRLLSDDRTEVPQLVNANQYSPCVSIVPSTVWEDGDYYRKQLSPLEGGGWLRASGSTVAMTEQLQMGFGITVQYGTDTNSVCPKLEFANDTKIASQLGNCVEYSLYGVSGRGVFQNCTAVGVRQQRFVYDAYQNLVGYYSDDGNYYCLRACVSVPVSVIYDKETKTHATLFGSVACEHISSTMSQYSRSTRSMLKRRDSTYGPLQTPVGCVLGLVNSSLFVEDCKLPLGQSLCALPDTPSTLTPASVGSVPGEMRLASIAFNHPIQVDQLNSSYFKLSIPTNFSFGVTQEYIQTTIQKVTVDCKQYVCNGFQKCEQLLREYGQFCSKINQALHGANLRQDDSVRNLFASVKSSQSSPIIPGFGGDFNLTLLEPVSISTGSRSARSAIEDLLFDKVTIADPGYMQGYDDCMQQGPASARDLICAQYVAGYKVLPPLMDVNMEAAYTSSLLGSIAGVGWTAGLSSFAAIPFAQSIFYRLNGVGITQQVLSENQKLIANKFNQALGAMQTGFTTTNEAFQKVQDAVNNNAQALSKLASELSNTFGAISASIGDIIQRLDPPEQDAQIDRLINGRLTTLNAFVAQQLVRSESAALSAQLAKDKVNECVKAQSKRSGFCGQGTHIVSFVVNAPNGLYFMHVGYYPSNHIEVVSAYGLCDAANPTNCIAPVNGYFIKTNNTRIVDEWSYTGSSFYAPEPITSLNTKYVAPQVTYQNISTNLPPPLLGNSTGIDFQDELDEFFKNVSTSIPNFGSLTQINTTLLDLTYEMLSLQQVVKALNESYIDLKELGNYTY

SEQ ID NO: 93 - protein, 1273 aa, Artificial Sequence
  mutant spike of MERS-CoV comprising substitution V555K
VDVGPDSVKSACIEVDIQQTFFDKTWPRPIDVSKADGIIYPQGRTYSNITITYQGLFPYQGDHGDMYVYSAGHATGTTPQKLFVANYSQDVKQFANGFVVRIGAAANSTGTVIISPSTSATIRKIYPAFMLGSSVGNFSDGKMGRFFNHTLVLLPDGCGTLLRAFYCILEPRSGNHCPAGNSYTSFATYHTPATDCSDGNYNRNASLNSFKEYFNLRNCTFMYTYNITEDEILEWFGITQTAQGVHLFSSRYVDLYGGNMFQFATLPVYDTIKYYSIIPHSIRSIQSDRKAWAAFYVYKLQPLTFLLDFSVDGYIRRAIDCGFNDLSQLHCSYESFDVESGVYSVSSFEAKPSGSVVEQAEGVECDFSPLLSGTPPQVYNFKRLVFTNCNYNLTKLLSLFSVNDFTCSQISPAAIASNCYSSLILDYFSYPLSMKSDLSVSSAGPISQFNYKQSFSNPTCLILATVPHNLTTITKPLKYSYINKCSRLLSDDRTEVPQLVNANQYSPCVSIVPSTVWEDGDYYRKQLSPLEGGGWLKASGSTVAMTEQLQMGFGITVQYGTDTNSVCPKLEFANDTKIASQLGNCVEYSLYGVSGRGVFQNCTAVGVRQQRFVYDAYQNLVGYYSDDGNYYCLRACVSVPVSVIYDKETKTHATLFGSVACEHISSTMSQYSRSTRSMLKRRDSTYGPLQTPVGCVLGLVNSSLFVEDCKLPLGQSLCALPDTPSTLTPASVGSVPGEMRLASIAFNHPIQVDQLNSSYFKLSIPTNFSFGVTQEYIQTTIQKVTVDCKQYVCNGFQKCEQLLREYGQFCSKINQALHGANLRQDDSVRNLFASVKSSQSSPIIPGFGGDFNLTLLEPVSISTGSRSARSAIEDLLFDKVTIADPGYMQGYDDCMQQGPASARDLICAQYVAGYKVLPPLMDVNMEAAYTSSLLGSIAGVGWTAGLSSFAAIPFAQSIFYRLNGVGITQQVLSENQKLIANKFNQALGAMQTGFTTTNEAFQKVQDAVNNNAQALSKLASELSNTFGAISASIGDIIQRLDPPEQDAQIDRLINGRLTTLNAFVAQQLVRSESAALSAQLAKDKVNECVKAQSKRSGFCGQGTHIVSFVVNAPNGLYFMHVGYYPSNHIEVVSAYGLCDAANPTNCIAPVNGYFIKTNNTRIVDEWSYTGSSFYAPEPITSLNTKYVAPQVTYQNISTNLPPPLLGNSTGIDFQDELDEFFKNVSTSIPNFGSLTQINTTLLDLTYEMLSLQQVVKALNESYIDLKELGNYTY

SEQ ID NO: 94 - protein, 1273 aa, Artificial Sequence
  mutant spike of MERS-CoV comprising substitution S557Y
VDVGPDSVKSACIEVDIQQTFFDKTWPRPIDVSKADGIIYPQGRTYSNITITYQGLFPYQGDHGDMYVYSAGHATGTTPQKLFVANYSQDVKQFANGFVVRIGAAANSTGTVIISPSTSATIRKIYPAFMLGSSVGNFSDGKMGRFFNHTLVLLPDGCGTLLRAFYCILEPRSGNHCPAGNSYTSFATYHTPATDCSDGNYNRNASLNSFKEYFNLRNCTFMYTYNITEDEILEWFGITQTAQGVHLFSSRYVDLYGGNMFQFATLPVYDTIKYYSIIPHSIRSIQSDRKAWAAFYVYKLQPLTFLLDFSVDGYIRRAIDCGFNDLSQLHCSYESFDVESGVYSVSSFEAKPSGSVVEQAEGVECDFSPLLSGTPPQVYNFKRLVFTNCNYNLTKLLSLFSVNDFTCSQISPAAIASNCYSSLILDYFSYPLSMKSDLSVSSAGPISQFNYKQSFSNPTCLILATVPHNLTTITKPLKYSYINKCSRLLSDDRTEVPQLVNANQYSPCVSIVPSTVWEDGDYYRKQLSPLEGGGWLVAYGSTVAMTEQLQMGFGITVQYGTDTNSVCPKLEFANDTKIASQLGNCVEYSLYGVSGRGVFQNCTAVGVRQQRFVYDAYQNLVGYYSDDGNYYCLRACVSVPVSVIYDKETKTHATLFGSVACEHISSTMSQYSRSTRSMLKRRDSTYGPLQTPVGCVLGLVNSSLFVEDCKLPLGQSLCALPDTPSTLTPASVGSVPGEMRLASIAFNHPIQVDQLNSSYFKLSIPTNFSFGVTQEYIQTTIQKVTVDCKQYVCNGFQKCEQLLREYGQFCSKINQALHGANLRQDDSVRNLFASVKSSQSSPIIPGFGGDFNLTLLEPVSISTGSRSARSAIEDLLFDKVTIADPGYMQGYDDCMQQGPASARDLICAQYVAGYKVLPPLMDVNMEAAYTSSLLGSIAGVGWTAGLSSFAAIPFAQSIFYRLNGVGITQQVLSENQKLIANKFNQALGAMQTGFTTTNEAFQKVQDAVNNNAQALSKLASELSNTFGAISASIGDIIQRLDPPEQDAQIDRLINGRLTTLNAFVAQQLVRSESAALSAQLAKDKVNECVKAQSKRSGFCGQGTHIVSFVVNAPNGLYFMHVGYYPSNHIEVVSAYGLCDAANPTNCIAPVNGYFIKTNNTRIVDEWSYTGSSFYAPEPITSLNTKYVAPQVTYQNISTNLPPPLLGNSTGIDFQDELDEFFKNVSTSIPNFGSLTQINTTLLDLTYEMLSLQQVVKALNESYIDLKELGNYTY

SEQ ID NO: 95 - protein, 1273 aa, Artificial Sequence
  mutant spike of MERS-CoV comprising substitution S557W
VDVGPDSVKSACIEVDIQQTFFDKTWPRPIDVSKADGIIYPQGRTYSNITITYQGLFPYQGDHGDMYVYSAGHATGTTPQKLFVANYSQDVKQFANGFVVRIGAAANSTGTVIISPSTSATIRKIYPAFMLGSSVGNFSDGKMGRFFNHTLVLLPDGCGTLLRAFYCILEPRSGNHCPAGNSYTSFATYHTPATDCSDGNYNRNASLNSFKEYFNLRNCTFMYTYNITEDEILEWFGITQTAQGVHLFSSRYVDLYGGNMFQFATLPVYDTIKYYSIIPHSIRSIQSDRKAWAAFYVYKLQPLTFLLDFSVDGYIRRAIDCGFNDLSQLHCSYESFDVESGVYSVSSFEAKPSGSVVEQAEGVECDFSPLLSGTPPQVYNFKRLVFTNCNYNLTKLLSLFSVNDFTCSQISPAAIASNCYSSLILDYFSYPLSMKSDLSVSSAGPISQFNYKQSFSNPTCLILATVPHNLTTITKPLKYSYINKCSRLLSDDRTEVPQLVNANQYSPCVSIVPSTVWEDGDYYRKQLSPLEGGGWLVAWGSTVAMTEQLQMGFGITVQYGTDTNSVCPKLEFANDTKIASQLGNCVEYSLYGVSGRGVFQNCTAVGVRQQRFVYDAYQNLVGYYSDDGNYYCLRACVSVPVSVIYDKETKTHATLFGSVACEHISSTMSQYSRSTRSMLKRRDSTYGPLQTPVGCVLGLVNSSLFVEDCKLPLGQSLCALPDTPSTLTPASVGSVPGEMRLASIAFNHPIQVDQLNSSYFKLSIPTNFSFGVTQEYIQTTIQKVTVDCKQYVCNGFQKCEQLLREYGQFCSKINQALHGANLRQDDSVRNLFASVKSSQSSPIIPGFGGDFNLTLLEPVSISTGSRSARSAIEDLLFDKVTIADPGYMQGYDDCMQQGPASARDLICAQYVAGYKVLPPLMDVNMEAAYTSSLLGSIAGVGWTAGLSSFAAIPFAQSIFYRLNGVGITQQVLSENQKLIANKFNQALGAMQTGFTTTNEAFQKVQDAVNNNAQALSKLASELSNTFGAISASIGDIIQRLDPPEQDAQIDRLINGRLTTLNAFVAQQLVRSESAALSAQLAKDKVNECVKAQSKRSGFCGQGTHIVSFVVNAPNGLYFMHVGYYPSNHIEVVSAYGLCDAANPTNCIAPVNGYFIKTNNTRIVDEWSYTGSSFYAPEPITSLNTKYVAPQVTYQNISTNLPPPLLGNSTGIDFQDELDEFFKNVSTSIPNFGSLTQINTTLLDLTYEMLSLQQVVKALNESYIDLKELGNYTY

SEQ ID NO: 96 - protein, 1273 aa, Artificial Sequence
  mutant spike of MERS-CoV comprising substitution S557F
VDVGPDSVKSACIEVDIQQTFFDKTWPRPIDVSKADGIIYPQGRTYSNITITYQGLFPYQGDHGDMYVYSAGHATGTTPQKLFVANYSQDVKQFANGFVVRIGAAANSTGTVIISPSTSATIRKIYPAFMLGSSVGNFSDGKMGRFFNHTLVLLPDGCGTLLRAFYCILEPRSGNHCPAGNSYTSFATYHTPATDCSDGNYNRNASLNSFKEYFNLRNCTFMYTYNITEDEILEWFGITQTAQGVHLFSSRYVDLYGGNMFQFATLPVYDTIKYYSIIPHSIRSIQSDRKAWAAFYVYKLQPLTFLLDFSVDGYIRRAIDCGFNDLSQLHCSYESFDVESGVYSVSSFEAKPSGSVVEQAEGVECDFSPLLSGTPPQVYNFKRLVFTNCNYNLTKLLSLFSVNDFTCSQISPAAIASNCYSSLILDYFSYPLSMKSDLSVSSAGPISQFNYKQSFSNPTCLILATVPHNLTTITKPLKYSYINKCSRLLSDDRTEVPQLVNANQYSPCVSIVPSTVWEDGDYYRKQLSPLEGGGWLVAFGSTVAMTEQLQMGFGITVQYGTDTNSVCPKLEFANDTKIASQLGNCVEYSLYGVSGRGVFQNCTAVGVRQQRFVYDAYQNLVGYYSDDGNYYCLRACVSVPVSVIYDKETKTHATLFGSVACEHISSTMSQYSRSTRSMLKRRDSTYGPLQTPVGCVLGLVNSSLFVEDCKLPLGQSLCALPDTPSTLTPASVGSVPGEMRLASIAFNHPIQVDQLNSSYFKLSIPTNFSFGVTQEYIQTTIQKVTVDCKQYVCNGFQKCEQLLREYGQFCSKINQALHGANLRQDDSVRNLFASVKSSQSSPIIPGFGGDFNLTLLEPVSISTGSRSARSAIEDLLFDKVTIADPGYMQGYDDCMQQGPASARDLICAQYVAGYKVLPPLMDVNMEAAYTSSLLGSIAGVGWTAGLSSFAAIPFAQSIFYRLNGVGITQQVLSENQKLIANKFNQALGAMQTGFTTTNEAFQKVQDAVNNNAQALSKLASELSNTFGAISASIGDIIQRLDPPEQDAQIDRLINGRLTTLNAFVAQQLVRSESAALSAQLAKDKVNECVKAQSKRSGFCGQGTHIVSFVVNAPNGLYFMHVGYYPSNHIEVVSAYGLCDAANPTNCIAPVNGYFIKTNNTRIVDEWSYTGSSFYAPEPITSLNTKYVAPQVTYQNISTNLPPPLLGNSTGIDFQDELDEFFKNVSTSIPNFGSLTQINTTLLDLTYEMLSLQQVVKALNESYIDLKELGNYTY

SEQ ID NO: 97 - protein, 1273 aa, Artificial Sequence
  mutant spike of MERS-CoV comprising substitution R505L
VDVGPDSVKSACIEVDIQQTFFDKTWPRPIDVSKADGIIYPQGRTYSNITITYQGLFPYQGDHGDMYVYSAGHATGTTPQKLFVANYSQDVKQFANGFVVRIGAAANSTGTVIISPSTSATIRKIYPAFMLGSSVGNFSDGKMGRFFNHTLVLLPDGCGTLLRAFYCILEPRSGNHCPAGNSYTSFATYHTPATDCSDGNYNRNASLNSFKEYFNLRNCTFMYTYNITEDEILEWFGITQTAQGVHLFSSRYVDLYGGNMFQFATLPVYDTIKYYSIIPHSIRSIQSDRKAWAAFYVYKLQPLTFLLDFSVDGYIRRAIDCGFNDLSQLHCSYESFDVESGVYSVSSFEAKPSGSVVEQAEGVECDFSPLLSGTPPQVYNFKRLVFTNCNYNLTKLLSLFSVNDFTCSQISPAAIASNCYSSLILDYFSYPLSMKSDLSVSSAGPISQFNYKQSFSNPTCLILATVPHNLTTITKPLKYSYINKCSLLLSDDRTEVPQLVNANQYSPCVSIVPSTVWEDGDYYRKQLSPLEGGGWLVASGSTVAMTEQLQMGFGITVQYGTDTNSVCPKLEFANDTKIASQLGNCVEYSLYGVSGRGVFQNCTAVGVRQQRFVYDAYQNLVGYYSDDGNYYCLRACVSVPVSVIYDKETKTHATLFGSVACEHISSTMSQYSRSTRSMLKRRDSTYGPLQTPVGCVLGLVNSSLFVEDCKLPLGQSLCALPDTPSTLTPASVGSVPGEMRLASIAFNHPIQVDQLNSSYFKLSIPTNFSFGVTQEYIQTTIQKVTVDCKQYVCNGFQKCEQLLREYGQFCSKINQALHGANLRQDDSVRNLFASVKSSQSSPIIPGFGGDFNLTLLEPVSISTGSRSARSAIEDLLFDKVTIADPGYMQGYDDCMQQGPASARDLICAQYVAGYKVLPPLMDVNMEAAYTSSLLGSIAGVGWTAGLSSFAAIPFAQSIFYRLNGVGITQQVLSENQKLIANKFNQALGAMQTGFTTTNEAFQKVQDAVNNNAQALSKLASELSNTFGAISASIGDIIQRLDPPEQDAQIDRLINGRLTTLNAFVAQQLVRSESAALSAQLAKDKVNECVKAQSKRSGFCGQGTHIVSFVVNAPNGLYFMHVGYYPSNHIEVVSAYGLCDAANPTNCIAPVNGYFIKTNNTRIVDEWSYTGSSFYAPEPITSLNTKYVAPQVTYQNISTNLPPPLLGNSTGIDFQDELDEFFKNVSTSIPNFGSLTQINTTLLDLTYEMLSLQQVVKALNESYIDLKELGNYTY

SEQ ID NO: 98 - protein, 1273 aa, Artificial Sequence
  mutant spike of MERS-CoV comprising substitution V534W
VDVGPDSVKSACIEVDIQQTFFDKTWPRPIDVSKADGIIYPQGRTYSNITITYQGLFPYQGDHGDMYVYSAGHATGTTPQKLFVANYSQDVKQFANGFVVRIGAAANSTGTVIISPSTSATIRKIYPAFMLGSSVGNFSDGKMGRFFNHTLVLLPDGCGTLLRAFYCILEPRSGNHCPAGNSYTSFATYHTPATDCSDGNYNRNASLNSFKEYFNLRNCTFMYTYNITEDEILEWFGITQTAQGVHLFSSRYVDLYGGNMFQFATLPVYDTIKYYSIIPHSIRSIQSDRKAWAAFYVYKLQPLTFLLDFSVDGYIRRAIDCGFNDLSQLHCSYESFDVESGVYSVSSFEAKPSGSVVEQAEGVECDFSPLLSGTPPQVYNFKRLVFTNCNYNLTKLLSLFSVNDFTCSQISPAAIASNCYSSLILDYFSYPLSMKSDLSVSSAGPISQFNYKQSFSNPTCLILATVPHNLTTITKPLKYSYINKCSRLLSDDRTEVPQLVNANQYSPCVSIVPSTWWEDGDYYRKQLSPLEGGGWLVASGSTVAMTEQLQMGFGITVQYGTDTNSVCPKLEFANDTKIASQLGNCVEYSLYGVSGRGVFQNCTAVGVRQQRFVYDAYQNLVGYYSDDGNYYCLRACVSVPVSVIYDKETKTHATLFGSVACEHISSTMSQYSRSTRSMLKRRDSTYGPLQTPVGCVLGLVNSSLFVEDCKLPLGQSLCALPDTPSTLTPASVGSVPGEMRLASIAFNHPIQVDQLNSSYFKLSIPTNFSFGVTQEYIQTTIQKVTVDCKQYVCNGFQKCEQLLREYGQFCSKINQALHGANLRQDDSVRNLFASVKSSQSSPIIPGFGGDFNLTLLEPVSISTGSRSARSAIEDLLFDKVTIADPGYMQGYDDCMQQGPASARDLICAQYVAGYKVLPPLMDVNMEAAYTSSLLGSIAGVGWTAGLSSFAAIPFAQSIFYRLNGVGITQQVLSENQKLIANKFNQALGAMQTGFTTTNEAFQKVQDAVNNNAQALSKLASELSNTFGAISASIGDIIQRLDPPEQDAQIDRLINGRLTTLNAFVAQQLVRSESAALSAQLAKDKVNECVKAQSKRSGFCGQGTHIVSFVVNAPNGLYFMHVGYYPSNHIEVVSAYGLCDAANPTNCIAPVNGYFIKTNNTRIVDEWSYTGSSFYAPEPITSLNTKYVAPQVTYQNISTNLPPPLLGNSTGIDFQDELDEFFKNVSTSIPNFGSLTQINTTLLDLTYEMLSLQQVVKALNESYIDLKELGNYTY

SEQ ID NO: 99 - protein, 1273 aa, Artificial Sequence
  mutant spike of MERS-CoV comprising substitution A556W
VDVGPDSVKSACIEVDIQQTFFDKTWPRPIDVSKADGIIYPQGRTYSNITITYQGLFPYQGDHGDMYVYSAGHATGTTPQKLFVANYSQDVKQFANGFVVRIGAAANSTGTVIISPSTSATIRKIYPAFMLGSSVGNFSDGKMGRFFNHTLVLLPDGCGTLLRAFYCILEPRSGNHCPAGNSYTSFATYHTPATDCSDGNYNRNASLNSFKEYFNLRNCTFMYTYNITEDEILEWFGITQTAQGVHLFSSRYVDLYGGNMFQFATLPVYDTIKYYSIIPHSIRSIQSDRKAWAAFYVYKLQPLTFLLDFSVDGYIRRAIDCGFNDLSQLHCSYESFDVESGVYSVSSFEAKPSGSVVEQAEGVECDFSPLLSGTPPQVYNFKRLVFTNCNYNLTKLLSLFSVNDFTCSQISPAAIASNCYSSLILDYFSYPLSMKSDLSVSSAGPISQFNYKQSFSNPTCLILATVPHNLTTITKPLKYSYINKCSRLLSDDRTEVPQLVNANQYSPCVSIVPSTVWEDGDYYRKQLSPLEGGGWLVWSGSTVAMTEQLQMGFGITVQYGTDTNSVCPKLEFANDTKIASQLGNCVEYSLYGVSGRGVFQNCTAVGVRQQRFVYDAYQNLVGYYSDDGNYYCLRACVSVPVSVIYDKETKTHATLFGSVACEHISSTMSQYSRSTRSMLKRRDSTYGPLQTPVGCVLGLVNSSLFVEDCKLPLGQSLCALPDTPSTLTPASVGSVPGEMRLASIAFNHPIQVDQLNSSYFKLSIPTNFSFGVTQEYIQTTIQKVTVDCKQYVCNGFQKCEQLLREYGQFCSKINQALHGANLRQDDSVRNLFASVKSSQSSPIIPGFGGDFNLTLLEPVSISTGSRSARSAIEDLLFDKVTIADPGYMQGYDDCMQQGPASARDLICAQYVAGYKVLPPLMDVNMEAAYTSSLLGSIAGVGWTAGLSSFAAIPFAQSIFYRLNGVGITQQVLSENQKLIANKFNQALGAMQTGFTTTNEAFQKVQDAVNNNAQALSKLASELSNTFGAISASIGDIIQRLDPPEQDAQIDRLINGRLTTLNAFVAQQLVRSESAALSAQLAKDKVNECVKAQSKRSGFCGQGTHIVSFVVNAPNGLYFMHVGYYPSNHIEVVSAYGLCDAANPTNCIAPVNGYFIKTNNTRIVDEWSYTGSSFYAPEPITSLNTKYVAPQVTYQNISTNLPPPLLGNSTGIDFQDELDEFFKNVSTSIPNFGSLTQINTTLLDLTYEMLSLQQVVKALNESYIDLKELGNYTY

SEQ ID NO: 100 - protein, 1273 aa, Artificial Sequence
  mutant spike of MERS-CoV comprising substitution S559W
VDVGPDSVKSACIEVDIQQTFFDKTWPRPIDVSKADGIIYPQGRTYSNITITYQGLFPYQGDHGDMYVYSAGHATGTTPQKLFVANYSQDVKQFANGFVVRIGAAANSTGTVIISPSTSATIRKIYPAFMLGSSVGNFSDGKMGRFFNHTLVLLPDGCGTLLRAFYCILEPRSGNHCPAGNSYTSFATYHTPATDCSDGNYNRNASLNSFKEYFNLRNCTFMYTYNITEDEILEWFGITQTAQGVHLFSSRYVDLYGGNMFQFATLPVYDTIKYYSIIPHSIRSIQSDRKAWAAFYVYKLQPLTFLLDFSVDGYIRRAIDCGFNDLSQLHCSYESFDVESGVYSVSSFEAKPSGSVVEQAEGVECDFSPLLSGTPPQVYNFKRLVFTNCNYNLTKLLSLFSVNDFTCSQISPAAIASNCYSSLILDYFSYPLSMKSDLSVSSAGPISQFNYKQSFSNPTCLILATVPHNLTTITKPLKYSYINKCSRLLSDDRTEVPQLVNANQYSPCVSIVPSTVWEDGDYYRKQLSPLEGGGWLVASGWTVAMTEQLQMGFGITVQYGTDTNSVCPKLEFANDTKIASQLGNCVEYSLYGVSGRGVFQNCTAVGVRQQRFVYDAYQNLVGYYSDDGNYYCLRACVSVPVSVIYDKETKTHATLFGSVACEHISSTMSQYSRSTRSMLKRRDSTYGPLQTPVGCVLGLVNSSLFVEDCKLPLGQSLCALPDTPSTLTPASVGSVPGEMRLASIAFNHPIQVDQLNSSYFKLSIPTNFSFGVTQEYIQTTIQKVTVDCKQYVCNGFQKCEQLLREYGQFCSKINQALHGANLRQDDSVRNLFASVKSSQSSPIIPGFGGDFNLTLLEPVSISTGSRSARSAIEDLLFDKVTIADPGYMQGYDDCMQQGPASARDLICAQYVAGYKVLPPLMDVNMEAAYTSSLLGSIAGVGWTAGLSSFAAIPFAQSIFYRLNGVGITQQVLSENQKLIANKFNQALGAMQTGFTTTNEAFQKVQDAVNNNAQALSKLASELSNTFGAISASIGDIIQRLDPPEQDAQIDRLINGRLTTLNAFVAQQLVRSESAALSAQLAKDKVNECVKAQSKRSGFCGQGTHIVSFVVNAPNGLYFMHVGYYPSNHIEVVSAYGLCDAANPTNCIAPVNGYFIKTNNTRIVDEWSYTGSSFYAPEPITSLNTKYVAPQVTYQNISTNLPPPLLGNSTGIDFQDELDEFFKNVSTSIPNFGSLTQINTTLLDLTYEMLSLQQVVKALNESYIDLKELGNYTY

SEQ ID NO: 101 - protein, 19 aa, Artificial Sequence
  IgH signal peptide DPP4
MGWSCIILFLVATATGVHS

SEQ ID NO: 102 - protein, 31 aa, Artificial Sequence
  N-terminal domain pcDNA3.1+MERS RBD: Signal peptide, AviTag, GG linker
MFVFLVLLPLVSSQGLNDIFEAQKIEWHEGG

SEQ ID NO: 103 - protein, 39 aa, Artificial Sequence
  C-terminal Domain pcDNA3.1+ MERS RBD: GGGGS-linker, Twin-Strep-Tag, 6xHis-Tag
GGGGSWSHPQFEKGGGSGGGSGGSAWSHPQFEKHHHHHH

SEQ ID NO: 104 - protein, 76 aa, Artificial Sequence
  C-terminal Domain MERS Spike: TEV protease site, foldontrimerization motif, 6xHis-tag
SGRENLYFQGGGGSGYIPEAPRDGQAYVRKDGEWVLLSTFLGWSHPQFEKGGGSGGGSGGSAWSHPQFEKHHHHHH

SEQ ID NO: 105 - skipped

SEQ ID NO: 106 - DNA, 73 bp, Artificial Sequence
  forward primer
ctgcaaccggtgtacattctgaggtgcagctgctggagagcggcggcggcctggtgaagcccggcggcagcct

SEQ ID NO: 107 - DNA, 120 bp, Artificial Sequence
  forward primer
ggtgaagcccggcggcagcctgaggctgagctgcgaggccagcggcctgaccttcagcaacgtgtggatgagctgggtgaggcaggcccccggcaagggcctggagtgggtgggcaggat

SEQ ID NO: 108 - DNA, 120 bp, Artificial Sequence
  reverse primer
tgcaggtacacggtgttcttgctgtcgtccctgctcagggtgaacctgcccttcacgggggcgccgtagtcggtggtggcgccctcgctcttcctcttgatcctgcccacccactccagg

SEQ ID NO: 109 - DNA, 120 bp, Artificial Sequence
  reverse primer
ccagtagtcgaagtagtagctgctgctccacacgtcgccgcccctggtcagggtgctgcagtagtacacggcggtgtcgtcgatcttcaggctgttcatctgcaggtacacggtgttctt

SEQ ID NO: 110 - DNA, 69 bp, Artificial Sequence
  reverse primer
ctaggtcccttggtcgacgcgctgctcacggtcaccagggcgccctggccccagtagtcgaagtagtag

SEQ ID NO: 111 - DNA, 95 bp, Artificial Sequence
  forward primer
ctgcaaccggtgtacattcacagagcgccctgacccagcccgccagcgtgagcggcagccccggccagagcatcaccatcagctgcaccggcacc

SEQ ID NO: 112 - DNA, 120 bp, Artificial Sequence
  forward primer
accatcagctgcaccggcaccagcagcgacgtgggcacctacgacctggtgagctggtaccagcagcaccccggcaagagccccaagctgatgatctacgccgacatcaagaggcccagc

SEQ ID NO: 113 - DNA, 93 bp, Artificial Sequence
  reverse primer
ctgggggcggccaccgtacgggtcaccttggtgccgccgccgaagatcacgctggtgctgctgccggcgtacaggcagcagtagtagtcggcc

SEQ ID NO: 114 - DNA, 120 bp, Artificial Sequence
  reverse primer
ggcagcagtagtagtcggcctcgtcggcgctctgcaggccgctgatggtcaggctggcggtgttgccgctcttgctgccgctgaacctgtggctcacgccgctgggcctcttgatgtcgg

SEQ ID NO: 115 - DNA, 105 bp, Artificial Sequence
  forward primer
ctgcaaccggtgtacattctcaggtgcagctgcaggagagcggcggcggcctggtgaagcccggcggcagcctgaagctgagctgcgccgccagcggcttcacct

SEQ ID NO: 116 - DNA, 120 bp, Artificial Sequence
  forward primer
gcgccgccagcggcttcaccttcagcagctacaccatgagctgggtgaggcagacccccgacaagaggctggagtgggtggccaccatcagcagcggcggcagctacacctactaccccg

SEQ ID NO: 117 - DNA, 104 bp, Artificial Sequence
  reverse primer
ctaggtcccttggtcgacgcgctgctcacggtcaccatggtgccctggccccagtagtcgtagtcgttgccgtccctggcgcagtagtacatggcggtgtcctc

SEQ ID NO: 118 - DNA, 120 bp, Artificial Sequence
  reverse primer
tagtacatggcggtgtcctcgctcttcaggctgctcatctgcaggtacagggtgttcttggcgttgtccctgctgatggtgaacctgcccttcacgctgtcggggtagtaggtgtagctg

SEQ ID NO: 119 - DNA, 92 bp, Artificial Sequence
  forward primer
ctgcaaccggtgtacattcagacatccagctgacccagagccccagcagcctgagcgccagcatcggcgacagggtgaccatcacctgccag

SEQ ID NO: 120 - DNA, 120 bp, Artificial Sequence
  forward primer
agggtgaccatcacctgccaggccagccaggacatcagcaactacctgaactggtaccagcagaggcccggccaggcccccaagctgctgatctactacaccagcaggctgcacagcggc

SEQ ID NO: 121 - DNA, 90 bp, Artificial Sequence
  reverse primer
ctgggggcggccaccgtacgcttgatctccaccctggtgccgccgccgaaggtcctgggcagggtgttgccctgctggcagaagtaggtg

SEQ ID NO: 122 - DNA, 120 bp, Artificial Sequence
  reverse primer
cctgctggcagaagtaggtgccgatgtcctcggcctggaagctgttgatggcgatggtgaagctggtgccgctgcccctgccgctgaacctgctgggcacgccgctgtgcagcctgctgg

SEQ ID NO: 123 - DNA, 105 bp, Artificial Sequence
  forward primer
ctgcaaccggtgtacattctgaggtgaagctggtggagagcggcggcggcctggtgaagcccggcggcagcctgaagctgagctgcgccgccagcggcttcacct

SEQ ID NO: 124 - DNA, 120 bp, Artificial Sequence
  forward primer
gcgccgccagcggcttcaccttcagcagctacgccatgagctgggtgaggcagacccccgagaagaggctggagtgggtggccaccatcagcagcggcggcacctacacctactaccccg

SEQ ID NO: 125 - DNA, 104 bp, Artificial Sequence
  reverse primer
ctaggtcccttggtcgacgcgctgctcacggtcacgctggtgccctggccccagtagtccatgctgttgccgtccctcacgcagtagtacatggcggtgtcctc

SEQ ID NO: 126 - DNA, 120 bp, Artificial Sequence
  reverse primer
tagtacatggcggtgtcctcgctcctcaggctgctcatctgcaggtacagggtgttctcggcgttgtccctgctgatggtgaacctgcccttcacgctgtcggggtagtaggtgtaggtg

SEQ ID NO: 127 - DNA, 92 bp, Artificial Sequence
  forward primer
ctgcaaccggtgtacattcagacatccagatgacccagaccaccagcagcctgagcgccagcctgggcgacagggtgaccatcatctgcagg

SEQ ID NO: 128 - DNA, 117 bp, Artificial Sequence
  forward primer
agggtgaccatcatctgcagggccagccaggacatcaacaactacctgaactggtaccagaagcccgacggcaccgtgaagctgctgatctactacaccagcaggctgcacagcggc

SEQ ID NO: 129 - DNA, 90 bp, Artificial Sequence
  reverse primer
ctgggggcggccaccgtacgcctcagctccagcttggtgccggcgccgaaggtggggggcagggtgttggcctgctggcagaagtaggtg

SEQ ID NO: 130 - DNA, 120 bp, Artificial Sequence
  reverse primer
cctgctggcagaagtaggtggcgatgtcctcctgctccaggttgctgatggtcaggctgtagtcgctgccgctgccgctgccgctgaacctgctgggcacgccgctgtgcagcctgctgg

SEQ ID NO: 131 - DNA, 99 bp, Artificial Sequence
  forward primer
ctgcaaccggtgtacattctgaggtgcagctggtggagagcggcggcggcctggtgcagcccggcaggagcctgaggctgagctgcgccgccagcggct

SEQ ID NO: 132 - DNA, 120 bp, Artificial Sequence
  forward primer
tgagctgcgccgccagcggcttcaccttcagcaactacgccatgtactgggtgaggcaggcccccggcaagggcctggagtgggtggccctgatcagctacgacatcagcaccgactact

SEQ ID NO: 133 - DNA, 98 bp, Artificial Sequence
  reverse primer
ctaggtcccttggtcgacgcgctgctcacggtcaccagggtgccctggccccagtagtaggtgttggtgcagtagtacagggcggtgtcctcggtcct

SEQ ID NO: 134 - DNA, 120 bp, Artificial Sequence
  reverse primer
agggcggtgtcctcggtcctcaggttgttcatctgcaggtagatggtgttcttgctgttgtccctgctgatggtgaacctgcccttcacgctgtcggcgtagtagtcggtgctgatgtcg

SEQ ID NO: 135 - DNA, 96 bp, Artificial Sequence
  forward primer
ctgcaaccggtgtacattcacagagcgtgctgacccagagccccagcgccagcggcacccccggccagagggtgaccatcagctgcagcggcagca

SEQ ID NO: 136 - DNA, 120 bp, Artificial Sequence
  forward primer
ccatcagctgcagcggcagcagcagcaacatcggcaacaactacgtgtactggtaccagcagctgcccggcaccgcccccaagctgctgatctactggaacgaccagaggcccagcggcg

SEQ ID NO: 137 - DNA, 95 bp, Artificial Sequence
  reverse primer
ctgggggcggccaccgtacgcagcacggtcagctgggtgccgccgccgaacacggcgccgctcaggctgtcgtcccaggcggcgcagtagtagtc

SEQ ID NO: 138 - DNA, 120 bp, Artificial Sequence
  reverse primer
caggcggcgcagtagtagtcggcctcgtcctcgctcctcaggccgctgatggccaggctggcgctggtgccgctcttgctgccgctgaacctgtcgggcacgccgctgggcctctggtcg

SEQ ID NO: 139 - protein, 127 aa, Artificial Sequence
  LCA60 heavy chain insert
EVQLLESGGGLVKPGGSLRLSCEASGLTFSNVWMSWVRQAPGKGLEWVGRIKRKSEGATTDYGAPVKGRFTLSRDDSKNTVYLQMNSLKIDDTAVYYCSTLTRGGDVWSSSYYFDYWGQGALVTVSS

SEQ ID NO: 140 - protein, 109 aa, Artificial Sequence
  LCA60 light chain insert
QSALTQPASVSGSPGQSITISCTGTSSDVGTYDLVSWYQQHPGKSPKLMIYADIKRPSGVSHRFSGSKSGNTASLTISGLQSADEADYYCCLYAGSSTSVIFGGGTKVT

SEQ ID NO: 141 - protein, 116 aa, Artificial Sequence
  4C2h heavy chain insert
QVQLQESGGGLVKPGGSLKLSCAASGFTFSSYTMSWVRQTPDKRLEWVATISSGGSYTYYPDSVKGRFTISRDNAKNTLYLQMSSLKSEDTAMYYCARDGNDYDYWGQGTMVTVSS

SEQ ID NO: 142 - protein, 107 aa, Artificial Sequence
  4C2h light chain insert
DIQLTQSPSSLSASIGDRVTITCQASQDISNYLNWYQQRPGQAPKLLIYYTSRLHSGVPSRFSGRGSGTSFTIAINSFQAEDIGTYFCQQGNTLPRTFGGGTRVEIK

SEQ ID NO: 143 - protein, 116 aa, Artificial Sequence
  D12 heavy chain insert
EVKLVESGGGLVKPGGSLKLSCAASGFTFSSYAMSWVRQTPEKRLEWVATISSGGTYTYYPDSVKGRFTISRDNAENTLYLQMSSLRSEDTAMYYCVRDGNSMDYWGQGTSVTVSS

SEQ ID NO: 144 - protein, 107 aa, Artificial Sequence
  D12 light chain insert
DIQMTQTTSSLSASLGDRVTIICRASQDINNYLNWYQQKPDGTVKLLIYYTSRLHSGVPSRFSGSGSGSDYSLTISNLEQEDIATYFCQQANTLPPTFGAGTKLELR

SEQ ID NO: 145 - protein, 112 aa, Artificial Sequence
  MERS-4V2 heavy chain insert
EVQLVESGGGLVQPGRSLRLSCAASGFTFSNYAMYWVRQAPGKGLEWVALISYDISTDYYADSVKGRFTISRDNSKNTIYLQMNNLRTEDTALYYCTNTYYWGQGTLVTVSS

SEQ ID NO: 146 - protein, 110 aa, Artificial Sequence
  MERS-4V2 light chain insert
QSVLTQSPSASGTPGQRVTISCSGSSSNIGNNYVYWYQQLPGTAPKLLIYWNDQRPSGVPDRFSGSKSGTSASLAISGLRSEDEADYYCAAWDDSLSGAVFGGGTQLTVL

SEQ ID NO: 147 - protein, 1273 aa, Artificial Sequence
  mutant spike of MERS-CoV comprising substitution TS T424C S459C + G538E
VDVGPDSVKSACIEVDIQQTFFDKTWPRPIDVSKADGIIYPQGRTYSNITITYQGLFPYQGDHGDMYVYSAGHATGTTPQKLFVANYSQDVKQFANGFVVRIGAAANSTGTVIISPSTSATIRKIYPAFMLGSSVGNFSDGKMGRFFNHTLVLLPDGCGTLLRAFYCILEPRSGNHCPAGNSYTSFATYHTPATDCSDGNYNRNASLNSFKEYFNLRNCTFMYTYNITEDEILEWFGITQTAQGVHLFSSRYVDLYGGNMFQFATLPVYDTIKYYSIIPHSIRSIQSDRKAWAAFYVYKLQPLTFLLDFSVDGYIRRAIDCGFNDLSQLHCSYESFDVESGVYSVSSFEAKPSGSVVEQAEGVECDFSPLLSGTPPQVYNFKRLVFTNCNYNLTKLLSLFSVNDFCCSQISPAAIASNCYSSLILDYFSYPLSMKSDLSVCSAGPISQFNYKQSFSNPTCLILATVPHNLTTITKPLKYSYINKCSRLLSDDRTEVPQLVNANQYSPCVSIVPSTVWEDEDYYRKQLSPLEGGGWLVASGSTVAMTEQLQMGFGITVQYGTDTNSVCPKLEFANDTKIASQLGNCVEYSLYGVSGRGVFQNCTAVGVRQQRFVYDAYQNLVGYYSDDGNYYCLRACVSVPVSVIYDKETKTHATLFGSVACEHISSTMSQYSRSTRSMLKRRDSTYGPLQTPVGCVLGLVNSSLFVEDCKLPLGQSLCALPDTPSTLTPASVGSVPGEMRLASIAFNHPIQVDQLNSSYFKLSIPTNFSFGVTQEYIQTTIQKVTVDCKQYVCNGFQKCEQLLREYGQFCSKINQALHGANLRQDDSVRNLFASVKSSQSSPIIPGFGGDFNLTLLEPVSISTGSRSARSAIEDLLFDKVTIADPGYMQGYDDCMQQGPASARDLICAQYVAGYKVLPPLMDVNMEAAYTSSLLGSIAGVGWTAGLSSFAAIPFAQSIFYRLNGVGITQQVLSENQKLIANKFNQALGAMQTGFTTTNEAFQKVQDAVNNNAQALSKLASELSNTFGAISASIGDIIQRLDPPEQDAQIDRLINGRLTTLNAFVAQQLVRSESAALSAQLAKDKVNECVKAQSKRSGFCGQGTHIVSFVVNAPNGLYFMHVGYYPSNHIEVVSAYGLCDAANPTNCIAPVNGYFIKTNNTRIVDEWSYTGSSFYAPEPITSLNTKYVAPQVTYQNISTNLPPPLLGNSTGIDFQDELDEFFKNVSTSIPNFGSLTQINTTLLDLTYEMLSLQQVVKALNESYIDLKELGNYTY

SEQ ID NO: 148 - protein, 1273 aa, Artificial Sequence
  mutant spike of MERS-CoV comprising substitution TS T424C S459C + G538K
VDVGPDSVKSACIEVDIQQTFFDKTWPRPIDVSKADGIIYPQGRTYSNITITYQGLFPYQGDHGDMYVYSAGHATGTTPQKLFVANYSQDVKQFANGFVVRIGAAANSTGTVIISPSTSATIRKIYPAFMLGSSVGNFSDGKMGRFFNHTLVLLPDGCGTLLRAFYCILEPRSGNHCPAGNSYTSFATYHTPATDCSDGNYNRNASLNSFKEYFNLRNCTFMYTYNITEDEILEWFGITQTAQGVHLFSSRYVDLYGGNMFQFATLPVYDTIKYYSIIPHSIRSIQSDRKAWAAFYVYKLQPLTFLLDFSVDGYIRRAIDCGFNDLSQLHCSYESFDVESGVYSVSSFEAKPSGSVVEQAEGVECDFSPLLSGTPPQVYNFKRLVFTNCNYNLTKLLSLFSVNDFCCSQISPAAIASNCYSSLILDYFSYPLSMKSDLSVCSAGPISQFNYKQSFSNPTCLILATVPHNLTTITKPLKYSYINKCSRLLSDDRTEVPQLVNANQYSPCVSIVPSTVWEDKDYYRKQLSPLEGGGWLVASGSTVAMTEQLQMGFGITVQYGTDTNSVCPKLEFANDTKIASQLGNCVEYSLYGVSGRGVFQNCTAVGVRQQRFVYDAYQNLVGYYSDDGNYYCLRACVSVPVSVIYDKETKTHATLFGSVACEHISSTMSQYSRSTRSMLKRRDSTYGPLQTPVGCVLGLVNSSLFVEDCKLPLGQSLCALPDTPSTLTPASVGSVPGEMRLASIAFNHPIQVDQLNSSYFKLSIPTNFSFGVTQEYIQTTIQKVTVDCKQYVCNGFQKCEQLLREYGQFCSKINQALHGANLRQDDSVRNLFASVKSSQSSPIIPGFGGDFNLTLLEPVSISTGSRSARSAIEDLLFDKVTIADPGYMQGYDDCMQQGPASARDLICAQYVAGYKVLPPLMDVNMEAAYTSSLLGSIAGVGWTAGLSSFAAIPFAQSIFYRLNGVGITQQVLSENQKLIANKFNQALGAMQTGFTTTNEAFQKVQDAVNNNAQALSKLASELSNTFGAISASIGDIIQRLDPPEQDAQIDRLINGRLTTLNAFVAQQLVRSESAALSAQLAKDKVNECVKAQSKRSGFCGQGTHIVSFVVNAPNGLYFMHVGYYPSNHIEVVSAYGLCDAANPTNCIAPVNGYFIKTNNTRIVDEWSYTGSSFYAPEPITSLNTKYVAPQVTYQNISTNLPPPLLGNSTGIDFQDELDEFFKNVSTSIPNFGSLTQINTTLLDLTYEMLSLQQVVKALNESYIDLKELGNYTY

SEQ ID NO: 149 - protein, 1273 aa, Artificial Sequence
  mutant spike of MERS-CoV comprising substitution TS T424C S459C + G538Q
VDVGPDSVKSACIEVDIQQTFFDKTWPRPIDVSKADGIIYPQGRTYSNITITYQGLFPYQGDHGDMYVYSAGHATGTTPQKLFVANYSQDVKQFANGFVVRIGAAANSTGTVIISPSTSATIRKIYPAFMLGSSVGNFSDGKMGRFFNHTLVLLPDGCGTLLRAFYCILEPRSGNHCPAGNSYTSFATYHTPATDCSDGNYNRNASLNSFKEYFNLRNCTFMYTYNITEDEILEWFGITQTAQGVHLFSSRYVDLYGGNMFQFATLPVYDTIKYYSIIPHSIRSIQSDRKAWAAFYVYKLQPLTFLLDFSVDGYIRRAIDCGFNDLSQLHCSYESFDVESGVYSVSSFEAKPSGSVVEQAEGVECDFSPLLSGTPPQVYNFKRLVFTNCNYNLTKLLSLFSVNDFCCSQISPAAIASNCYSSLILDYFSYPLSMKSDLSVCSAGPISQFNYKQSFSNPTCLILATVPHNLTTITKPLKYSYINKCSRLLSDDRTEVPQLVNANQYSPCVSIVPSTVWEDQDYYRKQLSPLEGGGWLVASGSTVAMTEQLQMGFGITVQYGTDTNSVCPKLEFANDTKIASQLGNCVEYSLYGVSGRGVFQNCTAVGVRQQRFVYDAYQNLVGYYSDDGNYYCLRACVSVPVSVIYDKETKTHATLFGSVACEHISSTMSQYSRSTRSMLKRRDSTYGPLQTPVGCVLGLVNSSLFVEDCKLPLGQSLCALPDTPSTLTPASVGSVPGEMRLASIAFNHPIQVDQLNSSYFKLSIPTNFSFGVTQEYIQTTIQKVTVDCKQYVCNGFQKCEQLLREYGQFCSKINQALHGANLRQDDSVRNLFASVKSSQSSPIIPGFGGDFNLTLLEPVSISTGSRSARSAIEDLLFDKVTIADPGYMQGYDDCMQQGPASARDLICAQYVAGYKVLPPLMDVNMEAAYTSSLLGSIAGVGWTAGLSSFAAIPFAQSIFYRLNGVGITQQVLSENQKLIANKFNQALGAMQTGFTTTNEAFQKVQDAVNNNAQALSKLASELSNTFGAISASIGDIIQRLDPPEQDAQIDRLINGRLTTLNAFVAQQLVRSESAALSAQLAKDKVNECVKAQSKRSGFCGQGTHIVSFVVNAPNGLYFMHVGYYPSNHIEVVSAYGLCDAANPTNCIAPVNGYFIKTNNTRIVDEWSYTGSSFYAPEPITSLNTKYVAPQVTYQNISTNLPPPLLGNSTGIDFQDELDEFFKNVSTSIPNFGSLTQINTTLLDLTYEMLSLQQVVKALNESYIDLKELGNYTY

SEQ ID NO: 150 - protein, 1273 aa, Artificial Sequence
  mutant spike of MERS-CoV comprising substitution V555Y + F39A
VDVGPDSVKSACIEVDIQQTAFDKTWPRPIDVSKADGIIYPQGRTYSNITITYQGLFPYQGDHGDMYVYSAGHATGTTPQKLFVANYSQDVKQFANGFVVRIGAAANSTGTVIISPSTSATIRKIYPAFMLGSSVGNFSDGKMGRFFNHTLVLLPDGCGTLLRAFYCILEPRSGNHCPAGNSYTSFATYHTPATDCSDGNYNRNASLNSFKEYFNLRNCTFMYTYNITEDEILEWFGITQTAQGVHLFSSRYVDLYGGNMFQFATLPVYDTIKYYSIIPHSIRSIQSDRKAWAAFYVYKLQPLTFLLDFSVDGYIRRAIDCGFNDLSQLHCSYESFDVESGVYSVSSFEAKPSGSVVEQAEGVECDFSPLLSGTPPQVYNFKRLVFTNCNYNLTKLLSLFSVNDFTCSQISPAAIASNCYSSLILDYFSYPLSMKSDLSVSSAGPISQFNYKQSFSNPTCLILATVPHNLTTITKPLKYSYINKCSRLLSDDRTEVPQLVNANQYSPCVSIVPSTVWEDGDYYRKQLSPLEGGGWLYASGSTVAMTEQLQMGFGITVQYGTDTNSVCPKLEFANDTKIASQLGNCVEYSLYGVSGRGVFQNCTAVGVRQQRFVYDAYQNLVGYYSDDGNYYCLRACVSVPVSVIYDKETKTHATLFGSVACEHISSTMSQYSRSTRSMLKRRDSTYGPLQTPVGCVLGLVNSSLFVEDCKLPLGQSLCALPDTPSTLTPASVGSVPGEMRLASIAFNHPIQVDQLNSSYFKLSIPTNFSFGVTQEYIQTTIQKVTVDCKQYVCNGFQKCEQLLREYGQFCSKINQALHGANLRQDDSVRNLFASVKSSQSSPIIPGFGGDFNLTLLEPVSISTGSRSARSAIEDLLFDKVTIADPGYMQGYDDCMQQGPASARDLICAQYVAGYKVLPPLMDVNMEAAYTSSLLGSIAGVGWTAGLSSFAAIPFAQSIFYRLNGVGITQQVLSENQKLIANKFNQALGAMQTGFTTTNEAFQKVQDAVNNNAQALSKLASELSNTFGAISASIGDIIQRLDPPEQDAQIDRLINGRLTTLNAFVAQQLVRSESAALSAQLAKDKVNECVKAQSKRSGFCGQGTHIVSFVVNAPNGLYFMHVGYYPSNHIEVVSAYGLCDAANPTNCIAPVNGYFIKTNNTRIVDEWSYTGSSFYAPEPITSLNTKYVAPQVTYQNISTNLPPPLLGNSTGIDFQDELDEFFKNVSTSIPNFGSLTQINTTLLDLTYEMLSLQQVVKALNESYIDLKELGNYTY

SEQ ID NO: 151 - protein, 1273 aa, Artificial Sequence
  mutant spike of MERS-CoV comprising substitution V555Y + S133A
VDVGPDSVKSACIEVDIQQTFFDKTWPRPIDVSKADGIIYPQGRTYSNITITYQGLFPYQGDHGDMYVYSAGHATGTTPQKLFVANYSQDVKQFANGFVVRIGAAANSTGTVIIAPSTSATIRKIYPAFMLGSSVGNFSDGKMGRFFNHTLVLLPDGCGTLLRAFYCILEPRSGNHCPAGNSYTSFATYHTPATDCSDGNYNRNASLNSFKEYFNLRNCTFMYTYNITEDEILEWFGITQTAQGVHLFSSRYVDLYGGNMFQFATLPVYDTIKYYSIIPHSIRSIQSDRKAWAAFYVYKLQPLTFLLDFSVDGYIRRAIDCGFNDLSQLHCSYESFDVESGVYSVSSFEAKPSGSVVEQAEGVECDFSPLLSGTPPQVYNFKRLVFTNCNYNLTKLLSLFSVNDFTCSQISPAAIASNCYSSLILDYFSYPLSMKSDLSVSSAGPISQFNYKQSFSNPTCLILATVPHNLTTITKPLKYSYINKCSRLLSDDRTEVPQLVNANQYSPCVSIVPSTVWEDGDYYRKQLSPLEGGGWLYASGSTVAMTEQLQMGFGITVQYGTDTNSVCPKLEFANDTKIASQLGNCVEYSLYGVSGRGVFQNCTAVGVRQQRFVYDAYQNLVGYYSDDGNYYCLRACVSVPVSVIYDKETKTHATLFGSVACEHISSTMSQYSRSTRSMLKRRDSTYGPLQTPVGCVLGLVNSSLFVEDCKLPLGQSLCALPDTPSTLTPASVGSVPGEMRLASIAFNHPIQVDQLNSSYFKLSIPTNFSFGVTQEYIQTTIQKVTVDCKQYVCNGFQKCEQLLREYGQFCSKINQALHGANLRQDDSVRNLFASVKSSQSSPIIPGFGGDFNLTLLEPVSISTGSRSARSAIEDLLFDKVTIADPGYMQGYDDCMQQGPASARDLICAQYVAGYKVLPPLMDVNMEAAYTSSLLGSIAGVGWTAGLSSFAAIPFAQSIFYRLNGVGITQQVLSENQKLIANKFNQALGAMQTGFTTTNEAFQKVQDAVNNNAQALSKLASELSNTFGAISASIGDIIQRLDPPEQDAQIDRLINGRLTTLNAFVAQQLVRSESAALSAQLAKDKVNECVKAQSKRSGFCGQGTHIVSFVVNAPNGLYFMHVGYYPSNHIEVVSAYGLCDAANPTNCIAPVNGYFIKTNNTRIVDEWSYTGSSFYAPEPITSLNTKYVAPQVTYQNISTNLPPPLLGNSTGIDFQDELDEFFKNVSTSIPNFGSLTQINTTLLDLTYEMLSLQQVVKALNESYIDLKELGNYTY

SEQ ID NO: 152 - protein, 1273 aa, Artificial Sequence
  mutant spike of MERS-CoV comprising substitution V555Y + R307A
VDVGPDSVKSACIEVDIQQTFFDKTWPRPIDVSKADGIIYPQGRTYSNITITYQGLFPYQGDHGDMYVYSAGHATGTTPQKLFVANYSQDVKQFANGFVVRIGAAANSTGTVIISPSTSATIRKIYPAFMLGSSVGNFSDGKMGRFFNHTLVLLPDGCGTLLRAFYCILEPRSGNHCPAGNSYTSFATYHTPATDCSDGNYNRNASLNSFKEYFNLRNCTFMYTYNITEDEILEWFGITQTAQGVHLFSSRYVDLYGGNMFQFATLPVYDTIKYYSIIPHSIRSIQSDAKAWAAFYVYKLQPLTFLLDFSVDGYIRRAIDCGFNDLSQLHCSYESFDVESGVYSVSSFEAKPSGSVVEQAEGVECDFSPLLSGTPPQVYNFKRLVFTNCNYNLTKLLSLFSVNDFTCSQISPAAIASNCYSSLILDYFSYPLSMKSDLSVSSAGPISQFNYKQSFSNPTCLILATVPHNLTTITKPLKYSYINKCSRLLSDDRTEVPQLVNANQYSPCVSIVPSTVWEDGDYYRKQLSPLEGGGWLYASGSTVAMTEQLQMGFGITVQYGTDTNSVCPKLEFANDTKIASQLGNCVEYSLYGVSGRGVFQNCTAVGVRQQRFVYDAYQNLVGYYSDDGNYYCLRACVSVPVSVIYDKETKTHATLFGSVACEHISSTMSQYSRSTRSMLKRRDSTYGPLQTPVGCVLGLVNSSLFVEDCKLPLGQSLCALPDTPSTLTPASVGSVPGEMRLASIAFNHPIQVDQLNSSYFKLSIPTNFSFGVTQEYIQTTIQKVTVDCKQYVCNGFQKCEQLLREYGQFCSKINQALHGANLRQDDSVRNLFASVKSSQSSPIIPGFGGDFNLTLLEPVSISTGSRSARSAIEDLLFDKVTIADPGYMQGYDDCMQQGPASARDLICAQYVAGYKVLPPLMDVNMEAAYTSSLLGSIAGVGWTAGLSSFAAIPFAQSIFYRLNGVGITQQVLSENQKLIANKFNQALGAMQTGFTTTNEAFQKVQDAVNNNAQALSKLASELSNTFGAISASIGDIIQRLDPPEQDAQIDRLINGRLTTLNAFVAQQLVRSESAALSAQLAKDKVNECVKAQSKRSGFCGQGTHIVSFVVNAPNGLYFMHVGYYPSNHIEVVSAYGLCDAANPTNCIAPVNGYFIKTNNTRIVDEWSYTGSSFYAPEPITSLNTKYVAPQVTYQNISTNLPPPLLGNSTGIDFQDELDEFFKNVSTSIPNFGSLTQINTTLLDLTYEMLSLQQVVKALNESYIDLKELGNYTY

SEQ ID NO: 153 - protein, 1273 aa, Artificial Sequence
  mutant spike of MERS-CoV comprising substitution V555Y + H91A
VDVGPDSVKSACIEVDIQQTFFDKTWPRPIDVSKADGIIYPQGRTYSNITITYQGLFPYQGDHGDMYVYSAGAATGTTPQKLFVANYSQDVKQFANGFVVRIGAAANSTGTVIISPSTSATIRKIYPAFMLGSSVGNFSDGKMGRFFNHTLVLLPDGCGTLLRAFYCILEPRSGNHCPAGNSYTSFATYHTPATDCSDGNYNRNASLNSFKEYFNLRNCTFMYTYNITEDEILEWFGITQTAQGVHLFSSRYVDLYGGNMFQFATLPVYDTIKYYSIIPHSIRSIQSDRKAWAAFYVYKLQPLTFLLDFSVDGYIRRAIDCGFNDLSQLHCSYESFDVESGVYSVSSFEAKPSGSVVEQAEGVECDFSPLLSGTPPQVYNFKRLVFTNCNYNLTKLLSLFSVNDFTCSQISPAAIASNCYSSLILDYFSYPLSMKSDLSVSSAGPISQFNYKQSFSNPTCLILATVPHNLTTITKPLKYSYINKCSRLLSDDRTEVPQLVNANQYSPCVSIVPSTVWEDGDYYRKQLSPLEGGGWLYASGSTVAMTEQLQMGFGITVQYGTDTNSVCPKLEFANDTKIASQLGNCVEYSLYGVSGRGVFQNCTAVGVRQQRFVYDAYQNLVGYYSDDGNYYCLRACVSVPVSVIYDKETKTHATLFGSVACEHISSTMSQYSRSTRSMLKRRDSTYGPLQTPVGCVLGLVNSSLFVEDCKLPLGQSLCALPDTPSTLTPASVGSVPGEMRLASIAFNHPIQVDQLNSSYFKLSIPTNFSFGVTQEYIQTTIQKVTVDCKQYVCNGFQKCEQLLREYGQFCSKINQALHGANLRQDDSVRNLFASVKSSQSSPIIPGFGGDFNLTLLEPVSISTGSRSARSAIEDLLFDKVTIADPGYMQGYDDCMQQGPASARDLICAQYVAGYKVLPPLMDVNMEAAYTSSLLGSIAGVGWTAGLSSFAAIPFAQSIFYRLNGVGITQQVLSENQKLIANKFNQALGAMQTGFTTTNEAFQKVQDAVNNNAQALSKLASELSNTFGAISASIGDIIQRLDPPEQDAQIDRLINGRLTTLNAFVAQQLVRSESAALSAQLAKDKVNECVKAQSKRSGFCGQGTHIVSFVVNAPNGLYFMHVGYYPSNHIEVVSAYGLCDAANPTNCIAPVNGYFIKTNNTRIVDEWSYTGSSFYAPEPITSLNTKYVAPQVTYQNISTNLPPPLLGNSTGIDFQDELDEFFKNVSTSIPNFGSLTQINTTLLDLTYEMLSLQQVVKALNESYIDLKELGNYTY